European Patent Application EP 4 610 269 A1, published September 3, 2025. Title: Urokinase plasminogen activator surface receptor (uPAR) ligands for diagnostic or therapeutic use. Applicant: 3B Pharmaceuticals GmbH. Application EP. The sequence listing filed with the application follows.

SEQUENCE LISTING (357 sequences)

SEQ ID NO: 1 - protein, 335 aa, Homo sapiens
MGHPPLLPLLLLLHTCVPASWGLRCMQCKTNGDCRVEECALGQDLCRTTIVRLWEEGEELELVEKSCTHSEKTNRTLSYRTGLKITSLTEVVCGLDLCNQGNSGRAVTYSRSRYLECISCGSSDMSCERGRHQSLQCRSPEEQCLDVVTHWIQEGEEGRPKDDRHLRGCGYLPGCPGSNGFHNNDTFHFLKCCNTTKCNEGPILELENLPQNGRQCYSCKGNSTHGCSSEETFLIDCRGPMNQCLVATGTHEPKNQSYMVRGCATASMCQHAHLGDAFSMNHIDVSCCTKSGCNHPDLDVQYRSGAAPQPGPAHLSLTITLLMTARLWGGTLLWT

SEQ ID NO: 2 - protein, 11 aa, synthetic construct
  REGION 1..11: note = synthetic
  SITE 1: note = MISC_FEATURE - n-butyloxycarbonyl attached to Cys
  REGION 1..10: note = MISC_FEATURE - cycle formed
  SITE 3: note = MISC_FEATURE - Xaa is l-lysine DOTA conjugate
  SITE 6: note = MISC_FEATURE - Xaa is (2S,4S)-4-fluoro-pyrrolidine-2-carboxylic acid
  SITE 7: note = MISC_FEATURE - Xaa is 4-(R)-hydroxy-l-proline
  SITE 9: note = MISC_FEATURE - Xaa is l-norvaline
  SITE 11: note = MISC_FEATURE - Xaa is -alanine
CTXYFXXIXCX

SEQ ID NO: 3 - protein, 10 aa, synthetic construct
  REGION 1..10: note = synthetic
  SITE 1: note = MISC_FEATURE - n-butyloxycarbonyl attached to Cys
  REGION 1..10: note = MISC_FEATURE - cycle formed
  SITE 3: note = MISC_FEATURE - Xaa is l-lysine DOTA conjugate
  SITE 6: note = MISC_FEATURE - Xaa is 4-(R)-hydroxy-l-proline
  SITE 7: note = MISC_FEATURE - Xaa is 4-(R)-hydroxy-l-proline
  SITE 9: note = MISC_FEATURE - Xaa is l-norvaline
  SITE 10: note = MISC_FEATURE - NH2 attached to Cys
CTXYFXXIXC

SEQ ID NO: 4 - protein, 10 aa, synthetic construct
  REGION 1..10: note = synthetic
  SITE 1: note = MISC_FEATURE - n-butyloxycarbonyl attached to Cys
  REGION 1..10: note = MISC_FEATURE - cycle formed
  SITE 3: note = MISC_FEATURE - Xaa is l-lysine DOTA conjugate
  SITE 6: note = MISC_FEATURE - Xaa is (2S,4S)-4-fluoro-pyrrolidine-2-carboxylic acid
  SITE 7: note = MISC_FEATURE - Xaa is 4-(R)-hydroxy-l-proline
  SITE 9: note = MISC_FEATURE - Xaa is N,N-dimethyl diamino propionic acid
  SITE 10: note = MISC_FEATURE - NH2 attached to Cys
CTXYFXXIXC

SEQ ID NO: 5 - protein, 10 aa, synthetic construct
  REGION 1..10: note = synthetic
  SITE 1: note = MISC_FEATURE - isocaproic acid attached to Cys
  REGION 1..10: note = MISC_FEATURE - cycle formed
  SITE 2: note = MISC_FEATURE - Xaa is d-lysine DOTA conjugate
  SITE 7: note = MISC_FEATURE - Xaa is d-alanine
  SITE 10: note = MISC_FEATURE - NH2 attached to Cys
CXQYFPXILC

SEQ ID NO: 6 - protein, 10 aa, synthetic construct
  REGION 1..10: note = synthetic
  SITE 1: note = MISC_FEATURE - isocaproic acid attached to Cys
  REGION 1..10: note = MISC_FEATURE - cycle formed
  SITE 2: note = MISC_FEATURE - Xaa is l-Citrulline
  SITE 7: note = MISC_FEATURE - Xaa is d-alanine
CXQYFPXILC

SEQ ID NO: 7 - protein, 10 aa, synthetic construct
  REGION 1..10: note = synthetic
  SITE 1: note = MISC_FEATURE - pentanoic acid attached to Cys
  REGION 1..10: note = MISC_FEATURE - cycle formed
  SITE 2: note = MISC_FEATURE - Xaa is l-Citrulline
  SITE 3: note = MISC_FEATURE - Xaa is l-lysine Gd (III) DOTA conjugate
  SITE 5: note = MISC_FEATURE - Xaa is ortho-chloro-l-phenylalanine
  SITE 7: note = MISC_FEATURE - Xaa is 4-(R)-hydroxy-l-proline
  SITE 9: note = MISC_FEATURE - Xaa is l-norvaline
  SITE 10: note = MISC_FEATURE - NH2 attached to Cys
CXXYXPXIXC

SEQ ID NO: 8 - protein, 12 aa, synthetic construct
  REGION 1..12: note = synthetic
  SITE 1: note = MISC_FEATURE - Acetyl attached to d-aspartic acid
  SITE 1: note = MISC_FEATURE - Xaa is d-aspartic acid
  REGION 3..12: note = MISC_FEATURE - cycle formed
  SITE 5: note = MISC_FEATURE - Xaa is l-norleucine
  SITE 12: note = MISC_FEATURE - NH2 attached to Cys
XLCRXYFPAILC

SEQ ID NO: 9 - protein, 10 aa, synthetic construct
  REGION 1..10: note = synthetic
  SITE 1: note = MISC_FEATURE - n-butyloxycarbonyl attached to Cys
  REGION 1..10: note = MISC_FEATURE - cycle formed
  SITE 3: note = MISC_FEATURE - Xaa is l-lysine DOTA conjugate
  SITE 5: note = MISC_FEATURE - Xaa is l-thienylalanine
  SITE 7: note = MISC_FEATURE - Xaa is 4-(R)-hydroxy-l-proline
  SITE 9: note = MISC_FEATURE - Xaa is l-norvaline
  SITE 10: note = MISC_FEATURE - NH2 attached to Cys
CTXYXPXIXC

SEQ ID NO: 10 - protein, 10 aa, synthetic construct
  REGION 1..10: note = synthetic
  SITE 1: note = MISC_FEATURE - pentanoic acid attached to Cys
  REGION 1..10: note = MISC_FEATURE - cycle formed
  SITE 3: note = MISC_FEATURE - Xaa is l-lysine DOTA conjugate
  SITE 6: note = MISC_FEATURE - Xaa is 4-(R)-hydroxy-l-proline
  SITE 7: note = MISC_FEATURE - Xaa is 4-(R)-hydroxy-l-proline
  SITE 9: note = MISC_FEATURE - Xaa is l-norvaline
  SITE 10: note = MISC_FEATURE - NH2 attached to Cys
CTXYFXXIXC

SEQ ID NO: 11 - protein, 10 aa, synthetic construct
  REGION 1..10: note = synthetic
  SITE 1: note = MISC_FEATURE - isocaproic acid attached to Cys
  REGION 1..10: note = MISC_FEATURE - cycle formed
  SITE 2: note = MISC_FEATURE - Xaa is l-Citrulline
  SITE 7: note = MISC_FEATURE - Xaa is d-alanine
  SITE 8: note = MISC_FEATURE - Xaa is l-norvaline
  SITE 10: note = MISC_FEATURE - NH2 attached to Cys
CXQYFPXXLC

SEQ ID NO: 12 - protein, 12 aa, synthetic construct
  REGION 1..12: note = synthetic
  SITE 1: note = MISC_FEATURE - Acetyl attached to Asp
  REGION 3..12: note = MISC_FEATURE - cycle formed
  SITE 5: note = MISC_FEATURE - Xaa is l-norleucine
  SITE 11: note = MISC_FEATURE - Xaa is d-leucine
  SITE 12: note = MISC_FEATURE - NH2 attached to Cys
DLCRXYFPAIXC

SEQ ID NO: 13 - protein, 10 aa, synthetic construct
  REGION 1..10: note = synthetic
  SITE 1: note = MISC_FEATURE - pentanoic acid attached to Cys
  REGION 1..10: note = MISC_FEATURE - cycle formed
  SITE 2: note = MISC_FEATURE - Xaa is l-Citrulline
  SITE 3: note = MISC_FEATURE - Xaa is l-lysine DOTA conjugate
  SITE 4: note = MISC_FEATURE - Xaa is 3-pyridyl-alanine
  SITE 7: note = MISC_FEATURE - Xaa is 4-(R)-hydroxy-l-proline
  SITE 9: note = MISC_FEATURE - Xaa is l-norvaline
  SITE 10: note = MISC_FEATURE - NH2 attached to Cys
CXXXFPXIXC

SEQ ID NO: 14 - protein, 10 aa, synthetic construct
  REGION 1..10: note = synthetic
  SITE 1: note = MISC_FEATURE - butyric acid attached to Cys
  REGION 1..10: note = MISC_FEATURE - cycle formed
  SITE 2: note = MISC_FEATURE - Xaa is l-Citrulline
  SITE 7: note = MISC_FEATURE - Xaa is d-alanine
  SITE 10: note = MISC_FEATURE - NH2 attached to Cys
CXQYFPXILC

SEQ ID NO: 15 - protein, 12 aa, synthetic construct
  REGION 1..12: note = synthetic
  SITE 1: note = MISC_FEATURE - hexanoic acid attached to l-lysine DOTA conjugate
  SITE 1: note = MISC_FEATURE - Xaa is l-lysine DOTA conjugate
  REGION 3..12: note = MISC_FEATURE - cycle formed
  SITE 12: note = MISC_FEATURE - NH2 attached to Cys
XLCRMYFPAILC

SEQ ID NO: 16 - protein, 11 aa, synthetic construct
  REGION 1..11: note = synthetic
  SITE 1: note = MISC_FEATURE - n-butyloxycarbonyl attached to Cys
  REGION 1..10: note = MISC_FEATURE - cycle formed
  SITE 3: note = MISC_FEATURE - Xaa is l-lysine DOTA conjugate
  SITE 6: note = MISC_FEATURE - Xaa is (2S,4S)-4-fluoro-pyrrolidine-2-carboxylic acid
  SITE 7: note = MISC_FEATURE - Xaa is 4-(R)-hydroxy-l-proline
  SITE 9: note = MISC_FEATURE - Xaa is l-norvaline
  SITE 11: note = MISC_FEATURE - NH2 attached to Asp
CTXYFXXIXCD

SEQ ID NO: 17 - protein, 11 aa, synthetic construct
  REGION 1..11: note = synthetic
  SITE 1: note = MISC_FEATURE - 2,2 ,2 ,2 -(1,4,7,10-Tetraazacyclododecane-1,4,7,10-tetrayl)tetraacetic acid attached to Leu
  SITE 2: note = MISC_FEATURE - Xaa is N-methyl-l-cysteine
  REGION 2..11: note = MISC_FEATURE - cycle formed
  SITE 3: note = MISC_FEATURE - Xaa is l-Citrulline
  SITE 8: note = MISC_FEATURE - Xaa is 4-(R)-hydroxy-l-proline
  SITE 10: note = MISC_FEATURE - Xaa is l-norvaline
  SITE 11: note = MISC_FEATURE - NH2 attached to Cys
LXXQYFPXIXC

SEQ ID NO: 18 - protein, 12 aa, synthetic construct
  REGION 1..12: note = synthetic
  SITE 1: note = MISC_FEATURE - hexanoic acid attached to Thr
  REGION 3..12: note = MISC_FEATURE - cycle formed
  SITE 12: note = MISC_FEATURE - NH2 attached to Cys
TLCEYYFPAILC

SEQ ID NO: 19 - protein, 10 aa, synthetic construct
  REGION 1..10: note = synthetic
  SITE 1: note = MISC_FEATURE - isocaproic acid attached to Cys
  REGION 1..10: note = MISC_FEATURE - cycle formed
  SITE 2: note = MISC_FEATURE - Xaa is l-Citrulline
  SITE 4: note = MISC_FEATURE - Xaa is Levodopa / l-3,4-dihydroxyphenylalanine
  SITE 7: note = MISC_FEATURE - Xaa is d-alanine
  SITE 10: note = MISC_FEATURE - NH2 attached to Cys
CXQXFPXILC

SEQ ID NO: 20 - protein, 10 aa, synthetic construct
  REGION 1..10: note = synthetic
  SITE 1: note = MISC_FEATURE - isocaproic acid attached to Cys
  REGION 1..10: note = MISC_FEATURE - cycle formed
  SITE 2: note = MISC_FEATURE - Xaa is l-Citrulline
  SITE 7: note = MISC_FEATURE - Xaa is l-lysine DOTA conjugate
  SITE 10: note = MISC_FEATURE - NH2 attached to Cys
CXQYFPXILC

SEQ ID NO: 21 - protein, 10 aa, synthetic construct
  REGION 1..10: note = synthetic
  SITE 1: note = MISC_FEATURE - pentanoic acid attached to Cys
  REGION 1..10: note = MISC_FEATURE - cycle formed
  SITE 2: note = MISC_FEATURE - Xaa is l-Citrulline
  SITE 7: note = MISC_FEATURE - Xaa is 4-(R)-hydroxy-l-proline
  SITE 9: note = MISC_FEATURE - Xaa is l-norvaline
  SITE 10: note = MISC_FEATURE - n-ethylamine at C-terminus attached to Cys
CXQYFPXIXC

SEQ ID NO: 22 - protein, 10 aa, synthetic construct
  REGION 1..10: note = synthetic
  SITE 1: note = MISC_FEATURE - isocaproic acid attached to Cys
  REGION 1..10: note = MISC_FEATURE - cycle formed
  SITE 2: note = MISC_FEATURE - Xaa is l-Citrulline
  SITE 5: note = MISC_FEATURE - Xaa is 3-(2-naphthyl)-l-alanine
  SITE 7: note = MISC_FEATURE - Xaa is d-alanine
  SITE 10: note = MISC_FEATURE - NH2 attached to Cys
CXQYXPXILC

SEQ ID NO: 23 - protein, 10 aa, synthetic construct
  REGION 1..10: note = synthetic
  SITE 1: note = MISC_FEATURE - isocaproic acid attached to Cys
  REGION 1..10: note = MISC_FEATURE - cycle formed
  SITE 3: note = MISC_FEATURE - Xaa is l-lysine In(III) DOTA conjugate
  SITE 7: note = MISC_FEATURE - Xaa is d-alanine
  SITE 10: note = MISC_FEATURE - NH2 attached to Cys
CRXYFPXILC

SEQ ID NO: 24 - protein, 10 aa, synthetic construct
  REGION 1..10: note = synthetic
  SITE 1: note = MISC_FEATURE - pentanoic acid attached to Cys
  REGION 1..10: note = MISC_FEATURE - cycle formed
  SITE 2: note = MISC_FEATURE - Xaa is l-Citrulline
  SITE 3: note = MISC_FEATURE - Xaa is l-lysine DOTA conjugate
  SITE 4: note = MISC_FEATURE - Xaa is l-4-guanidino-phenylalanine
  SITE 7: note = MISC_FEATURE - Xaa is 4-(R)-hydroxy-l-proline
  SITE 9: note = MISC_FEATURE - Xaa is l-norvaline
  SITE 10: note = MISC_FEATURE - NH2 attached to Cys
CXXXFPXIXC

SEQ ID NO: 25 - protein, 14 aa, synthetic construct
  REGION 1..14: note = synthetic
  SITE 1: note = MISC_FEATURE - hexanoic acid attached to Asp
  REGION 3..12: note = MISC_FEATURE - cycle formed
  SITE 13: note = MISC_FEATURE - Xaa is 1,13-diamino-4,7,10-trioxatridecan-succinamic acid
  SITE 14: note = MISC_FEATURE - NH2 attached to l-lysine DOTA conjugate
  SITE 14: note = MISC_FEATURE - Xaa is l-lysine DOTA conjugate
DLCRMYFPAILCXX

SEQ ID NO: 26 - protein, 10 aa, synthetic construct
  REGION 1..10: note = synthetic
  SITE 1: note = MISC_FEATURE - pentanoic acid attached to Cys
  REGION 1..10: note = MISC_FEATURE - cycle formed
  SITE 2: note = MISC_FEATURE - Xaa is l-Citrulline
  SITE 3: note = MISC_FEATURE - Xaa is l-lysine Lu(III) DOTA conjugate
  SITE 7: note = MISC_FEATURE - Xaa is N-methyl-d-alanine
  SITE 9: note = MISC_FEATURE - Xaa is l-norvaline
  SITE 10: note = MISC_FEATURE - NH2 attached to Cys
CXXYFPXIXC

SEQ ID NO: 27 - protein, 10 aa, synthetic construct
  REGION 1..10: note = synthetic
  SITE 1: note = MISC_FEATURE - isocaproic acid attached to Cys
  REGION 1..10: note = MISC_FEATURE - cycle formed
  SITE 7: note = MISC_FEATURE - Xaa is 4-aminopiperidine-4-carboxylic acid DOTA conjugate
  SITE 10: note = MISC_FEATURE - NH2 attached to Cys
CRQYFPXILC

SEQ ID NO: 28 - protein, 10 aa, synthetic construct
  REGION 1..10: note = synthetic
  SITE 1: note = MISC_FEATURE - pentanoic acid attached to Cys
  REGION 1..10: note = MISC_FEATURE - cycle formed
  SITE 2: note = MISC_FEATURE - Xaa is N ,N ,N -trimethyl-l-lysine
  SITE 3: note = MISC_FEATURE - Xaa is l-lysine DOTA conjugate
  SITE 7: note = MISC_FEATURE - Xaa is 4-(R)-hydroxy-l-proline
  SITE 9: note = MISC_FEATURE - Xaa is l-norvaline
  SITE 10: note = MISC_FEATURE - NH2 attached to Cys
CXXYFPXIXC

SEQ ID NO: 29 - protein, 10 aa, synthetic construct
  REGION 1..10: note = synthetic
  SITE 1: note = MISC_FEATURE - pentanoic acid attached to Cys
  REGION 1..10: note = MISC_FEATURE - cycle formed
  SITE 9: note = MISC_FEATURE - Xaa is l-norvaline
  SITE 10: note = MISC_FEATURE - NH2 attached to Cys
CRQYFPSIXC

SEQ ID NO: 30 - protein, 10 aa, synthetic construct
  REGION 1..10: note = synthetic
  SITE 1: note = MISC_FEATURE - n-butyloxycarbonyl attached to Cys
  REGION 1..10: note = MISC_FEATURE - cycle formed
  SITE 2: note = MISC_FEATURE - Xaa is l-Citrulline
  SITE 7: note = MISC_FEATURE - Xaa is d-alanine
  SITE 10: note = MISC_FEATURE - NH2 attached to Cys
CXQYFPXILC

SEQ ID NO: 31 - protein, 10 aa, synthetic construct
  REGION 1..10: note = synthetic
  SITE 1: note = MISC_FEATURE - pentanoic acid attached to Cys
  REGION 1..10: note = MISC_FEATURE - cycle formed
  SITE 7: note = MISC_FEATURE - Xaa is 4-(R)-hydroxy-l-proline
  SITE 9: note = MISC_FEATURE - Xaa is -methyl-l-leucine
  SITE 10: note = MISC_FEATURE - NH2 attached to Cys
CRQYFPXIXC

SEQ ID NO: 32 - protein, 10 aa, synthetic construct
  REGION 1..10: note = synthetic
  SITE 1: note = MISC_FEATURE - isocaproic acid attached to Cys
  REGION 1..10: note = MISC_FEATURE - cycle formed
  SITE 2: note = MISC_FEATURE - Xaa is l-lysine DOTA conjugate
  SITE 7: note = MISC_FEATURE - Xaa is d-alanine
  SITE 10: note = MISC_FEATURE - NH2 attached to Cys
CXQYFPXILC

SEQ ID NO: 33 - protein, 10 aa, synthetic construct
  REGION 1..10: note = synthetic
  SITE 1: note = MISC_FEATURE - isocaproic acid attached to Cys
  REGION 1..10: note = MISC_FEATURE - cycle formed
  SITE 2: note = MISC_FEATURE - Xaa is l-Citrulline
  SITE 7: note = MISC_FEATURE - Xaa is d-alanine
  SITE 10: note = MISC_FEATURE - NH2 attached to Cys
CXQAFPXILC

SEQ ID NO: 34 - protein, 10 aa, synthetic construct
  REGION 1..10: note = synthetic
  SITE 1: note = MISC_FEATURE - isocaproic acid attached to Cys
  REGION 1..10: note = MISC_FEATURE - cycle formed
  SITE 2: note = MISC_FEATURE - Xaa is l-Citrulline
  SITE 7: note = MISC_FEATURE - Xaa is d-alanine
  SITE 10: note = MISC_FEATURE - NH2 attached to Cys
CXRYFPXILC

SEQ ID NO: 35 - protein, 10 aa, synthetic construct
  REGION 1..10: note = synthetic
  SITE 1: note = MISC_FEATURE - pentanoic acid attached to Cys
  REGION 1..10: note = MISC_FEATURE - cycle formed
  SITE 7: note = MISC_FEATURE - Xaa is d-aspartic acid
  SITE 9: note = MISC_FEATURE - Xaa is l-norvaline
  SITE 10: note = MISC_FEATURE - NH2 attached to Cys
CRQYFPXIXC

SEQ ID NO: 36 - protein, 11 aa, synthetic construct
  REGION 1..11: note = synthetic
  SITE 1: note = MISC_FEATURE - Acetyl attached to Leu
  REGION 2..11: note = MISC_FEATURE - cycle formed
  SITE 4: note = MISC_FEATURE - Xaa is l-lysine DOTA conjugate
  SITE 8: note = MISC_FEATURE - Xaa is d-alanine
  SITE 11: note = MISC_FEATURE - NH2 attached to Cys
LCRXYFPXILC

SEQ ID NO: 37 - protein, 10 aa, synthetic construct
  REGION 1..10: note = synthetic
  SITE 1: note = MISC_FEATURE - isocaproic acid attached to Cys
  REGION 1..10: note = MISC_FEATURE - cycle formed
  SITE 2: note = MISC_FEATURE - Xaa is l-Citrulline
  SITE 6: note = MISC_FEATURE - Xaa is (2S,4R)-4-amino-1-pyrrolidin-2-carboxylic acid
  SITE 7: note = MISC_FEATURE - Xaa is d-alanine
  SITE 10: note = MISC_FEATURE - NH2 attached to Cys
CXQYFXXILC

SEQ ID NO: 38 - protein, 10 aa, synthetic construct
  REGION 1..10: note = synthetic
  SITE 1: note = MISC_FEATURE - isocaproic acid attached to Cys
  REGION 1..10: note = MISC_FEATURE - cycle formed
  SITE 2: note = MISC_FEATURE - Xaa is l-Citrulline
  SITE 7: note = MISC_FEATURE - Xaa is d-alanine
  SITE 10: note = MISC_FEATURE - NH2 attached to Cys
CXQYFPXALC

SEQ ID NO: 39 - protein, 10 aa, synthetic construct
  REGION 1..10: note = synthetic
  SITE 1: note = MISC_FEATURE - n-butyloxycarbonyl attached to Cys
  REGION 1..10: note = MISC_FEATURE - cycle formed
  SITE 3: note = MISC_FEATURE - Xaa is l-lysine DOTA conjugate
  SITE 4: note = MISC_FEATURE - Xaa is 3-pyridyl-alanine
  SITE 6: note = MISC_FEATURE - Xaa is (2S,4S)-4-fluoro-pyrrolidine-2-carboxylic acid
  SITE 7: note = MISC_FEATURE - Xaa is 4-(R)-hydroxy-l-proline
  SITE 9: note = MISC_FEATURE - Xaa is l-norvaline
  SITE 10: note = MISC_FEATURE - NH2 attached to Cys
CTXXFXXIXC

SEQ ID NO: 40 - protein, 10 aa, synthetic construct
  REGION 1..10: note = synthetic
  SITE 1: note = MISC_FEATURE - pentanoic acid attached to Cys
  REGION 1..10: note = MISC_FEATURE - cycle formed
  SITE 2: note = MISC_FEATURE - Xaa is l-Citrulline
  SITE 3: note = MISC_FEATURE - Xaa is l-lysine La(III) DOTA conjugate
  SITE 5: note = MISC_FEATURE - Xaa is l-thienylalanine
  SITE 7: note = MISC_FEATURE - Xaa is 4-(R)-hydroxy-l-proline
  SITE 9: note = MISC_FEATURE - Xaa is l-norvaline
  SITE 10: note = MISC_FEATURE - NH2 attached to Cys
CXXYXPXIXC

SEQ ID NO: 41 - protein, 10 aa, synthetic construct
  REGION 1..10: note = synthetic
  SITE 1: note = MISC_FEATURE - isocaproic acid attached to Cys
  REGION 1..10: note = MISC_FEATURE - cycle formed
  SITE 2: note = MISC_FEATURE - Xaa is l-homoarginine
  SITE 7: note = MISC_FEATURE - Xaa is 4-(R)-hydroxy-l-proline
  SITE 10: note = MISC_FEATURE - NH2 attached to Cys
CXQYFPXILC

SEQ ID NO: 42 - protein, 10 aa, synthetic construct
  REGION 1..10: note = synthetic
  SITE 1: note = MISC_FEATURE - isocaproic acid attached to Cys
  REGION 1..10: note = MISC_FEATURE - cycle formed
  SITE 7: note = MISC_FEATURE - Xaa is d-alanine
  SITE 10: note = MISC_FEATURE - NH2 attached to Cys
CAQYFPXILC

SEQ ID NO: 43 - skipped

SEQ ID NO: 44 - protein, 12 aa, synthetic construct
  REGION 1..12: note = synthetic
  SITE 1: note = MISC_FEATURE - Lu(III) DOTA complex attached to 6-aminohexanoic acid
  SITE 1: note = MISC_FEATURE - Xaa is 6-aminohexanoic acid
  REGION 3..12: note = MISC_FEATURE - cycle formed
  SITE 9: note = MISC_FEATURE - Xaa is d-alanine
  SITE 12: note = MISC_FEATURE - NH2 attached to Cys
XLCRQYFPXILC

SEQ ID NO: 45 - protein, 10 aa, synthetic construct
  REGION 1..10: note = synthetic
  SITE 1: note = MISC_FEATURE - pentanoic acid attached to Cys
  REGION 1..10: note = MISC_FEATURE - cycle formed
  SITE 7: note = MISC_FEATURE - Xaa is 4-(R)-hydroxy-l-proline
  SITE 10: note = MISC_FEATURE - NH2 attached to Cys
CRQYFPXIFC

SEQ ID NO: 46 - protein, 10 aa, synthetic construct
  REGION 1..10: note = synthetic
  SITE 1: note = MISC_FEATURE - 3-ethoxypropanoic acid attached to Cys
  REGION 1..10: note = MISC_FEATURE - cycle formed
  SITE 2: note = MISC_FEATURE - Xaa is l-Citrulline
  SITE 7: note = MISC_FEATURE - Xaa is d-alanine
  SITE 10: note = MISC_FEATURE - NH2 attached to Cys
CXQYFPXILC

SEQ ID NO: 47 - protein, 10 aa, synthetic construct
  REGION 1..10: note = synthetic
  SITE 1: note = MISC_FEATURE - pentanoic acid attached to Cys
  REGION 1..10: note = MISC_FEATURE - cycle formed
  SITE 2: note = MISC_FEATURE - Xaa is l-Citrulline
  SITE 3: note = MISC_FEATURE - Xaa is l-lysine DOTA conjugate
  SITE 7: note = MISC_FEATURE - Xaa is N -methyl-l-lysine
  SITE 9: note = MISC_FEATURE - Xaa is l-norvaline
  SITE 10: note = MISC_FEATURE - NH2 attached to Cys
CXXYFPXIXC

SEQ ID NO: 48 - protein, 10 aa, synthetic construct
  REGION 1..10: note = synthetic
  SITE 1: note = MISC_FEATURE - isocaproic acid attached to Cys
  REGION 1..10: note = MISC_FEATURE - cycle formed
  SITE 2: note = MISC_FEATURE - Xaa is l-Citrulline
  SITE 7: note = MISC_FEATURE - Xaa is 4-(R)-hydroxy-l-proline
  SITE 10: note = MISC_FEATURE - NH2 attached to Cys
CXQYFPXILC

SEQ ID NO: 49 - protein, 10 aa, synthetic construct
  REGION 1..10: note = synthetic
  SITE 1: note = MISC_FEATURE - isocaproic acid attached to Cys
  REGION 1..10: note = MISC_FEATURE - cycle formed
  SITE 3: note = MISC_FEATURE - Xaa is l-lysine DOTA conjugate
  SITE 7: note = MISC_FEATURE - Xaa is d-alanine
  SITE 10: note = MISC_FEATURE - NH2 attached to Cys
CRXYFPXILC

SEQ ID NO: 50 - protein, 10 aa, synthetic construct
  REGION 1..10: note = synthetic
  SITE 1: note = MISC_FEATURE - pentanoic acid attached to Cys
  REGION 1..10: note = MISC_FEATURE - cycle formed
  SITE 2: note = MISC_FEATURE - Xaa is l-Citrulline
  SITE 3: note = MISC_FEATURE - Xaa is l-lysine DOTA conjugate
  SITE 7: note = MISC_FEATURE - Xaa is N-methyl-glycine
  SITE 9: note = MISC_FEATURE - Xaa is l-norvaline
  SITE 10: note = MISC_FEATURE - NH2 attached to Cys
CXXYFPXIXC

SEQ ID NO: 51 - protein, 10 aa, synthetic construct
  REGION 1..10: note = synthetic
  SITE 1: note = MISC_FEATURE - isocaproic acid attached to Cys
  REGION 1..10: note = MISC_FEATURE - cycle formed
  SITE 2: note = MISC_FEATURE - Xaa is l-Citrulline
  SITE 6: note = MISC_FEATURE - Xaa is 4-(R)-Fluoro-l-proline
  SITE 7: note = MISC_FEATURE - Xaa is d-alanine
  SITE 10: note = MISC_FEATURE - NH2 attached to Cys
CXQYFXXILC

SEQ ID NO: 52 - protein, 10 aa, synthetic construct
  REGION 1..10: note = synthetic
  SITE 1: note = MISC_FEATURE - pentanoic acid attached to Cys
  REGION 1..10: note = MISC_FEATURE - cycle formed
  SITE 7: note = MISC_FEATURE - Xaa is 4-(R)-hydroxy-l-proline
  SITE 8: note = MISC_FEATURE - Xaa is diethylgylcine
  SITE 9: note = MISC_FEATURE - Xaa is l-norvaline
  SITE 10: note = MISC_FEATURE - NH2 attached to Cys
CRQYFPXXXC

SEQ ID NO: 53 - protein, 10 aa, synthetic construct
  REGION 1..10: note = synthetic
  SITE 1: note = MISC_FEATURE - isocaproic acid attached to Cys
  REGION 1..10: note = MISC_FEATURE - cycle formed
  SITE 2: note = MISC_FEATURE - Xaa is l-Citrulline
  SITE 5: note = MISC_FEATURE - Xaa is l-homophenylalanine
  SITE 7: note = MISC_FEATURE - Xaa is d-alanine
  SITE 10: note = MISC_FEATURE - NH2 attached to Cys
CXQYXPXILC

SEQ ID NO: 54 - protein, 10 aa, synthetic construct
  REGION 1..10: note = synthetic
  SITE 1: note = MISC_FEATURE - n-butyloxycarbonyl attached to Cys
  REGION 1..10: note = MISC_FEATURE - cycle formed
  SITE 3: note = MISC_FEATURE - Xaa is l-lysine PPAc DOTA conjugate
  SITE 6: note = MISC_FEATURE - Xaa is (2S,4S)-4-fluoro-pyrrolidine-2-carboxylic acid
  SITE 7: note = MISC_FEATURE - Xaa is 4-(R)-hydroxy-l-proline
  SITE 9: note = MISC_FEATURE - Xaa is l-norvaline
  SITE 10: note = MISC_FEATURE - NH2 attached to Cys
CTXYFXXIXC

SEQ ID NO: 55 - protein, 10 aa, synthetic construct
  REGION 1..10: note = synthetic
  SITE 1: note = MISC_FEATURE - pentanoic acid attached to Cys
  REGION 1..10: note = MISC_FEATURE - cycle formed
  SITE 2: note = MISC_FEATURE - Xaa is l-Citrulline
  SITE 3: note = MISC_FEATURE - Xaa is l-lysine In(III) DOTA conjugate
  SITE 7: note = MISC_FEATURE - Xaa is 4-(R)-hydroxy-l-proline
  SITE 9: note = MISC_FEATURE - Xaa is l-norvaline
  SITE 10: note = MISC_FEATURE - NH2 attached to Cys
CXXYFPXIXC

SEQ ID NO: 56 - protein, 10 aa, synthetic construct
  REGION 1..10: note = synthetic
  SITE 1: note = MISC_FEATURE - pentanoic acid attached to Cys
  REGION 1..10: note = MISC_FEATURE - cycle formed
  SITE 2: note = MISC_FEATURE - Xaa is N ,N ,N -trimethyl-l-lysine
  SITE 3: note = MISC_FEATURE - Xaa is l-lysine La(III) DOTA conjugate
  SITE 7: note = MISC_FEATURE - Xaa is 4-(R)-hydroxy-l-proline
  SITE 9: note = MISC_FEATURE - Xaa is l-norvaline
  SITE 10: note = MISC_FEATURE - NH2 attached to Cys
CXXYFPXIXC

SEQ ID NO: 57 - protein, 10 aa, synthetic construct
  REGION 1..10: note = synthetic
  SITE 1: note = MISC_FEATURE - isocaproic acid attached to Cys
  REGION 1..10: note = MISC_FEATURE - cycle formed
  SITE 2: note = MISC_FEATURE - Xaa is l-Citrulline
  SITE 7: note = MISC_FEATURE - Xaa is d-alanine
  SITE 10: note = MISC_FEATURE - NH2 attached to Cys
CXQYFPXIVC

SEQ ID NO: 58 - protein, 10 aa, synthetic construct
  REGION 1..10: note = synthetic
  SITE 1: note = MISC_FEATURE - pentanoic acid attached to Cys
  REGION 1..10: note = MISC_FEATURE - cycle formed
  SITE 2: note = MISC_FEATURE - Xaa is 4-aminopiperidine-4-carboxylic acid
  SITE 7: note = MISC_FEATURE - Xaa is 4-(R)-hydroxy-l-proline
  SITE 9: note = MISC_FEATURE - Xaa is l-norvaline
  SITE 10: note = MISC_FEATURE - NH2 attached to Cys
CXQYFPXIXC

SEQ ID NO: 59 - protein, 10 aa, synthetic construct
  REGION 1..10: note = synthetic
  SITE 1: note = MISC_FEATURE - isocaproic acid attached to Cys
  REGION 1..10: note = MISC_FEATURE - cycle formed
  SITE 2: note = MISC_FEATURE - Xaa is l-Citrulline
  SITE 7: note = MISC_FEATURE - Xaa is d-alanine
  SITE 8: note = MISC_FEATURE - Xaa is l-cyclopropyl glycine
  SITE 10: note = MISC_FEATURE - NH2 attached to Cys
CXQYFPXXLC

SEQ ID NO: 60 - protein, 10 aa, synthetic construct
  REGION 1..10: note = synthetic
  SITE 1: note = MISC_FEATURE - isocaproic acid attached to Cys
  REGION 1..10: note = MISC_FEATURE - cycle formed
  SITE 2: note = MISC_FEATURE - Xaa is l-Citrulline
  SITE 4: note = MISC_FEATURE - Xaa is l-3-chloro tyrosine
  SITE 7: note = MISC_FEATURE - Xaa is d-alanine
  SITE 10: note = MISC_FEATURE - NH2 attached to Cys
CXQXFPXILC

SEQ ID NO: 61 - protein, 12 aa, synthetic construct
  REGION 1..12: note = synthetic
  SITE 1: note = MISC_FEATURE - Acetyl attached to Asp
  REGION 3..12: note = MISC_FEATURE - cycle formed
  SITE 4: note = MISC_FEATURE - Xaa is l-Citrulline
  SITE 5: note = MISC_FEATURE - Xaa is l-lysine DOTA conjugate
  SITE 9: note = MISC_FEATURE - Xaa is d-alanine
  SITE 12: note = MISC_FEATURE - NH2 attached to Cys
DLCXXYFPXILC

SEQ ID NO: 62 - protein, 10 aa, synthetic construct
  REGION 1..10: note = synthetic
  SITE 1: note = MISC_FEATURE - pentanoic acid attached to Cys
  REGION 1..10: note = MISC_FEATURE - cycle formed
  SITE 7: note = MISC_FEATURE - Xaa is (2S,3aS,7aS)- octahydroindolecarboxylic acid
  SITE 9: note = MISC_FEATURE - Xaa is l-norvaline
  SITE 10: note = MISC_FEATURE - NH2 attached to Cys
CRQYFPXIXC

SEQ ID NO: 63 - protein, 10 aa, synthetic construct
  REGION 1..10: note = synthetic
  SITE 1: note = MISC_FEATURE - n-butyloxycarbonyl attached to Cys
  REGION 1..10: note = MISC_FEATURE - cycle formed
  SITE 3: note = MISC_FEATURE - Xaa is l-lysine In(III) DOTA conjugate
  SITE 4: note = MISC_FEATURE - Xaa is Levodopa / l-3,4-dihydroxyphenylalanine
  SITE 6: note = MISC_FEATURE - Xaa is (2S,4S)-4-fluoro-pyrrolidine-2-carboxylic acid
  SITE 7: note = MISC_FEATURE - Xaa is 4-(R)-hydroxy-l-proline
  SITE 9: note = MISC_FEATURE - Xaa is l-norvaline
  SITE 10: note = MISC_FEATURE - NH2 attached to Cys
CTXXFXXIXC

SEQ ID NO: 64 - protein, 10 aa, synthetic construct
  REGION 1..10: note = synthetic
  SITE 1: note = MISC_FEATURE - n-butyloxycarbonyl attached to Cys
  REGION 1..10: note = MISC_FEATURE - cycle formed
  SITE 3: note = MISC_FEATURE - Xaa is l-ornithine DOTA conjugate
  SITE 6: note = MISC_FEATURE - Xaa is (2S,4S)-4-fluoro-pyrrolidine-2-carboxylic acid
  SITE 7: note = MISC_FEATURE - Xaa is 4-(R)-hydroxy-l-proline
  SITE 9: note = MISC_FEATURE - Xaa is l-norvaline
  SITE 10: note = MISC_FEATURE - NH2 attached to Cys
CTXYFXXIXC

SEQ ID NO: 65 - protein, 10 aa, synthetic construct
  REGION 1..10: note = synthetic
  SITE 1: note = MISC_FEATURE - octanoic acid attached to Cys
  REGION 1..10: note = MISC_FEATURE - cycle formed
  SITE 7: note = MISC_FEATURE - Xaa is 4-(R)-hydroxy-l-proline
  SITE 9: note = MISC_FEATURE - Xaa is l-norvaline
  SITE 10: note = MISC_FEATURE - NH2 attached to Cys
CRQYFPXIXC

SEQ ID NO: 66 - protein, 10 aa, synthetic construct
  REGION 1..10: note = synthetic
  SITE 1: note = MISC_FEATURE - n-butyloxycarbonyl attached to Cys
  REGION 1..10: note = MISC_FEATURE - cycle formed
  SITE 3: note = MISC_FEATURE - Xaa is l-lysine Kzw DOTA conjugate
  SITE 4: note = MISC_FEATURE - Xaa is Levodopa / l-3,4-dihydroxyphenylalanine
  SITE 6: note = MISC_FEATURE - Xaa is (2S,4S)-4-fluoro-pyrrolidine-2-carboxylic acid
  SITE 7: note = MISC_FEATURE - Xaa is 4-(R)-hydroxy-l-proline
  SITE 9: note = MISC_FEATURE - Xaa is l-norvaline
  SITE 10: note = MISC_FEATURE - NH2 attached to Cys
CTXXFXXIXC

SEQ ID NO: 67 - protein, 10 aa, synthetic construct
  REGION 1..10: note = synthetic
  SITE 1: note = MISC_FEATURE - pentanoic acid attached to Cys
  REGION 1..10: note = MISC_FEATURE - cycle formed
  SITE 7: note = MISC_FEATURE - Xaa is 4-(R)-hydroxy-l-proline
  SITE 9: note = MISC_FEATURE - Xaa is l-norvaline
  SITE 10: note = MISC_FEATURE - NH2 attached to Cys
CRQLFPXIXC

SEQ ID NO: 68 - protein, 10 aa, synthetic construct
  REGION 1..10: note = synthetic
  SITE 1: note = MISC_FEATURE - pentanoic acid attached to Cys
  REGION 1..10: note = MISC_FEATURE - cycle formed
  SITE 4: note = MISC_FEATURE - Xaa is l-phenylglycine
  SITE 7: note = MISC_FEATURE - Xaa is 4-(R)-hydroxy-l-proline
  SITE 9: note = MISC_FEATURE - Xaa is l-norvaline
  SITE 10: note = MISC_FEATURE - NH2 attached to Cys
CRQXFPXIXC

SEQ ID NO: 69 - protein, 10 aa, synthetic construct
  REGION 1..10: note = synthetic
  SITE 1: note = MISC_FEATURE - pentanoic acid attached to Cys
  REGION 1..10: note = MISC_FEATURE - cycle formed
  SITE 7: note = MISC_FEATURE - Xaa is 4-(R)-hydroxy-l-proline
  SITE 9: note = MISC_FEATURE - Xaa is l-norvaline
  SITE 10: note = MISC_FEATURE - NH2 attached to Cys
CRQYLPXIXC

SEQ ID NO: 70 - protein, 12 aa, synthetic construct
  REGION 1..12: note = synthetic
  SITE 1: note = MISC_FEATURE - Acetyl attached to Asp
  REGION 3..12: note = MISC_FEATURE - cycle formed
  SITE 5: note = MISC_FEATURE - Xaa is l-norleucine
  SITE 6: note = MISC_FEATURE - Xaa is d-tyrosine
  SITE 12: note = MISC_FEATURE - NH2 attached to Cys
DLCRXXFPAILC

SEQ ID NO: 71 - protein, 10 aa, synthetic construct
  REGION 1..10: note = synthetic
  SITE 1: note = MISC_FEATURE - n-butyloxycarbonyl attached to Cys
  REGION 1..10: note = MISC_FEATURE - cycle formed
  SITE 3: note = MISC_FEATURE - Xaa is l-lysine PPAc DOTA conjugate
  SITE 4: note = MISC_FEATURE - Xaa is Levodopa / l-3,4-dihydroxyphenylalanine
  SITE 6: note = MISC_FEATURE - Xaa is (2S,4S)-4-fluoro-pyrrolidine-2-carboxylic acid
  SITE 7: note = MISC_FEATURE - Xaa is 4-(R)-hydroxy-l-proline
  SITE 9: note = MISC_FEATURE - Xaa is l-norvaline
  SITE 10: note = MISC_FEATURE - NH2 attached to Cys
CTXXFXXIXC

SEQ ID NO: 72 - protein, 10 aa, synthetic construct
  REGION 1..10: note = synthetic
  SITE 1: note = MISC_FEATURE - pentanoic acid attached to Cys
  REGION 1..10: note = MISC_FEATURE - cycle formed
  SITE 2: note = MISC_FEATURE - Xaa is l-Citrulline
  SITE 3: note = MISC_FEATURE - Xaa is l-lysine PEG12 DOTA conjugate
  SITE 7: note = MISC_FEATURE - Xaa is 4-(R)-hydroxy-l-proline
  SITE 9: note = MISC_FEATURE - Xaa is l-norvaline
  SITE 10: note = MISC_FEATURE - NH2 attached to Cys
CXXYFPXIXC

SEQ ID NO: 73 - protein, 10 aa, synthetic construct
  REGION 1..10: note = synthetic
  SITE 1: note = MISC_FEATURE - isocaproic acid attached to Cys
  REGION 1..10: note = MISC_FEATURE - cycle formed
  SITE 2: note = MISC_FEATURE - Xaa is l-Citrulline
  SITE 7: note = MISC_FEATURE - Xaa is d-alanine
  SITE 8: note = MISC_FEATURE - Xaa is l-tert-leucine
  SITE 10: note = MISC_FEATURE - NH2 attached to Cys
CXQYFPXXLC

SEQ ID NO: 74 - protein, 12 aa, synthetic construct
  REGION 1..12: note = synthetic
  SITE 1: note = MISC_FEATURE - hexanoic acid attached to Ser
  REGION 3..12: note = MISC_FEATURE - cycle formed
  SITE 12: note = MISC_FEATURE - NH2 attached to Cys
SLCDQFFPAILC

SEQ ID NO: 75 - protein, 10 aa, synthetic construct
  REGION 1..10: note = synthetic
  SITE 1: note = MISC_FEATURE - pentanoic acid attached to Cys
  REGION 1..10: note = MISC_FEATURE - cycle formed
  SITE 5: note = MISC_FEATURE - Xaa is l-phenylglycine
  SITE 7: note = MISC_FEATURE - Xaa is 4-(R)-hydroxy-l-proline
  SITE 9: note = MISC_FEATURE - Xaa is l-norvaline
  SITE 10: note = MISC_FEATURE - NH2 attached to Cys
CRQYXPXIXC

SEQ ID NO: 76 - protein, 10 aa, synthetic construct
  REGION 1..10: note = synthetic
  SITE 1: note = MISC_FEATURE - pentanoic acid attached to Cys
  REGION 1..10: note = MISC_FEATURE - cycle formed
  SITE 7: note = MISC_FEATURE - Xaa is 4-(R)-hydroxy-l-proline
  SITE 8: note = MISC_FEATURE - Xaa is 4-chloro-l-phenylalanine
  SITE 9: note = MISC_FEATURE - Xaa is l-norvaline
  SITE 10: note = MISC_FEATURE - NH2 attached to Cys
CRQYFPXXXC

SEQ ID NO: 77 - protein, 10 aa, synthetic construct
  REGION 1..10: note = synthetic
  SITE 1: note = MISC_FEATURE - pentanoic acid attached to Ala
  SITE 2: note = MISC_FEATURE - Xaa is l-Citrulline
  SITE 7: note = MISC_FEATURE - Xaa is 4-(R)-hydroxy-l-proline
  SITE 9: note = MISC_FEATURE - Xaa is l-norvaline
  SITE 10: note = MISC_FEATURE - NH2 attached to S-methyl-l-cysteine
  SITE 10: note = MISC_FEATURE - Xaa is S-methyl-l-cysteine
AXQYFPXIXX

SEQ ID NO: 78 - protein, 11 aa, synthetic construct
  REGION 1..11: note = synthetic
  SITE 1: note = MISC_FEATURE - pentanoic acid attached to Cys
  REGION 1..10: note = MISC_FEATURE - cycle formed
  SITE 2: note = MISC_FEATURE - Xaa is l-Citrulline
  SITE 7: note = MISC_FEATURE - Xaa is 4-(R)-hydroxy-l-proline
  SITE 9: note = MISC_FEATURE - Xaa is l-norvaline
  SITE 11: note = MISC_FEATURE - NH2 attached to Gly
CXQYFPXIXCG

SEQ ID NO: 79 - protein, 10 aa, synthetic construct
  REGION 1..10: note = synthetic
  SITE 1: note = MISC_FEATURE - pentanoic acid attached to Cys
  REGION 1..10: note = MISC_FEATURE - cycle formed
  SITE 2: note = MISC_FEATURE - Xaa is l-Citrulline
  SITE 3: note = MISC_FEATURE - Xaa is l-lysine DOTA conjugate
  SITE 5: note = MISC_FEATURE - Xaa is 3-pyridyl-alanine
  SITE 7: note = MISC_FEATURE - Xaa is 4-(R)-Fluoro-l-proline
  SITE 9: note = MISC_FEATURE - Xaa is l-norvaline
  SITE 10: note = MISC_FEATURE - NH2 attached to Cys
CXXYXPXIXC

SEQ ID NO: 80 - protein, 10 aa, synthetic construct
  REGION 1..10: note = synthetic
  SITE 1: note = MISC_FEATURE - Cyclopentane carboxylic acid attached to Cys
  REGION 1..10: note = MISC_FEATURE - cycle formed
  SITE 2: note = MISC_FEATURE - Xaa is l-Citrulline
  SITE 7: note = MISC_FEATURE - Xaa is d-alanine
  SITE 10: note = MISC_FEATURE - NH2 attached to Cys
CXQYFPXILC

SEQ ID NO: 81 - protein, 10 aa, synthetic construct
  REGION 1..10: note = synthetic
  SITE 1: note = MISC_FEATURE - pentanoic acid attached to Cys
  REGION 1..10: note = MISC_FEATURE - cycle formed
  SITE 2: note = MISC_FEATURE - Xaa is l-Citrulline
  SITE 3: note = MISC_FEATURE - Xaa is l-lysine DOTA conjugate
  SITE 4: note = MISC_FEATURE - Xaa is 4-sulfo phenylalanine
  SITE 7: note = MISC_FEATURE - Xaa is 4-(R)-hydroxy-l-proline
  SITE 9: note = MISC_FEATURE - Xaa is l-norvaline
  SITE 10: note = MISC_FEATURE - NH2 attached to Cys
CXXXFPXIXC

SEQ ID NO: 82 - protein, 10 aa, synthetic construct
  REGION 1..10: note = synthetic
  SITE 1: note = MISC_FEATURE - n-propyl-carbamoyl attached to Cys
  REGION 1..10: note = MISC_FEATURE - cycle formed
  SITE 2: note = MISC_FEATURE - Xaa is l-Citrulline
  SITE 3: note = MISC_FEATURE - Xaa is l-lysine DOTA conjugate
  SITE 7: note = MISC_FEATURE - Xaa is 4-(R)-hydroxy-l-proline
  SITE 9: note = MISC_FEATURE - Xaa is l-norvaline
  SITE 10: note = MISC_FEATURE - NH2 attached to Cys
CXXYFPXIXC

SEQ ID NO: 83 - protein, 10 aa, synthetic construct
  REGION 1..10: note = synthetic
  SITE 1: note = MISC_FEATURE - pentanoic acid attached to Cys
  REGION 1..10: note = MISC_FEATURE - cycle formed
  SITE 6: note = MISC_FEATURE - Xaa is N-methyl-d-alanine
  SITE 7: note = MISC_FEATURE - Xaa is 4-(R)-hydroxy-l-proline
  SITE 9: note = MISC_FEATURE - Xaa is l-norvaline
  SITE 10: note = MISC_FEATURE - NH2 attached to Cys
CRQYFXXIXC

SEQ ID NO: 84 - protein, 10 aa, synthetic construct
  REGION 1..10: note = synthetic
  SITE 1: note = MISC_FEATURE - 2-propoxyacetic acid attached to Cys
  REGION 1..10: note = MISC_FEATURE - cycle formed
  SITE 2: note = MISC_FEATURE - Xaa is l-Citrulline
  SITE 7: note = MISC_FEATURE - Xaa is d-alanine
  SITE 10: note = MISC_FEATURE - NH2 attached to Cys
CXQYFPXILC

SEQ ID NO: 85 - protein, 10 aa, synthetic construct
  REGION 1..10: note = synthetic
  SITE 1: note = MISC_FEATURE - pentanoic acid attached to Cys
  REGION 1..10: note = MISC_FEATURE - cycle formed
  SITE 7: note = MISC_FEATURE - Xaa is 4-(R)-hydroxy-l-proline
  SITE 9: note = MISC_FEATURE - Xaa is l-norvaline
  SITE 10: note = MISC_FEATURE - NH2 attached to l-homocysteine
  SITE 10: note = MISC_FEATURE - Xaa is l-homocysteine
CRQYFPXIXX

SEQ ID NO: 86 - protein, 10 aa, synthetic construct
  REGION 1..10: note = synthetic
  SITE 1: note = MISC_FEATURE - pentanoic acid attached to Cys
  REGION 1..10: note = MISC_FEATURE - cycle formed
  SITE 2: note = MISC_FEATURE - Xaa is l-Citrulline
  SITE 3: note = MISC_FEATURE - Xaa is l-lysine DOTA conjugate
  SITE 7: note = MISC_FEATURE - Xaa is 4-(S)-hydroxy-l-proline
  SITE 9: note = MISC_FEATURE - Xaa is l-norvaline
  SITE 10: note = MISC_FEATURE - NH2 attached to Cys
CXXYFPXIXC

SEQ ID NO: 87 - protein, 10 aa, synthetic construct
  REGION 1..10: note = synthetic
  SITE 1: note = MISC_FEATURE - pentanoic acid attached to l-cysteine bound to methylene (in thioacetal linkage)
  SITE 1: note = MISC_FEATURE - Xaa is l-cysteine bound to methylene (in thioacetal linkage)
  REGION 1..10: note = MISC_FEATURE - cycle formed
  SITE 2: note = MISC_FEATURE - Xaa is l-Citrulline
  SITE 7: note = MISC_FEATURE - Xaa is 4-(R)-hydroxy-l-proline
  SITE 9: note = MISC_FEATURE - Xaa is l-norvaline
  SITE 10: note = MISC_FEATURE - NH2 attached to Cys
XXQYFPXIXC

SEQ ID NO: 88 - protein, 12 aa, synthetic construct
  REGION 1..12: note = synthetic
  SITE 1: note = MISC_FEATURE - 2,2 ,2 ,2 -(1,4,7,10-Tetraazacyclododecane-1,4,7,10-tetrayl)tetraacetic acid attached to 8-amino-3,6-dioxaoctanoic acid
  SITE 1: note = MISC_FEATURE - Xaa is 8-amino-3,6-dioxaoctanoic acid
  REGION 3..12: note = MISC_FEATURE - cycle formed
  SITE 4: note = MISC_FEATURE - Xaa is d-alanine
  SITE 9: note = MISC_FEATURE - Xaa is d-alanine
  SITE 12: note = MISC_FEATURE - NH2 attached to Cys
XLCXQYFPXILC

SEQ ID NO: 89 - protein, 10 aa, synthetic construct
  REGION 1..10: note = synthetic
  SITE 1: note = MISC_FEATURE - pentanoic acid attached to Cys
  REGION 1..10: note = MISC_FEATURE - cycle formed
  SITE 2: note = MISC_FEATURE - Xaa is l-Citrulline
  SITE 7: note = MISC_FEATURE - Xaa is 4-(R)-hydroxy-l-proline
  SITE 9: note = MISC_FEATURE - Xaa is l-norvaline
  SITE 10: note = MISC_FEATURE - NH2 attached to l-penicillamine
  SITE 10: note = MISC_FEATURE - Xaa is l-penicillamine
CXQYFPXIXX

SEQ ID NO: 90 - protein, 12 aa, synthetic construct
  REGION 1..12: note = synthetic
  SITE 1: note = MISC_FEATURE - Acetyl attached to Asp
  REGION 3..12: note = MISC_FEATURE - cycle formed
  SITE 5: note = MISC_FEATURE - Xaa is l-norleucine
  SITE 8: note = MISC_FEATURE - Xaa is d-proline
  SITE 12: note = MISC_FEATURE - NH2 attached to Cys
DLCRXYFXAILC

SEQ ID NO: 91 - protein, 10 aa, synthetic construct
  REGION 1..10: note = synthetic
  SITE 1: note = MISC_FEATURE - isocaproic acid attached to Cys
  REGION 1..10: note = MISC_FEATURE - cycle formed
  SITE 2: note = MISC_FEATURE - Xaa is l-Citrulline
  SITE 7: note = MISC_FEATURE - Xaa is 4-aminopiperidine-4-carboxylic acid DOTA conjugate
  SITE 10: note = MISC_FEATURE - NH2 attached to Cys
CXQYFPXILC

SEQ ID NO: 92 - protein, 10 aa, synthetic construct
  REGION 1..10: note = synthetic
  SITE 1: note = MISC_FEATURE - isocaproic acid attached to Cys
  REGION 1..10: note = MISC_FEATURE - cycle formed
  SITE 2: note = MISC_FEATURE - Xaa is l-Citrulline
  SITE 7: note = MISC_FEATURE - Xaa is 4-(R)-Fluoro-l-proline
  SITE 10: note = MISC_FEATURE - NH2 attached to Cys
CXQYFPXILC

SEQ ID NO: 93 - protein, 10 aa, synthetic construct
  REGION 1..10: note = synthetic
  SITE 1: note = MISC_FEATURE - isocaproic acid attached to Cys
  REGION 1..10: note = MISC_FEATURE - cycle formed
  SITE 2: note = MISC_FEATURE - Xaa is l-Citrulline
  SITE 5: note = MISC_FEATURE - Xaa is ortho-chloro-l-phenylalanine
  SITE 7: note = MISC_FEATURE - Xaa is d-alanine
  SITE 10: note = MISC_FEATURE - NH2 attached to Cys
CXQYXPXILC

SEQ ID NO: 94 - protein, 10 aa, synthetic construct
  REGION 1..10: note = synthetic
  SITE 1: note = MISC_FEATURE - pentanoic acid attached to Cys
  REGION 1..10: note = MISC_FEATURE - cycle formed
  SITE 2: note = MISC_FEATURE - Xaa is l-Citrulline
  SITE 3: note = MISC_FEATURE - Xaa is l-lysine DOTA conjugate
  SITE 5: note = MISC_FEATURE - Xaa is (S)-4-pyridyl-alanine
  SITE 7: note = MISC_FEATURE - Xaa is 4-(R)-hydroxy-l-proline
  SITE 9: note = MISC_FEATURE - Xaa is l-norvaline
  SITE 10: note = MISC_FEATURE - NH2 attached to Cys
CXXYXPXIXC

SEQ ID NO: 95 - protein, 11 aa, synthetic construct
  REGION 1..11: note = synthetic
  SITE 1: note = MISC_FEATURE - 2,2 ,2 ,2 -(1,4,7,10-Tetraazacyclododecane-1,4,7,10-tetrayl)tetraacetic acid attached to Phe
  REGION 2..11: note = MISC_FEATURE - cycle formed
  SITE 8: note = MISC_FEATURE - Xaa is 4-(R)-hydroxy-l-proline
  SITE 10: note = MISC_FEATURE - Xaa is l-norvaline
  SITE 11: note = MISC_FEATURE - NH2 attached to Cys
FCRQYFPXIXC

SEQ ID NO: 96 - protein, 10 aa, synthetic construct
  REGION 1..10: note = synthetic
  SITE 1: note = MISC_FEATURE - pentanoic acid attached to Cys
  REGION 1..10: note = MISC_FEATURE - cycle formed
  SITE 2: note = MISC_FEATURE - Xaa is l-ornithine Tris-Nta(Tris) conjugate
  SITE 3: note = MISC_FEATURE - Xaa is l-lysine DOTA conjugate
  SITE 7: note = MISC_FEATURE - Xaa is 4-(R)-hydroxy-l-proline
  SITE 9: note = MISC_FEATURE - Xaa is l-norvaline
  SITE 10: note = MISC_FEATURE - NH2 attached to Cys
CXXYFPXIXC

SEQ ID NO: 97 - protein, 10 aa, synthetic construct
  REGION 1..10: note = synthetic
  SITE 1: note = MISC_FEATURE - isocaproic acid attached to Cys
  REGION 1..10: note = MISC_FEATURE - cycle formed
  SITE 2: note = MISC_FEATURE - Xaa is l-Citrulline
  SITE 7: note = MISC_FEATURE - Xaa is d-alanine
  SITE 8: note = MISC_FEATURE - Xaa is l-cyclohexyl-glycine
  SITE 10: note = MISC_FEATURE - NH2 attached to Cys
CXQYFPXXLC

SEQ ID NO: 98 - protein, 10 aa, synthetic construct
  REGION 1..10: note = synthetic
  SITE 1: note = MISC_FEATURE - pentanoic acid attached to Cys
  REGION 1..10: note = MISC_FEATURE - cycle formed
  SITE 9: note = MISC_FEATURE - Xaa is l-norvaline
  SITE 10: note = MISC_FEATURE - NH2 attached to Cys
CRQYFPYIXC

SEQ ID NO: 99 - protein, 10 aa, synthetic construct
  REGION 1..10: note = synthetic
  SITE 1: note = MISC_FEATURE - isocaproic acid attached to Cys
  REGION 1..10: note = MISC_FEATURE - cycle formed
  SITE 2: note = MISC_FEATURE - Xaa is l-Citrulline
  SITE 5: note = MISC_FEATURE - Xaa is 3-chloro-l-phenylalanine
  SITE 7: note = MISC_FEATURE - Xaa is d-alanine
  SITE 10: note = MISC_FEATURE - NH2 attached to Cys
CXQYXPXILC

SEQ ID NO: 100 - protein, 10 aa, synthetic construct
  REGION 1..10: note = synthetic
  SITE 1: note = MISC_FEATURE - n-butyloxycarbonyl attached to Cys
  REGION 1..10: note = MISC_FEATURE - cycle formed
  SITE 3: note = MISC_FEATURE - Xaa is Dab DOTA conjugate
  SITE 6: note = MISC_FEATURE - Xaa is (2S,4S)-4-fluoro-pyrrolidine-2-carboxylic acid
  SITE 7: note = MISC_FEATURE - Xaa is 4-(R)-hydroxy-l-proline
  SITE 9: note = MISC_FEATURE - Xaa is l-norvaline
  SITE 10: note = MISC_FEATURE - NH2 attached to Cys
CTXYFXXIXC

SEQ ID NO: 101 - protein, 12 aa, synthetic construct
  REGION 1..12: note = synthetic
  SITE 1: note = MISC_FEATURE - 2,2 ,2 ,2 -(1,4,7,10-Tetraazacyclododecane-1,4,7,10-tetrayl)tetraacetic acid attached to 8-amino-3,6-dioxaoctanoic acid
  SITE 1: note = MISC_FEATURE - Xaa is 8-amino-3,6-dioxaoctanoic acid
  REGION 3..12: note = MISC_FEATURE - cycle formed
  SITE 4: note = MISC_FEATURE - Xaa is l-Citrulline
  SITE 12: note = MISC_FEATURE - NH2 attached to Cys
XLCXQYFPPILC

SEQ ID NO: 102 - protein, 12 aa, synthetic construct
  REGION 1..12: note = synthetic
  SITE 1: note = MISC_FEATURE - Acetyl attached to Asp
  REGION 3..12: note = MISC_FEATURE - cycle formed
  SITE 5: note = MISC_FEATURE - Xaa is l-norleucine
  SITE 7: note = MISC_FEATURE - Xaa is d-phenylalanine
  SITE 12: note = MISC_FEATURE - NH2 attached to Cys
DLCRXYXPAILC

SEQ ID NO: 103 - protein, 10 aa, synthetic construct
  REGION 1..10: note = synthetic
  SITE 1: note = MISC_FEATURE - isocaproic acid attached to Cys
  REGION 1..10: note = MISC_FEATURE - cycle formed
  SITE 2: note = MISC_FEATURE - Xaa is d-alanine
  SITE 7: note = MISC_FEATURE - Xaa is d-alanine
  SITE 10: note = MISC_FEATURE - NH2 attached to Cys
CXQYFPXILC

SEQ ID NO: 104 - protein, 10 aa, synthetic construct
  REGION 1..10: note = synthetic
  SITE 1: note = MISC_FEATURE - isocaproic acid attached to Cys
  REGION 1..10: note = MISC_FEATURE - cycle formed
  SITE 2: note = MISC_FEATURE - Xaa is l-Citrulline
  SITE 6: note = MISC_FEATURE - Xaa is (S)-pipecolic Acid
  SITE 7: note = MISC_FEATURE - Xaa is d-alanine
  SITE 10: note = MISC_FEATURE - NH2 attached to Cys
CXQYFXXILC

SEQ ID NO: 105 - protein, 10 aa, synthetic construct
  REGION 1..10: note = synthetic
  SITE 1: note = MISC_FEATURE - pentanoic acid attached to Cys
  REGION 1..10: note = MISC_FEATURE - cycle formed
  SITE 2: note = MISC_FEATURE - Xaa is l-Citrulline
  SITE 3: note = MISC_FEATURE - Xaa is l-lysine DOTA conjugate
  SITE 5: note = MISC_FEATURE - Xaa is 4-chloro-l-phenylalanine
  SITE 7: note = MISC_FEATURE - Xaa is 4-(R)-hydroxy-l-proline
  SITE 9: note = MISC_FEATURE - Xaa is l-norvaline
  SITE 10: note = MISC_FEATURE - NH2 attached to Cys
CXXYXPXIXC

SEQ ID NO: 106 - protein, 10 aa, synthetic construct
  REGION 1..10: note = synthetic
  SITE 1: note = MISC_FEATURE - n-butyloxycarbonyl attached to Cys
  REGION 1..10: note = MISC_FEATURE - cycle formed
  SITE 3: note = MISC_FEATURE - Xaa is l-ornithine DOTA conjugate
  SITE 4: note = MISC_FEATURE - Xaa is 3-amino-l-tyrosine
  SITE 6: note = MISC_FEATURE - Xaa is (2S,4S)-4-fluoro-pyrrolidine-2-carboxylic acid
  SITE 7: note = MISC_FEATURE - Xaa is 4-(R)-hydroxy-l-proline
  SITE 9: note = MISC_FEATURE - Xaa is l-norvaline
  SITE 10: note = MISC_FEATURE - NH2 attached to Cys
CTXXFXXIXC

SEQ ID NO: 107 - protein, 12 aa, synthetic construct
  REGION 1..12: note = synthetic
  SITE 1: note = MISC_FEATURE - hexanoic acid attached to Asp
  REGION 3..12: note = MISC_FEATURE - cycle formed
  SITE 4: note = MISC_FEATURE - Xaa is l-lysine DOTA conjugate
  SITE 12: note = MISC_FEATURE - NH2 attached to Cys
DLCXMYFPAILC

SEQ ID NO: 108 - protein, 10 aa, synthetic construct
  REGION 1..10: note = synthetic
  SITE 1: note = MISC_FEATURE - pentanoic acid attached to Cys
  REGION 1..10: note = MISC_FEATURE - cycle formed
  SITE 7: note = MISC_FEATURE - Xaa is 4-(R)-hydroxy-l-proline
  SITE 9: note = MISC_FEATURE - Xaa is l-norvaline
  SITE 10: note = MISC_FEATURE - NH2 attached to Cys
CGQYFPXIXC

SEQ ID NO: 109 - protein, 10 aa, synthetic construct
  REGION 1..10: note = synthetic
  SITE 1: note = MISC_FEATURE - n-butyloxycarbonyl attached to Cys
  REGION 1..10: note = MISC_FEATURE - cycle formed
  SITE 3: note = MISC_FEATURE - Xaa is l-lysine DOTA conjugate
  SITE 6: note = MISC_FEATURE - Xaa is (2S,4S)-4-fluoro-pyrrolidine-2-carboxylic acid
  SITE 7: note = MISC_FEATURE - Xaa is 4-(R)-hydroxy-l-proline
  SITE 9: note = MISC_FEATURE - Xaa is l-norvaline
  SITE 10: note = MISC_FEATURE - NH2 attached to Cys
CTXYFXXIXC

SEQ ID NO: 110 - protein, 10 aa, synthetic construct
  REGION 1..10: note = synthetic
  SITE 1: note = MISC_FEATURE - n-butyloxycarbonyl attached to Cys
  REGION 1..10: note = MISC_FEATURE - cycle formed
  SITE 3: note = MISC_FEATURE - Xaa is l-lysine Lu(III) DOTA conjugate
  SITE 4: note = MISC_FEATURE - Xaa is Levodopa / l-3,4-dihydroxyphenylalanine
  SITE 6: note = MISC_FEATURE - Xaa is (2S,4S)-4-fluoro-pyrrolidine-2-carboxylic acid
  SITE 7: note = MISC_FEATURE - Xaa is 4-(R)-hydroxy-l-proline
  SITE 9: note = MISC_FEATURE - Xaa is l-norvaline
  SITE 10: note = MISC_FEATURE - NH2 attached to Cys
CTXXFXXIXC

SEQ ID NO: 111 - protein, 12 aa, synthetic construct
  REGION 1..12: note = synthetic
  SITE 1: note = MISC_FEATURE - Acetyl attached to Asp
  REGION 3..12: note = MISC_FEATURE - cycle formed
  SITE 5: note = MISC_FEATURE - Xaa is l-norleucine
  SITE 12: note = MISC_FEATURE - NH2 attached to Cys
DLCEXYFPAILC

SEQ ID NO: 112 - protein, 10 aa, synthetic construct
  REGION 1..10: note = synthetic
  SITE 1: note = MISC_FEATURE - isocaproic acid attached to Cys
  REGION 1..10: note = MISC_FEATURE - cycle formed
  SITE 2: note = MISC_FEATURE - Xaa is l-Citrulline
  SITE 3: note = MISC_FEATURE - Xaa is l-lysine DOTA conjugate
  SITE 7: note = MISC_FEATURE - Xaa is 4-(R)-hydroxy-l-proline
  SITE 10: note = MISC_FEATURE - NH2 attached to Cys
CXXYFPXILC

SEQ ID NO: 113 - protein, 10 aa, synthetic construct
  REGION 1..10: note = synthetic
  SITE 1: note = MISC_FEATURE - n-butyloxycarbonyl attached to Cys
  REGION 1..10: note = MISC_FEATURE - cycle formed
  SITE 3: note = MISC_FEATURE - Xaa is l-lysine Ga(III) DOTA conjugate
  SITE 4: note = MISC_FEATURE - Xaa is Levodopa / l-3,4-dihydroxyphenylalanine
  SITE 6: note = MISC_FEATURE - Xaa is (2S,4S)-4-fluoro-pyrrolidine-2-carboxylic acid
  SITE 7: note = MISC_FEATURE - Xaa is 4-(R)-hydroxy-l-proline
  SITE 9: note = MISC_FEATURE - Xaa is l-norvaline
  SITE 10: note = MISC_FEATURE - NH2 attached to Cys
CTXXFXXIXC

SEQ ID NO: 114 - protein, 10 aa, synthetic construct
  REGION 1..10: note = synthetic
  SITE 1: note = MISC_FEATURE - n-butyl-carbamoyl attached to Cys
  REGION 1..10: note = MISC_FEATURE - cycle formed
  SITE 3: note = MISC_FEATURE - Xaa is l-lysine DOTA conjugate
  SITE 7: note = MISC_FEATURE - Xaa is 4-(R)-hydroxy-l-proline
  SITE 9: note = MISC_FEATURE - Xaa is l-norvaline
  SITE 10: note = MISC_FEATURE - NH2 attached to Cys
CTXYFPXIXC

SEQ ID NO: 115 - protein, 10 aa, synthetic construct
  REGION 1..10: note = synthetic
  SITE 1: note = MISC_FEATURE - Acetyl attached to Cys
  REGION 1..10: note = MISC_FEATURE - cycle formed
  SITE 2: note = MISC_FEATURE - Xaa is l-Citrulline
  SITE 7: note = MISC_FEATURE - Xaa is d-alanine
  SITE 10: note = MISC_FEATURE - NH2 attached to Cys
CXQYFPXILC

SEQ ID NO: 116 - protein, 12 aa, synthetic construct
  REGION 1..12: note = synthetic
  SITE 1: note = MISC_FEATURE - Acetyl attached to Asp
  SITE 2: note = MISC_FEATURE - Xaa is d-leucine
  REGION 3..12: note = MISC_FEATURE - cycle formed
  SITE 5: note = MISC_FEATURE - Xaa is l-norleucine
  SITE 12: note = MISC_FEATURE - NH2 attached to Cys
DXCRXYFPAILC

SEQ ID NO: 117 - protein, 12 aa, synthetic construct
  REGION 1..12: note = synthetic
  SITE 1: note = MISC_FEATURE - 2,2 ,2 ,2 -(1,4,7,10-Tetraazacyclododecane-1,4,7,10-tetrayl)tetraacetic acid attached to 8-amino-3,6-dioxaoctanoic acid
  SITE 1: note = MISC_FEATURE - Xaa is 8-amino-3,6-dioxaoctanoic acid
  REGION 3..12: note = MISC_FEATURE - cycle formed
  SITE 4: note = MISC_FEATURE - Xaa is l-Citrulline
  SITE 9: note = MISC_FEATURE - Xaa is d-alanine
  SITE 12: note = MISC_FEATURE - NH2 attached to Cys
XLCXQYFPXILC

SEQ ID NO: 118 - protein, 10 aa, synthetic construct
  REGION 1..10: note = synthetic
  SITE 1: note = MISC_FEATURE - pentanoic acid attached to Cys
  REGION 1..10: note = MISC_FEATURE - cycle formed
  SITE 2: note = MISC_FEATURE - Xaa is l-Citrulline
  SITE 3: note = MISC_FEATURE - Xaa is l-lysine DOTA conjugate
  SITE 7: note = MISC_FEATURE - Xaa is 4-(R)-Fluoro-l-proline
  SITE 9: note = MISC_FEATURE - Xaa is l-norvaline
  SITE 10: note = MISC_FEATURE - NH2 attached to Cys
CXXYFPXIXC

SEQ ID NO: 119 - protein, 10 aa, synthetic construct
  REGION 1..10: note = synthetic
  SITE 1: note = MISC_FEATURE - pentanoic acid attached to Cys
  REGION 1..10: note = MISC_FEATURE - cycle formed
  SITE 2: note = MISC_FEATURE - Xaa is l-ornithine Tris-PEG conjugate
  SITE 3: note = MISC_FEATURE - Xaa is l-lysine DOTA conjugate
  SITE 7: note = MISC_FEATURE - Xaa is 4-(R)-hydroxy-l-proline
  SITE 9: note = MISC_FEATURE - Xaa is l-norvaline
  SITE 10: note = MISC_FEATURE - NH2 attached to Cys
CXXYFPXIXC

SEQ ID NO: 120 - protein, 10 aa, synthetic construct
  REGION 1..10: note = synthetic
  SITE 1: note = MISC_FEATURE - n-butyloxycarbonyl attached to Cys
  REGION 1..10: note = MISC_FEATURE - cycle formed
  SITE 3: note = MISC_FEATURE - Xaa is l-lysine DOTA conjugate
  SITE 7: note = MISC_FEATURE - Xaa is 4-(R)-hydroxy-l-proline
  SITE 9: note = MISC_FEATURE - Xaa is l-norvaline
  SITE 10: note = MISC_FEATURE - NH2 attached to Cys
CTXYFPXIXC

SEQ ID NO: 121 - protein, 10 aa, synthetic construct
  REGION 1..10: note = synthetic
  SITE 1: note = MISC_FEATURE - n-butyloxycarbonyl attached to Cys
  REGION 1..10: note = MISC_FEATURE - cycle formed
  SITE 3: note = MISC_FEATURE - Xaa is l-lysine DOTA conjugate
  SITE 4: note = MISC_FEATURE - Xaa is Levodopa / l-3,4-dihydroxyphenylalanine
  SITE 6: note = MISC_FEATURE - Xaa is (2S,4S)-4-fluoro-pyrrolidine-2-carboxylic acid
  SITE 7: note = MISC_FEATURE - Xaa is 4-(R)-hydroxy-l-proline
  SITE 9: note = MISC_FEATURE - Xaa is l-norvaline
  SITE 10: note = MISC_FEATURE - NH2 attached to Cys
CTXXFXXIXC

SEQ ID NO: 122 - protein, 10 aa, synthetic construct
  REGION 1..10: note = synthetic
  SITE 1: note = MISC_FEATURE - n-butyloxycarbonyl attached to Cys
  REGION 1..10: note = MISC_FEATURE - cycle formed
  SITE 3: note = MISC_FEATURE - Xaa is l-lysine NOTA conjugate
  SITE 4: note = MISC_FEATURE - Xaa is Levodopa / l-3,4-dihydroxyphenylalanine
  SITE 6: note = MISC_FEATURE - Xaa is (2S,4S)-4-fluoro-pyrrolidine-2-carboxylic acid
  SITE 7: note = MISC_FEATURE - Xaa is 4-(R)-hydroxy-l-proline
  SITE 9: note = MISC_FEATURE - Xaa is l-norvaline
  SITE 10: note = MISC_FEATURE - NH2 attached to Cys
CTXXFXXIXC

SEQ ID NO: 123 - protein, 10 aa, synthetic construct
  REGION 1..10: note = synthetic
  SITE 1: note = MISC_FEATURE - pentanoic acid attached to Cys
  REGION 1..10: note = MISC_FEATURE - cycle formed
  SITE 2: note = MISC_FEATURE - Xaa is l-Citrulline
  SITE 3: note = MISC_FEATURE - Xaa is l-lysine Gd (III) DOTA conjugate
  SITE 4: note = MISC_FEATURE - Xaa is 3-pyridyl-alanine
  SITE 7: note = MISC_FEATURE - Xaa is 4-(R)-hydroxy-l-proline
  SITE 9: note = MISC_FEATURE - Xaa is l-norvaline
  SITE 10: note = MISC_FEATURE - NH2 attached to Cys
CXXXFPXIXC

SEQ ID NO: 124 - protein, 10 aa, synthetic construct
  REGION 1..10: note = synthetic
  SITE 1: note = MISC_FEATURE - pentanoic acid attached to Cys
  REGION 1..10: note = MISC_FEATURE - cycle formed
  SITE 2: note = MISC_FEATURE - Xaa is l-Citrulline
  SITE 3: note = MISC_FEATURE - Xaa is l-lysine DOTA conjugate
  SITE 5: note = MISC_FEATURE - Xaa is (S)-1,2,3,4-tetrahydroisoquinoline-3-carboxylic acid
  SITE 7: note = MISC_FEATURE - Xaa is 4-(R)-hydroxy-l-proline
  SITE 9: note = MISC_FEATURE - Xaa is l-norvaline
  SITE 10: note = MISC_FEATURE - NH2 attached to Cys
CXXYXPXIXC

SEQ ID NO: 125 - protein, 10 aa, synthetic construct
  REGION 1..10: note = synthetic
  SITE 1: note = MISC_FEATURE - pentanoic acid attached to Cys
  REGION 1..10: note = MISC_FEATURE - cycle formed
  SITE 2: note = MISC_FEATURE - Xaa is l-Citrulline
  SITE 3: note = MISC_FEATURE - Xaa is l-lysine DOTA conjugate
  SITE 5: note = MISC_FEATURE - Xaa is 3-pyridyl-alanine
  SITE 7: note = MISC_FEATURE - Xaa is 4-(R)-hydroxy-l-proline
  SITE 9: note = MISC_FEATURE - Xaa is l-norvaline
  SITE 10: note = MISC_FEATURE - NH2 attached to Cys
CXXYXPXIXC

SEQ ID NO: 126 - protein, 10 aa, synthetic construct
  REGION 1..10: note = synthetic
  SITE 1: note = MISC_FEATURE - pentanoic acid attached to Cys
  REGION 1..10: note = MISC_FEATURE - cycle formed
  SITE 2: note = MISC_FEATURE - Xaa is l-Citrulline
  SITE 3: note = MISC_FEATURE - Xaa is l-lysine Lu(III) DOTA conjugate
  SITE 5: note = MISC_FEATURE - Xaa is 2,4-dichloro-l-phenylalanine
  SITE 7: note = MISC_FEATURE - Xaa is 4-(R)-hydroxy-l-proline
  SITE 9: note = MISC_FEATURE - Xaa is l-norvaline
  SITE 10: note = MISC_FEATURE - NH2 attached to Cys
CXXYXPXIXC

SEQ ID NO: 127 - protein, 10 aa, synthetic construct
  REGION 1..10: note = synthetic
  SITE 1: note = MISC_FEATURE - isocaproic acid attached to Cys
  REGION 1..10: note = MISC_FEATURE - cycle formed
  SITE 2: note = MISC_FEATURE - Xaa is l-Citrulline
  SITE 7: note = MISC_FEATURE - Xaa is d-alanine
  SITE 10: note = MISC_FEATURE - NH2 attached to Cys
CXEYFPXILC

SEQ ID NO: 128 - protein, 10 aa, synthetic construct
  REGION 1..10: note = synthetic
  SITE 1: note = MISC_FEATURE - isocaproic acid attached to Cys
  REGION 1..10: note = MISC_FEATURE - cycle formed
  SITE 2: note = MISC_FEATURE - Xaa is l-Citrulline
  SITE 3: note = MISC_FEATURE - Xaa is l-lysine DOTA conjugate
  SITE 7: note = MISC_FEATURE - Xaa is d-alanine
  SITE 10: note = MISC_FEATURE - NH2 attached to Cys
CXXYFPXILC

SEQ ID NO: 129 - protein, 10 aa, synthetic construct
  REGION 1..10: note = synthetic
  SITE 1: note = MISC_FEATURE - pentanoic acid attached to Cys
  REGION 1..10: note = MISC_FEATURE - cycle formed
  SITE 2: note = MISC_FEATURE - Xaa is l-Citrulline
  SITE 3: note = MISC_FEATURE - Xaa is l-lysine DOTA conjugate
  SITE 4: note = MISC_FEATURE - Xaa is 4-nitro-l-phenylalanine
  SITE 7: note = MISC_FEATURE - Xaa is 4-(R)-hydroxy-l-proline
  SITE 9: note = MISC_FEATURE - Xaa is l-norvaline
  SITE 10: note = MISC_FEATURE - NH2 attached to Cys
CXXXFPXIXC

SEQ ID NO: 130 - protein, 10 aa, synthetic construct
  REGION 1..10: note = synthetic
  SITE 1: note = MISC_FEATURE - pentanoic acid attached to l-cysteine bound to 2- methylbenzylidene
  SITE 1: note = MISC_FEATURE - Xaa is l-cysteine bound to 2- methylbenzylidene
  REGION 1..10: note = MISC_FEATURE - cycle formed
  SITE 7: note = MISC_FEATURE - Xaa is 4-(R)-hydroxy-l-proline
  SITE 9: note = MISC_FEATURE - Xaa is l-norvaline
  SITE 10: note = MISC_FEATURE - NH2 attached to Cys
XRQYFPXIXC

SEQ ID NO: 131 - protein, 10 aa, synthetic construct
  REGION 1..10: note = synthetic
  SITE 1: note = MISC_FEATURE - pentanoic acid attached to Cys
  REGION 1..10: note = MISC_FEATURE - cycle formed
  SITE 4: note = MISC_FEATURE - Xaa is 3-(2-naphthyl)-l-alanine
  SITE 7: note = MISC_FEATURE - Xaa is 4-(R)-hydroxy-l-proline
  SITE 9: note = MISC_FEATURE - Xaa is l-norvaline
  SITE 10: note = MISC_FEATURE - NH2 attached to Cys
CRQXFPXIXC

SEQ ID NO: 132 - protein, 10 aa, synthetic construct
  REGION 1..10: note = synthetic
  SITE 1: note = MISC_FEATURE - pentanoic acid attached to Cys
  REGION 1..10: note = MISC_FEATURE - cycle formed
  SITE 2: note = MISC_FEATURE - Xaa is l-Citrulline
  SITE 3: note = MISC_FEATURE - Xaa is l-lysine DOTA conjugate
  SITE 7: note = MISC_FEATURE - Xaa is 4-(R)-hydroxy-l-proline
  SITE 9: note = MISC_FEATURE - Xaa is l-norvaline
  SITE 10: note = MISC_FEATURE - NH2 attached to Cys
CXXYFPXIXC

SEQ ID NO: 133 - protein, 10 aa, synthetic construct
  REGION 1..10: note = synthetic
  SITE 1: note = MISC_FEATURE - isocaproic acid attached to Cys
  REGION 1..10: note = MISC_FEATURE - cycle formed
  SITE 2: note = MISC_FEATURE - Xaa is l-Citrulline
  SITE 7: note = MISC_FEATURE - Xaa is (S)-oxazolidine-4-carboxylic acid
  SITE 10: note = MISC_FEATURE - NH2 attached to Cys
CXQYFPXILC

SEQ ID NO: 134 - protein, 10 aa, synthetic construct
  REGION 1..10: note = synthetic
  SITE 1: note = MISC_FEATURE - isocaproic acid attached to Cys
  REGION 1..10: note = MISC_FEATURE - cycle formed
  SITE 2: note = MISC_FEATURE - Xaa is l-Citrulline
  SITE 7: note = MISC_FEATURE - Xaa is d-alanine
  SITE 10: note = MISC_FEATURE - NH2 attached to Cys
CXQYAPXILC

SEQ ID NO: 135 - protein, 10 aa, synthetic construct
  REGION 1..10: note = synthetic
  SITE 1: note = MISC_FEATURE - pentanoic acid attached to Cys
  REGION 1..10: note = MISC_FEATURE - cycle formed
  SITE 7: note = MISC_FEATURE - Xaa is 4-(R)-hydroxy-l-proline
  SITE 8: note = MISC_FEATURE - Xaa is 1-amino-1-cyclohexan-carboxylic acid
  SITE 9: note = MISC_FEATURE - Xaa is l-norvaline
  SITE 10: note = MISC_FEATURE - NH2 attached to Cys
CRQYFPXXXC

SEQ ID NO: 136 - protein, 10 aa, synthetic construct
  REGION 1..10: note = synthetic
  SITE 1: note = MISC_FEATURE - pentanoic acid attached to Cys
  REGION 1..10: note = MISC_FEATURE - cycle formed
  SITE 2: note = MISC_FEATURE - Xaa is l-Citrulline
  SITE 3: note = MISC_FEATURE - Xaa is l-lysine DOTA conjugate
  SITE 7: note = MISC_FEATURE - Xaa is N -methyl-l-ornithine
  SITE 9: note = MISC_FEATURE - Xaa is l-norvaline
  SITE 10: note = MISC_FEATURE - NH2 attached to Cys
CXXYFPXIXC

SEQ ID NO: 137 - protein, 10 aa, synthetic construct
  REGION 1..10: note = synthetic
  SITE 1: note = MISC_FEATURE - pentanoic acid attached to Cys
  REGION 1..10: note = MISC_FEATURE - cycle formed
  SITE 6: note = MISC_FEATURE - Xaa is l-cyclohexyl-alanine
  SITE 7: note = MISC_FEATURE - Xaa is 4-(R)-hydroxy-l-proline
  SITE 9: note = MISC_FEATURE - Xaa is l-norvaline
  SITE 10: note = MISC_FEATURE - NH2 attached to Cys
CRQYFXXIXC

SEQ ID NO: 138 - protein, 10 aa, synthetic construct
  REGION 1..10: note = synthetic
  SITE 1: note = MISC_FEATURE - n-propyloxycarbonyl attached to Cys
  REGION 1..10: note = MISC_FEATURE - cycle formed
  SITE 2: note = MISC_FEATURE - Xaa is l-Citrulline
  SITE 3: note = MISC_FEATURE - Xaa is l-lysine DOTA conjugate
  SITE 7: note = MISC_FEATURE - Xaa is 4-(R)-hydroxy-l-proline
  SITE 9: note = MISC_FEATURE - Xaa is l-norvaline
  SITE 10: note = MISC_FEATURE - NH2 attached to Cys
CXXYFPXIXC

SEQ ID NO: 139 - protein, 12 aa, synthetic construct
  REGION 1..12: note = synthetic
  SITE 1: note = MISC_FEATURE - 1-amino-1-deoxy-d-glucitol attached to glutaric acid as linker
  SITE 1: note = MISC_FEATURE - Xaa is glutaric acid as linker
  SITE 2: note = MISC_FEATURE - Xaa is l-norvaline
  REGION 3..12: note = MISC_FEATURE - cycle formed
  SITE 4: note = MISC_FEATURE - Xaa is l-Citrulline
  SITE 9: note = MISC_FEATURE - Xaa is 4-(R)-hydroxy-l-proline
  SITE 11: note = MISC_FEATURE - Xaa is l-norvaline
  SITE 12: note = MISC_FEATURE - NH2 attached to Cys
XXCXQYFPXIXC

SEQ ID NO: 140 - protein, 10 aa, synthetic construct
  REGION 1..10: note = synthetic
  SITE 1: note = MISC_FEATURE - isocaproic acid attached to Cys
  REGION 1..10: note = MISC_FEATURE - cycle formed
  SITE 2: note = MISC_FEATURE - Xaa is l-Citrulline
  SITE 3: note = MISC_FEATURE - Xaa is 1-amino-isobutyric acid
  SITE 7: note = MISC_FEATURE - Xaa is d-alanine
  SITE 10: note = MISC_FEATURE - NH2 attached to Cys
CXXYFPXILC

SEQ ID NO: 141 - protein, 12 aa, synthetic construct
  REGION 1..12: note = synthetic
  SITE 1: note = MISC_FEATURE - Acetyl attached to Asp
  REGION 3..12: note = MISC_FEATURE - cycle formed
  SITE 5: note = MISC_FEATURE - Xaa is l-norleucine
  SITE 12: note = MISC_FEATURE - NH2 attached to Cys
DLCRXYFPAILC

SEQ ID NO: 142 - protein, 9 aa, synthetic construct
  REGION 1..9: note = synthetic
  SITE 1: note = MISC_FEATURE - pentanoic acid attached to Cys
  REGION 1..9: note = MISC_FEATURE - cycle formed
  SITE 6: note = MISC_FEATURE - Xaa is 4-carboxymethyl piperazine
  SITE 8: note = MISC_FEATURE - Xaa is l-norvaline
  SITE 9: note = MISC_FEATURE - NH2 attached to Cys
CRQYFXIXC

SEQ ID NO: 143 - protein, 10 aa, synthetic construct
  REGION 1..10: note = synthetic
  SITE 1: note = MISC_FEATURE - 3-hydroxy propionic acid at the N-terminus attached to Cys
  REGION 1..10: note = MISC_FEATURE - cycle formed
  SITE 2: note = MISC_FEATURE - Xaa is l-Citrulline
  SITE 7: note = MISC_FEATURE - Xaa is d-alanine
  SITE 10: note = MISC_FEATURE - NH2 attached to Cys
CXQYFPXILC

SEQ ID NO: 144 - protein, 10 aa, synthetic construct
  REGION 1..10: note = synthetic
  SITE 1: note = MISC_FEATURE - pentanoic acid attached to Cys
  REGION 1..10: note = MISC_FEATURE - cycle formed
  SITE 5: note = MISC_FEATURE - Xaa is 3-(3-benzothienyl)-l-alanine
  SITE 7: note = MISC_FEATURE - Xaa is 4-(R)-hydroxy-l-proline
  SITE 9: note = MISC_FEATURE - Xaa is l-norvaline
  SITE 10: note = MISC_FEATURE - NH2 attached to Cys
CRQYXPXIXC

SEQ ID NO: 145 - protein, 12 aa, synthetic construct
  REGION 1..12: note = synthetic
  SITE 1: note = MISC_FEATURE - Acetyl attached to Asp
  REGION 3..12: note = MISC_FEATURE - cycle formed
  SITE 5: note = MISC_FEATURE - Xaa is d-norleucine
  SITE 12: note = MISC_FEATURE - NH2 attached to Cys
DLCRXYFPAILC

SEQ ID NO: 146 - protein, 10 aa, synthetic construct
  REGION 1..10: note = synthetic
  SITE 1: note = MISC_FEATURE - n-butyloxycarbonyl attached to Cys
  REGION 1..10: note = MISC_FEATURE - cycle formed
  SITE 2: note = MISC_FEATURE - Xaa is l-Citrulline
  SITE 3: note = MISC_FEATURE - Xaa is l-lysine DOTA conjugate
  SITE 7: note = MISC_FEATURE - Xaa is 4-(R)-hydroxy-l-proline
  SITE 9: note = MISC_FEATURE - Xaa is l-norvaline
  SITE 10: note = MISC_FEATURE - NH2 attached to Cys
CXXYFPXIXC

SEQ ID NO: 147 - protein, 10 aa, synthetic construct
  REGION 1..10: note = synthetic
  SITE 1: note = MISC_FEATURE - n-butyloxycarbonyl attached to Cys
  REGION 1..10: note = MISC_FEATURE - cycle formed
  SITE 3: note = MISC_FEATURE - Xaa is l-ornithine DOTA conjugate
  SITE 4: note = MISC_FEATURE - Xaa is 4-carbamoyl-l-phenylalanine
  SITE 6: note = MISC_FEATURE - Xaa is (2S,4S)-4-fluoro-pyrrolidine-2-carboxylic acid
  SITE 7: note = MISC_FEATURE - Xaa is 4-(R)-hydroxy-l-proline
  SITE 9: note = MISC_FEATURE - Xaa is l-norvaline
  SITE 10: note = MISC_FEATURE - NH2 attached to Cys
CTXXFXXIXC

SEQ ID NO: 148 - protein, 10 aa, synthetic construct
  REGION 1..10: note = synthetic
  SITE 1: note = MISC_FEATURE - pentanoic acid attached to Cys
  REGION 1..10: note = MISC_FEATURE - cycle formed
  SITE 2: note = MISC_FEATURE - Xaa is l-Citrulline
  SITE 3: note = MISC_FEATURE - Xaa is l-lysine DOTA conjugate
  SITE 7: note = MISC_FEATURE - Xaa is N-methyl-l-serine
  SITE 9: note = MISC_FEATURE - Xaa is l-norvaline
  SITE 10: note = MISC_FEATURE - NH2 attached to Cys
CXXYFPXIXC

SEQ ID NO: 149 - protein, 10 aa, synthetic construct
  REGION 1..10: note = synthetic
  SITE 1: note = MISC_FEATURE - pentanoic acid attached to Cys
  REGION 1..10: note = MISC_FEATURE - cycle formed
  SITE 2: note = MISC_FEATURE - Xaa is l-homoarginine
  SITE 3: note = MISC_FEATURE - Xaa is l-lysine DOTA conjugate
  SITE 7: note = MISC_FEATURE - Xaa is 4-(R)-hydroxy-l-proline
  SITE 9: note = MISC_FEATURE - Xaa is l-norvaline
  SITE 10: note = MISC_FEATURE - NH2 attached to Cys
CXXYFPXIXC

SEQ ID NO: 150 - protein, 10 aa, synthetic construct
  REGION 1..10: note = synthetic
  SITE 1: note = MISC_FEATURE - pentanoic acid attached to Cys
  REGION 1..10: note = MISC_FEATURE - cycle formed
  SITE 2: note = MISC_FEATURE - Xaa is l-Citrulline
  SITE 3: note = MISC_FEATURE - Xaa is l-lysine La(III) DOTA conjugate
  SITE 7: note = MISC_FEATURE - Xaa is 1-amino-isobutyric acid
  SITE 9: note = MISC_FEATURE - Xaa is l-norvaline
  SITE 10: note = MISC_FEATURE - NH2 attached to Cys
CXXYFPXIXC

SEQ ID NO: 151 - protein, 10 aa, synthetic construct
  REGION 1..10: note = synthetic
  SITE 1: note = MISC_FEATURE - n-butyloxycarbonyl attached to Cys
  REGION 1..10: note = MISC_FEATURE - cycle formed
  SITE 3: note = MISC_FEATURE - Xaa is l-ornithine DOTA conjugate
  SITE 4: note = MISC_FEATURE - Xaa is Levodopa / l-3,4-dihydroxyphenylalanine
  SITE 6: note = MISC_FEATURE - Xaa is (2S,4S)-4-fluoro-pyrrolidine-2-carboxylic acid
  SITE 7: note = MISC_FEATURE - Xaa is 4-(R)-hydroxy-l-proline
  SITE 9: note = MISC_FEATURE - Xaa is l-norvaline
  SITE 10: note = MISC_FEATURE - NH2 attached to Cys
CTXXFXXIXC

SEQ ID NO: 152 - protein, 10 aa, synthetic construct
  REGION 1..10: note = synthetic
  SITE 1: note = MISC_FEATURE - pentanoic acid attached to Cys
  REGION 1..10: note = MISC_FEATURE - cycle formed
  SITE 9: note = MISC_FEATURE - Xaa is l-norvaline
  SITE 10: note = MISC_FEATURE - NH2 attached to Cys
CRQYFPLIXC

SEQ ID NO: 153 - protein, 10 aa, synthetic construct
  REGION 1..10: note = synthetic
  SITE 1: note = MISC_FEATURE - pentanoic acid attached to Cys
  REGION 1..10: note = MISC_FEATURE - cycle formed
  SITE 3: note = MISC_FEATURE - Xaa is l-lysine DOTA conjugate
  SITE 7: note = MISC_FEATURE - Xaa is 4-(R)-hydroxy-l-proline
  SITE 9: note = MISC_FEATURE - Xaa is l-norvaline
  SITE 10: note = MISC_FEATURE - NH2 attached to Cys
CNXYFPXIXC

SEQ ID NO: 154 - protein, 10 aa, synthetic construct
  REGION 1..10: note = synthetic
  SITE 1: note = MISC_FEATURE - n-butyloxycarbonyl attached to Cys
  REGION 1..10: note = MISC_FEATURE - cycle formed
  SITE 3: note = MISC_FEATURE - Xaa is l-lysine DOTA conjugate
  SITE 4: note = MISC_FEATURE - Xaa is Levodopa / l-3,4-dihydroxyphenylalanine
  SITE 6: note = MISC_FEATURE - Xaa is 4-(R)-hydroxy-l-proline
  SITE 7: note = MISC_FEATURE - Xaa is 4-(R)-hydroxy-l-proline
  SITE 9: note = MISC_FEATURE - Xaa is l-norvaline
  SITE 10: note = MISC_FEATURE - NH2 attached to Cys
CTXXFXXIXC

SEQ ID NO: 155 - protein, 10 aa, synthetic construct
  REGION 1..10: note = synthetic
  SITE 1: note = MISC_FEATURE - isocaproic acid attached to Cys
  REGION 1..10: note = MISC_FEATURE - cycle formed
  SITE 2: note = MISC_FEATURE - Xaa is l-Citrulline
  SITE 4: note = MISC_FEATURE - Xaa is N-methyl-l-tyrosine
  SITE 7: note = MISC_FEATURE - Xaa is d-alanine
  SITE 10: note = MISC_FEATURE - NH2 attached to Cys
CXQXFPXILC

SEQ ID NO: 156 - protein, 10 aa, synthetic construct
  REGION 1..10: note = synthetic
  SITE 1: note = MISC_FEATURE - n-butyl-carbamoyl attached to Cys
  REGION 1..10: note = MISC_FEATURE - cycle formed
  SITE 2: note = MISC_FEATURE - Xaa is l-Citrulline
  SITE 7: note = MISC_FEATURE - Xaa is d-alanine
  SITE 10: note = MISC_FEATURE - NH2 attached to Cys
CXQYFPXILC

SEQ ID NO: 157 - protein, 10 aa, synthetic construct
  REGION 1..10: note = synthetic
  SITE 1: note = MISC_FEATURE - isocaproic acid attached to Cys
  REGION 1..10: note = MISC_FEATURE - cycle formed
  SITE 2: note = MISC_FEATURE - Xaa is N -methyl-l-arginine
  SITE 7: note = MISC_FEATURE - Xaa is d-alanine
  SITE 10: note = MISC_FEATURE - NH2 attached to Cys
CXQYFPXILC

SEQ ID NO: 158 - protein, 10 aa, synthetic construct
  REGION 1..10: note = synthetic
  SITE 1: note = MISC_FEATURE - pentanoic acid attached to Cys
  REGION 1..10: note = MISC_FEATURE - cycle formed
  SITE 3: note = MISC_FEATURE - Xaa is 4-aminopiperidine-4-carboxylic acid DOTA conjugate
  SITE 7: note = MISC_FEATURE - Xaa is 4-(R)-hydroxy-l-proline
  SITE 9: note = MISC_FEATURE - Xaa is l-norvaline
  SITE 10: note = MISC_FEATURE - NH2 attached to Cys
CTXYFPXIXC

SEQ ID NO: 159 - protein, 10 aa, synthetic construct
  REGION 1..10: note = synthetic
  SITE 1: note = MISC_FEATURE - n-butyloxycarbonyl attached to Cys
  REGION 1..10: note = MISC_FEATURE - cycle formed
  SITE 3: note = MISC_FEATURE - Xaa is l-lysine DOTA conjugate
  SITE 7: note = MISC_FEATURE - Xaa is 4-(R)-Fluoro-l-proline
  SITE 9: note = MISC_FEATURE - Xaa is l-norvaline
  SITE 10: note = MISC_FEATURE - NH2 attached to Cys
CTXYFPXIXC

SEQ ID NO: 160 - protein, 12 aa, synthetic construct
  REGION 1..12: note = synthetic
  SITE 1: note = MISC_FEATURE - Acetyl attached to Asp
  REGION 3..12: note = MISC_FEATURE - cycle formed
  SITE 12: note = MISC_FEATURE - NH2 attached to Cys
DLCRQYFPAILC

SEQ ID NO: 161 - protein, 12 aa, synthetic construct
  REGION 1..12: note = synthetic
  SITE 1: note = MISC_FEATURE - 2,2 ,2 ,2 -(1,4,7,10-Tetraazacyclododecane-1,4,7,10-tetrayl)tetraacetic acid attached to 6-aminohexanoic acid
  SITE 1: note = MISC_FEATURE - Xaa is 6-aminohexanoic acid
  REGION 3..12: note = MISC_FEATURE - cycle formed
  SITE 9: note = MISC_FEATURE - Xaa is d-alanine
  SITE 12: note = MISC_FEATURE - NH2 attached to Cys
XLCRQYFPXILC

SEQ ID NO: 162 - protein, 10 aa, synthetic construct
  REGION 1..10: note = synthetic
  SITE 1: note = MISC_FEATURE - pentanoic acid attached to Cys
  REGION 1..10: note = MISC_FEATURE - cycle formed
  SITE 2: note = MISC_FEATURE - Xaa is l-Citrulline
  SITE 7: note = MISC_FEATURE - Xaa is 4-(R)-hydroxy-l-proline
  SITE 9: note = MISC_FEATURE - Xaa is l-norvaline
  SITE 10: note = MISC_FEATURE - Xaa is l-cysteinol
CXQYFPXIXX

SEQ ID NO: 163 - protein, 11 aa, synthetic construct
  REGION 1..11: note = synthetic
  SITE 1: note = MISC_FEATURE - succinic acid at N-terminus attached to l-norvaline
  SITE 1: note = MISC_FEATURE - Xaa is l-norvaline
  REGION 2..11: note = MISC_FEATURE - cycle formed
  SITE 3: note = MISC_FEATURE - Xaa is l-Citrulline
  SITE 4: note = MISC_FEATURE - Xaa is l-lysine DOTA conjugate
  SITE 8: note = MISC_FEATURE - Xaa is 4-(R)-hydroxy-l-proline
  SITE 10: note = MISC_FEATURE - Xaa is l-norvaline
  SITE 11: note = MISC_FEATURE - NH2 attached to Cys
XCXXYFPXIXC

SEQ ID NO: 164 - protein, 10 aa, synthetic construct
  REGION 1..10: note = synthetic
  SITE 1: note = MISC_FEATURE - n-butyloxycarbonyl attached to Cys
  REGION 1..10: note = MISC_FEATURE - cycle formed
  SITE 3: note = MISC_FEATURE - Xaa is l-lysine In(III) DOTA conjugate
  SITE 6: note = MISC_FEATURE - Xaa is (2S,4S)-4-fluoro-pyrrolidine-2-carboxylic acid
  SITE 7: note = MISC_FEATURE - Xaa is 4-(R)-hydroxy-l-proline
  SITE 9: note = MISC_FEATURE - Xaa is l-norvaline
  SITE 10: note = MISC_FEATURE - NH2 attached to Cys
CTXYFXXIXC

SEQ ID NO: 165 - protein, 10 aa, synthetic construct
  REGION 1..10: note = synthetic
  SITE 1: note = MISC_FEATURE - isocaproic acid attached to Cys
  REGION 1..10: note = MISC_FEATURE - cycle formed
  SITE 2: note = MISC_FEATURE - Xaa is l-Citrulline
  SITE 7: note = MISC_FEATURE - Xaa is (2S,4R)-4-amino-1-pyrrolidin-2-carboxylic acid
  SITE 10: note = MISC_FEATURE - NH2 attached to Cys
CXQYFPXILC

SEQ ID NO: 166 - protein, 10 aa, synthetic construct
  REGION 1..10: note = synthetic
  SITE 1: note = MISC_FEATURE - pentanoic acid attached to Cys
  REGION 1..10: note = MISC_FEATURE - cycle formed
  SITE 2: note = MISC_FEATURE - Xaa is l-Citrulline
  SITE 3: note = MISC_FEATURE - Xaa is l-lysine La(III) DOTA conjugate
  SITE 4: note = MISC_FEATURE - Xaa is (S)-4-pyridyl-alanine
  SITE 7: note = MISC_FEATURE - Xaa is 4-(R)-hydroxy-l-proline
  SITE 9: note = MISC_FEATURE - Xaa is l-norvaline
  SITE 10: note = MISC_FEATURE - NH2 attached to Cys
CXXXFPXIXC

SEQ ID NO: 167 - protein, 11 aa, synthetic construct
  REGION 1..11: note = synthetic
  SITE 1: note = MISC_FEATURE - succinic acid at N-terminus attached to l-norvaline
  SITE 1: note = MISC_FEATURE - Xaa is l-norvaline
  REGION 2..11: note = MISC_FEATURE - cycle formed
  SITE 4: note = MISC_FEATURE - Xaa is l-lysine DOTA conjugate
  SITE 8: note = MISC_FEATURE - Xaa is 4-(R)-hydroxy-l-proline
  SITE 10: note = MISC_FEATURE - Xaa is l-norvaline
  SITE 11: note = MISC_FEATURE - NH2 attached to Cys
XCTXYFPXIXC

SEQ ID NO: 168 - protein, 10 aa, synthetic construct
  REGION 1..10: note = synthetic
  SITE 1: note = MISC_FEATURE - pentanoic acid attached to Cys
  REGION 1..10: note = MISC_FEATURE - cycle formed
  SITE 7: note = MISC_FEATURE - Xaa is 4-(R)-hydroxy-l-proline
  SITE 9: note = MISC_FEATURE - Xaa is l-norvaline
  SITE 10: note = MISC_FEATURE - NH2 attached to Cys
CRQYFKXIXC

SEQ ID NO: 169 - protein, 10 aa, synthetic construct
  REGION 1..10: note = synthetic
  SITE 1: note = MISC_FEATURE - pentanoic acid attached to Cys
  REGION 1..10: note = MISC_FEATURE - cycle formed
  SITE 2: note = MISC_FEATURE - Xaa is l-Citrulline
  SITE 3: note = MISC_FEATURE - Xaa is l-lysine DOTA conjugate
  SITE 7: note = MISC_FEATURE - Xaa is 1-amino-isobutyric acid
  SITE 9: note = MISC_FEATURE - Xaa is l-norvaline
  SITE 10: note = MISC_FEATURE - NH2 attached to Cys
CXXYFPXIXC

SEQ ID NO: 170 - protein, 10 aa, synthetic construct
  REGION 1..10: note = synthetic
  SITE 1: note = MISC_FEATURE - pentanoic acid attached to l-homocysteine
  SITE 1: note = MISC_FEATURE - Xaa is l-homocysteine
  REGION 1..10: note = MISC_FEATURE - cycle formed
  SITE 7: note = MISC_FEATURE - Xaa is 4-(R)-hydroxy-l-proline
  SITE 9: note = MISC_FEATURE - Xaa is l-norvaline
  SITE 10: note = MISC_FEATURE - NH2 attached to Cys
XRQYFPXIXC

SEQ ID NO: 171 - protein, 10 aa, synthetic construct
  REGION 1..10: note = synthetic
  SITE 1: note = MISC_FEATURE - pentanoic acid attached to Cys
  REGION 1..10: note = MISC_FEATURE - cycle formed
  SITE 3: note = MISC_FEATURE - Xaa is l-lysine DOTA conjugate
  SITE 7: note = MISC_FEATURE - Xaa is 4-(R)-hydroxy-l-proline
  SITE 9: note = MISC_FEATURE - Xaa is l-norvaline
  SITE 10: note = MISC_FEATURE - NH2 attached to Cys
CTXYFPXIXC

SEQ ID NO: 172 - protein, 10 aa, synthetic construct
  REGION 1..10: note = synthetic
  SITE 1: note = MISC_FEATURE - pentanoic acid attached to Cys
  REGION 1..10: note = MISC_FEATURE - cycle formed
  SITE 6: note = MISC_FEATURE - Xaa is N-methyl-l-leucine
  SITE 7: note = MISC_FEATURE - Xaa is 4-(R)-hydroxy-l-proline
  SITE 9: note = MISC_FEATURE - Xaa is l-norvaline
  SITE 10: note = MISC_FEATURE - NH2 attached to Cys
CRQYFXXIXC

SEQ ID NO: 173 - protein, 10 aa, synthetic construct
  REGION 1..10: note = synthetic
  SITE 1: note = MISC_FEATURE - pentanoic acid attached to Cys
  REGION 1..10: note = MISC_FEATURE - cycle formed
  SITE 2: note = MISC_FEATURE - Xaa is l-Citrulline
  SITE 3: note = MISC_FEATURE - Xaa is l-lysine La(III) DOTA conjugate
  SITE 6: note = MISC_FEATURE - Xaa is (2S,4S)-4-fluoro-pyrrolidine-2-carboxylic acid
  SITE 7: note = MISC_FEATURE - Xaa is 4-(R)-hydroxy-l-proline
  SITE 9: note = MISC_FEATURE - Xaa is l-norvaline
  SITE 10: note = MISC_FEATURE - NH2 attached to Cys
CXXYFXXIXC

SEQ ID NO: 174 - protein, 10 aa, synthetic construct
  REGION 1..10: note = synthetic
  SITE 1: note = MISC_FEATURE - n-butyloxycarbonyl attached to Cys
  REGION 1..10: note = MISC_FEATURE - cycle formed
  SITE 2: note = MISC_FEATURE - Xaa is l-Citrulline
  SITE 3: note = MISC_FEATURE - Xaa is l-lysine DOTA conjugate
  SITE 5: note = MISC_FEATURE - Xaa is 4-chloro-l-phenylalanine
  SITE 6: note = MISC_FEATURE - Xaa is (2S,4S)-4-fluoro-pyrrolidine-2-carboxylic acid
  SITE 7: note = MISC_FEATURE - Xaa is 4-(R)-hydroxy-l-proline
  SITE 9: note = MISC_FEATURE - Xaa is l-norvaline
  SITE 10: note = MISC_FEATURE - NH2 attached to Cys
CXXYXXXIXC

SEQ ID NO: 175 - protein, 10 aa, synthetic construct
  REGION 1..10: note = synthetic
  SITE 1: note = MISC_FEATURE - isocaproic acid attached to Cys
  REGION 1..10: note = MISC_FEATURE - cycle formed
  SITE 2: note = MISC_FEATURE - Xaa is l-Citrulline
  SITE 7: note = MISC_FEATURE - Xaa is d-proline
  SITE 10: note = MISC_FEATURE - NH2 attached to Cys
CXQYFPXILC

SEQ ID NO: 176 - protein, 12 aa, synthetic construct
  REGION 1..12: note = synthetic
  SITE 1: note = MISC_FEATURE - Acetyl attached to Asp
  REGION 3..12: note = MISC_FEATURE - cycle formed
  SITE 4: note = MISC_FEATURE - Xaa is l-Citrulline
  SITE 5: note = MISC_FEATURE - Xaa is l-lysine DOTA conjugate
  SITE 9: note = MISC_FEATURE - Xaa is d-arginine
  SITE 12: note = MISC_FEATURE - NH2 attached to Cys
DLCXXYFPXILC

SEQ ID NO: 177 - protein, 10 aa, synthetic construct
  REGION 1..10: note = synthetic
  SITE 1: note = MISC_FEATURE - isocaproic acid attached to Cys
  REGION 1..10: note = MISC_FEATURE - cycle formed
  SITE 2: note = MISC_FEATURE - Xaa is l-Citrulline
  SITE 7: note = MISC_FEATURE - Xaa is (2S,4S)-4-fluoro-pyrrolidine-2-carboxylic acid
  SITE 10: note = MISC_FEATURE - NH2 attached to Cys
CXQYFPXILC

SEQ ID NO: 178 - protein, 10 aa, synthetic construct
  REGION 1..10: note = synthetic
  SITE 1: note = MISC_FEATURE - pentanoic acid attached to Cys
  REGION 1..10: note = MISC_FEATURE - cycle formed
  SITE 7: note = MISC_FEATURE - Xaa is 4-(R)-hydroxy-l-proline
  SITE 9: note = MISC_FEATURE - Xaa is l-norvaline
  SITE 10: note = MISC_FEATURE - NH2 attached to Cys
CRQYWPXIXC

SEQ ID NO: 179 - protein, 10 aa, synthetic construct
  REGION 1..10: note = synthetic
  SITE 1: note = MISC_FEATURE - pentanoic acid attached to Cys
  REGION 1..10: note = MISC_FEATURE - cycle formed
  SITE 2: note = MISC_FEATURE - Xaa is l-Citrulline
  SITE 7: note = MISC_FEATURE - Xaa is 4-(R)-hydroxy-l-proline
  SITE 9: note = MISC_FEATURE - Xaa is l-norvaline
  SITE 10: note = MISC_FEATURE - NH2 attached to Cys
CXQYFPXIXC

SEQ ID NO: 180 - protein, 10 aa, synthetic construct
  REGION 1..10: note = synthetic
  SITE 1: note = MISC_FEATURE - isocaproic acid attached to Cys
  REGION 1..10: note = MISC_FEATURE - cycle formed
  SITE 2: note = MISC_FEATURE - Xaa is l-Citrulline
  SITE 5: note = MISC_FEATURE - Xaa is 3-(1-naphthyl)-l-alanine
  SITE 7: note = MISC_FEATURE - Xaa is d-alanine
  SITE 10: note = MISC_FEATURE - NH2 attached to Cys
CXQYXPXILC

SEQ ID NO: 181 - protein, 10 aa, synthetic construct
  REGION 1..10: note = synthetic
  SITE 1: note = MISC_FEATURE - pentanoic acid attached to Cys
  REGION 1..10: note = MISC_FEATURE - cycle formed
  SITE 2: note = MISC_FEATURE - Xaa is l-ornithine mPEG12 conjugate
  SITE 3: note = MISC_FEATURE - Xaa is l-lysine In(III) DOTA conjugate
  SITE 7: note = MISC_FEATURE - Xaa is 4-(R)-hydroxy-l-proline
  SITE 9: note = MISC_FEATURE - Xaa is l-norvaline
  SITE 10: note = MISC_FEATURE - NH2 attached to Cys
CXXYFPXIXC

SEQ ID NO: 182 - protein, 13 aa, synthetic construct
  REGION 1..13: note = synthetic
  REGION 4..13: note = MISC_FEATURE - cycle formed
  SITE 13: note = MISC_FEATURE - NH2 attached to Cys
MDLCRMYFPAILC

SEQ ID NO: 183 - protein, 10 aa, synthetic construct
  REGION 1..10: note = synthetic
  SITE 1: note = MISC_FEATURE - pentanoic acid attached to Cys
  REGION 1..10: note = MISC_FEATURE - cycle formed
  SITE 7: note = MISC_FEATURE - Xaa is (2S,4R)-4-amino-1-pyrrolidin-2-carboxylic acid
  SITE 9: note = MISC_FEATURE - Xaa is l-norvaline
  SITE 10: note = MISC_FEATURE - NH2 attached to Cys
CRRYFPXIXC

SEQ ID NO: 184 - protein, 10 aa, synthetic construct
  REGION 1..10: note = synthetic
  SITE 1: note = MISC_FEATURE - isocaproic acid attached to Cys
  REGION 1..10: note = MISC_FEATURE - cycle formed
  SITE 2: note = MISC_FEATURE - Xaa is l-Citrulline
  SITE 4: note = MISC_FEATURE - Xaa is 4-amino-l-phenylalanine
  SITE 7: note = MISC_FEATURE - Xaa is d-alanine
  SITE 10: note = MISC_FEATURE - NH2 attached to Cys
CXQXFPXILC

SEQ ID NO: 185 - protein, 10 aa, synthetic construct
  REGION 1..10: note = synthetic
  SITE 1: note = MISC_FEATURE - pentanoic acid attached to Cys
  REGION 1..10: note = MISC_FEATURE - cycle formed
  SITE 2: note = MISC_FEATURE - Xaa is l-Citrulline
  SITE 3: note = MISC_FEATURE - Xaa is l-lysine DOTA conjugate
  SITE 5: note = MISC_FEATURE - Xaa is 2,4-dichloro-l-phenylalanine
  SITE 7: note = MISC_FEATURE - Xaa is 4-(R)-hydroxy-l-proline
  SITE 9: note = MISC_FEATURE - Xaa is l-norvaline
  SITE 10: note = MISC_FEATURE - NH2 attached to Cys
CXXYXPXIXC

SEQ ID NO: 186 - protein, 10 aa, synthetic construct
  REGION 1..10: note = synthetic
  SITE 1: note = MISC_FEATURE - pentanoic acid attached to Cys
  REGION 1..10: note = MISC_FEATURE - cycle formed
  SITE 2: note = MISC_FEATURE - Xaa is l-Citrulline
  SITE 3: note = MISC_FEATURE - Xaa is l-lysine DOTA conjugate
  SITE 7: note = MISC_FEATURE - Xaa is N-methyl-l-alanine
  SITE 9: note = MISC_FEATURE - Xaa is l-norvaline
  SITE 10: note = MISC_FEATURE - NH2 attached to Cys
CXXYFPXIXC

SEQ ID NO: 187 - protein, 10 aa, synthetic construct
  REGION 1..10: note = synthetic
  SITE 1: note = MISC_FEATURE - pentanoic acid attached to Cys
  REGION 1..10: note = MISC_FEATURE - cycle formed
  SITE 2: note = MISC_FEATURE - Xaa is l-Citrulline
  SITE 3: note = MISC_FEATURE - Xaa is l-lysine d-(+)-biotin conjugate
  SITE 7: note = MISC_FEATURE - Xaa is N -methyl-l-lysine
  SITE 9: note = MISC_FEATURE - Xaa is l-norvaline
  SITE 10: note = MISC_FEATURE - NH2 attached to Cys
CXXYFPXIXC

SEQ ID NO: 188 - protein, 12 aa, synthetic construct
  REGION 1..12: note = synthetic
  SITE 1: note = MISC_FEATURE - hexanoic acid attached to Thr
  REGION 3..12: note = MISC_FEATURE - cycle formed
  SITE 12: note = MISC_FEATURE - NH2 attached to Cys
TLCDLYFPAILC

SEQ ID NO: 189 - protein, 10 aa, synthetic construct
  REGION 1..10: note = synthetic
  SITE 1: note = MISC_FEATURE - isocaproic acid attached to Cys
  REGION 1..10: note = MISC_FEATURE - cycle formed
  SITE 2: note = MISC_FEATURE - Xaa is l-Citrulline
  SITE 7: note = MISC_FEATURE - Xaa is d-alanine
  SITE 10: note = MISC_FEATURE - NH2 attached to Cys
CXQYFAXILC

SEQ ID NO: 190 - protein, 10 aa, synthetic construct
  REGION 1..10: note = synthetic
  SITE 1: note = MISC_FEATURE - pentanoic acid attached to Cys
  REGION 1..10: note = MISC_FEATURE - cycle formed
  SITE 2: note = MISC_FEATURE - Xaa is l-Citrulline
  SITE 3: note = MISC_FEATURE - Xaa is l-lysine DOTA conjugate
  SITE 4: note = MISC_FEATURE - Xaa is 4-amino-l-phenylalanine
  SITE 7: note = MISC_FEATURE - Xaa is 4-(R)-hydroxy-l-proline
  SITE 9: note = MISC_FEATURE - Xaa is l-norvaline
  SITE 10: note = MISC_FEATURE - NH2 attached to Cys
CXXXFPXIXC

SEQ ID NO: 191 - protein, 10 aa, synthetic construct
  REGION 1..10: note = synthetic
  SITE 1: note = MISC_FEATURE - isocaproic acid attached to Cys
  REGION 1..10: note = MISC_FEATURE - cycle formed
  SITE 2: note = MISC_FEATURE - Xaa is l-Citrulline
  SITE 6: note = MISC_FEATURE - Xaa is (S)-oxazolidine-4-carboxylic acid
  SITE 7: note = MISC_FEATURE - Xaa is d-alanine
  SITE 10: note = MISC_FEATURE - NH2 attached to Cys
CXQYFXXILC

SEQ ID NO: 192 - protein, 10 aa, synthetic construct
  REGION 1..10: note = synthetic
  SITE 1: note = MISC_FEATURE - pentanoic acid attached to Cys
  REGION 1..10: note = MISC_FEATURE - cycle formed
  SITE 7: note = MISC_FEATURE - Xaa is d-norvaline
  SITE 9: note = MISC_FEATURE - Xaa is l-norvaline
  SITE 10: note = MISC_FEATURE - NH2 attached to Cys
CRQYFPXIXC

SEQ ID NO: 193 - protein, 12 aa, synthetic construct
  REGION 1..12: note = synthetic
  SITE 1: note = MISC_FEATURE - Acetyl attached to Asp
  REGION 3..12: note = MISC_FEATURE - cycle formed
  SITE 5: note = MISC_FEATURE - Xaa is l-norleucine
  SITE 12: note = MISC_FEATURE - NH2 attached to d-cysteine
  SITE 12: note = MISC_FEATURE - Xaa is d-cysteine
DLCRXYFPAILX

SEQ ID NO: 194 - protein, 10 aa, synthetic construct
  REGION 1..10: note = synthetic
  SITE 1: note = MISC_FEATURE - pentanoic acid attached to Cys
  REGION 1..10: note = MISC_FEATURE - cycle formed
  SITE 2: note = MISC_FEATURE - Xaa is l-Citrulline
  SITE 3: note = MISC_FEATURE - Xaa is l-lysine DOTA conjugate
  SITE 7: note = MISC_FEATURE - Xaa is 4-(R)-hydroxy-l-proline
  SITE 9: note = MISC_FEATURE - Xaa is l-norvaline
  SITE 10: note = MISC_FEATURE - NH2 attached to Cys
CXXHFPXIXC

SEQ ID NO: 195 - protein, 10 aa, synthetic construct
  REGION 1..10: note = synthetic
  SITE 1: note = MISC_FEATURE - pentanoic acid attached to Cys
  REGION 1..10: note = MISC_FEATURE - cycle formed
  SITE 2: note = MISC_FEATURE - Xaa is l-Citrulline
  SITE 3: note = MISC_FEATURE - Xaa is l-lysine DOTA conjugate
  SITE 7: note = MISC_FEATURE - Xaa is 4-(S)-Amino-l-proline
  SITE 9: note = MISC_FEATURE - Xaa is l-norvaline
  SITE 10: note = MISC_FEATURE - NH2 attached to Cys
CXXYFPXIXC

SEQ ID NO: 196 - protein, 10 aa, synthetic construct
  REGION 1..10: note = synthetic
  SITE 1: note = MISC_FEATURE - isocaproic acid attached to Cys
  REGION 1..10: note = MISC_FEATURE - cycle formed
  SITE 2: note = MISC_FEATURE - Xaa is l-Citrulline
  SITE 7: note = MISC_FEATURE - Xaa is d-alanine
  SITE 8: note = MISC_FEATURE - Xaa is l-cyclohexyl-alanine
  SITE 10: note = MISC_FEATURE - NH2 attached to Cys
CXQYFPXXLC

SEQ ID NO: 197 - protein, 10 aa, synthetic construct
  REGION 1..10: note = synthetic
  SITE 1: note = MISC_FEATURE - pentanoic acid attached to Cys
  REGION 1..10: note = MISC_FEATURE - cycle formed
  SITE 2: note = MISC_FEATURE - Xaa is l-Citrulline
  SITE 3: note = MISC_FEATURE - Xaa is l-lysine DOTA conjugate
  SITE 7: note = MISC_FEATURE - Xaa is N-methyl-l-glutamic acid
  SITE 9: note = MISC_FEATURE - Xaa is l-norvaline
  SITE 10: note = MISC_FEATURE - NH2 attached to Cys
CXXYFPXIXC

SEQ ID NO: 198 - protein, 10 aa, synthetic construct
  REGION 1..10: note = synthetic
  SITE 1: note = MISC_FEATURE - pentyl sulfonyl attached to Cys
  REGION 1..10: note = MISC_FEATURE - cycle formed
  SITE 7: note = MISC_FEATURE - Xaa is 4-(R)-hydroxy-l-proline
  SITE 9: note = MISC_FEATURE - Xaa is l-norvaline
  SITE 10: note = MISC_FEATURE - NH2 attached to Cys
CRQYFPXIXC

SEQ ID NO: 199 - protein, 10 aa, synthetic construct
  REGION 1..10: note = synthetic
  SITE 1: note = MISC_FEATURE - pentanoic acid attached to Cys
  REGION 1..10: note = MISC_FEATURE - cycle formed
  SITE 7: note = MISC_FEATURE - Xaa is d-serine
  SITE 9: note = MISC_FEATURE - Xaa is l-norvaline
  SITE 10: note = MISC_FEATURE - NH2 attached to Cys
CRQYFPXIXC

SEQ ID NO: 200 - protein, 10 aa, synthetic construct
  REGION 1..10: note = synthetic
  SITE 1: note = MISC_FEATURE - pentanoic acid attached to Cys
  REGION 1..10: note = MISC_FEATURE - cycle formed
  SITE 7: note = MISC_FEATURE - Xaa is (R)-2,3-diaminopropionic acid
  SITE 9: note = MISC_FEATURE - Xaa is l-norvaline
  SITE 10: note = MISC_FEATURE - NH2 attached to Cys
CRQYFPXIXC

SEQ ID NO: 201 - protein, 10 aa, synthetic construct
  REGION 1..10: note = synthetic
  SITE 1: note = MISC_FEATURE - pentanoic acid attached to Cys
  REGION 1..10: note = MISC_FEATURE - cycle formed
  SITE 2: note = MISC_FEATURE - Xaa is l-Citrulline
  SITE 3: note = MISC_FEATURE - Xaa is l-lysine In(III) DOTA conjugate
  SITE 5: note = MISC_FEATURE - Xaa is 3-pyridyl-alanine
  SITE 7: note = MISC_FEATURE - Xaa is 4-(R)-hydroxy-l-proline
  SITE 9: note = MISC_FEATURE - Xaa is l-norvaline
  SITE 10: note = MISC_FEATURE - NH2 attached to Cys
CXXYXPXIXC

SEQ ID NO: 202 - protein, 10 aa, synthetic construct
  REGION 1..10: note = synthetic
  SITE 1: note = MISC_FEATURE - isocaproic acid attached to Cys
  REGION 1..10: note = MISC_FEATURE - cycle formed
  SITE 2: note = MISC_FEATURE - Xaa is l-Citrulline
  SITE 5: note = MISC_FEATURE - Xaa is 4-chloro-l-phenylalanine
  SITE 7: note = MISC_FEATURE - Xaa is d-alanine
  SITE 10: note = MISC_FEATURE - NH2 attached to Cys
CXQYXPXILC

SEQ ID NO: 203 - protein, 10 aa, synthetic construct
  REGION 1..10: note = synthetic
  SITE 1: note = MISC_FEATURE - N,N-dimethyl -alanine attached to Cys
  REGION 1..10: note = MISC_FEATURE - cycle formed
  SITE 2: note = MISC_FEATURE - Xaa is l-Citrulline
  SITE 7: note = MISC_FEATURE - Xaa is d-alanine
  SITE 10: note = MISC_FEATURE - NH2 attached to Cys
CXQYFPXILC

SEQ ID NO: 204 - protein, 11 aa, synthetic construct
  REGION 1..11: note = synthetic
  SITE 1: note = MISC_FEATURE - Acetyl attached to Gly
  REGION 2..11: note = MISC_FEATURE - cycle formed
  SITE 3: note = MISC_FEATURE - Xaa is l-Citrulline
  SITE 8: note = MISC_FEATURE - Xaa is d-alanine
  SITE 11: note = MISC_FEATURE - NH2 attached to Cys
GCXQYFPXILC

SEQ ID NO: 205 - protein, 10 aa, synthetic construct
  REGION 1..10: note = synthetic
  SITE 1: note = MISC_FEATURE - pentanoic acid attached to Cys
  REGION 1..10: note = MISC_FEATURE - cycle formed
  SITE 3: note = MISC_FEATURE - Xaa is l-lysine Lu(III) DOTA conjugate
  SITE 7: note = MISC_FEATURE - Xaa is 4-(R)-hydroxy-l-proline
  SITE 9: note = MISC_FEATURE - Xaa is l-norvaline
  SITE 10: note = MISC_FEATURE - NH2 attached to Cys
CNXYFPXIXC

SEQ ID NO: 206 - protein, 10 aa, synthetic construct
  REGION 1..10: note = synthetic
  SITE 1: note = MISC_FEATURE - pentanoic acid attached to Cys
  REGION 1..10: note = MISC_FEATURE - cycle formed
  SITE 2: note = MISC_FEATURE - Xaa is l-Citrulline
  SITE 3: note = MISC_FEATURE - Xaa is l-lysine DOTA conjugate
  SITE 4: note = MISC_FEATURE - Xaa is (S)-4-pyridyl-alanine
  SITE 7: note = MISC_FEATURE - Xaa is 4-(R)-hydroxy-l-proline
  SITE 9: note = MISC_FEATURE - Xaa is l-norvaline
  SITE 10: note = MISC_FEATURE - NH2 attached to Cys
CXXXFPXIXC

SEQ ID NO: 207 - protein, 10 aa, synthetic construct
  REGION 1..10: note = synthetic
  SITE 1: note = MISC_FEATURE - pentanoic acid attached to Cys
  REGION 1..10: note = MISC_FEATURE - cycle formed
  SITE 6: note = MISC_FEATURE - Xaa is N-methyl-l-norleucine
  SITE 7: note = MISC_FEATURE - Xaa is 4-(R)-hydroxy-l-proline
  SITE 9: note = MISC_FEATURE - Xaa is l-norvaline
  SITE 10: note = MISC_FEATURE - NH2 attached to Cys
CRQYFXXIXC

SEQ ID NO: 208 - protein, 10 aa, synthetic construct
  REGION 1..10: note = synthetic
  SITE 1: note = MISC_FEATURE - isocaproic acid attached to Cys
  REGION 1..10: note = MISC_FEATURE - cycle formed
  SITE 2: note = MISC_FEATURE - Xaa is l-Citrulline
  SITE 7: note = MISC_FEATURE - Xaa is d-alanine
  SITE 10: note = MISC_FEATURE - NH2 attached to Cys
CXQYFPXILC

SEQ ID NO: 209 - protein, 10 aa, synthetic construct
  REGION 1..10: note = synthetic
  SITE 1: note = MISC_FEATURE - isocaproic acid attached to Cys
  REGION 1..10: note = MISC_FEATURE - cycle formed
  SITE 2: note = MISC_FEATURE - Xaa is l-Citrulline
  SITE 7: note = MISC_FEATURE - Xaa is d-alanine
  SITE 10: note = MISC_FEATURE - NH2 attached to Cys
CXAYFPXILC

SEQ ID NO: 210 - protein, 10 aa, synthetic construct
  REGION 1..10: note = synthetic
  SITE 1: note = MISC_FEATURE - isocaproic acid attached to Cys
  REGION 1..10: note = MISC_FEATURE - cycle formed
  SITE 2: note = MISC_FEATURE - Xaa is l-Citrulline
  SITE 7: note = MISC_FEATURE - Xaa is d-alanine
  SITE 8: note = MISC_FEATURE - Xaa is N-methyl-l-isoleucine
  SITE 10: note = MISC_FEATURE - NH2 attached to Cys
CXQYFPXXLC

SEQ ID NO: 211 - protein, 12 aa, synthetic construct
  REGION 1..12: note = synthetic
  SITE 1: note = MISC_FEATURE - Acetyl attached to Asp
  REGION 3..12: note = MISC_FEATURE - cycle formed
  SITE 12: note = MISC_FEATURE - NH2 attached to Cys
DLCRMYFPAILC

SEQ ID NO: 212 - protein, 10 aa, synthetic construct
  REGION 1..10: note = synthetic
  SITE 1: note = MISC_FEATURE - pentanoic acid attached to Cys
  REGION 1..10: note = MISC_FEATURE - cycle formed
  SITE 3: note = MISC_FEATURE - Xaa is l-lysine DOTA conjugate
  SITE 7: note = MISC_FEATURE - Xaa is 4-(R)-hydroxy-l-proline
  SITE 9: note = MISC_FEATURE - Xaa is l-norvaline
  SITE 10: note = MISC_FEATURE - NH2 attached to Cys
CSXYFPXIXC

SEQ ID NO: 213 - protein, 10 aa, synthetic construct
  REGION 1..10: note = synthetic
  SITE 1: note = MISC_FEATURE - isocaproic acid attached to Cys
  REGION 1..10: note = MISC_FEATURE - cycle formed
  SITE 2: note = MISC_FEATURE - Xaa is l-Citrulline
  SITE 7: note = MISC_FEATURE - Xaa is d-alanine
  SITE 10: note = MISC_FEATURE - NH2 attached to Cys
CXQYYPXILC

SEQ ID NO: 214 - protein, 10 aa, synthetic construct
  REGION 1..10: note = synthetic
  SITE 1: note = MISC_FEATURE - pentanoic acid attached to Cys
  REGION 1..10: note = MISC_FEATURE - cycle formed
  SITE 9: note = MISC_FEATURE - Xaa is l-norvaline
  SITE 10: note = MISC_FEATURE - NH2 attached to Cys
CRQYFPDIXC

SEQ ID NO: 215 - protein, 10 aa, synthetic construct
  REGION 1..10: note = synthetic
  SITE 1: note = MISC_FEATURE - isocaproic acid attached to Cys
  REGION 1..10: note = MISC_FEATURE - cycle formed
  SITE 2: note = MISC_FEATURE - Xaa is l-Citrulline
  SITE 7: note = MISC_FEATURE - Xaa is d-alanine
  SITE 9: note = MISC_FEATURE - Xaa is l-norleucine
  SITE 10: note = MISC_FEATURE - NH2 attached to Cys
CXQYFPXIXC

SEQ ID NO: 216 - protein, 10 aa, synthetic construct
  REGION 1..10: note = synthetic
  SITE 1: note = MISC_FEATURE - n-butyl-carbamoyl attached to Cys
  REGION 1..10: note = MISC_FEATURE - cycle formed
  SITE 2: note = MISC_FEATURE - Xaa is l-Citrulline
  SITE 3: note = MISC_FEATURE - Xaa is l-lysine DOTA conjugate
  SITE 7: note = MISC_FEATURE - Xaa is 4-(R)-hydroxy-l-proline
  SITE 9: note = MISC_FEATURE - Xaa is l-norvaline
  SITE 10: note = MISC_FEATURE - NH2 attached to Cys
CXXYFPXIXC

SEQ ID NO: 217 - protein, 14 aa, synthetic construct
  REGION 1..14: note = synthetic
  SITE 1: note = MISC_FEATURE - 2,2 ,2 ,2 -(1,4,7,10-Tetraazacyclododecane-1,4,7,10-tetrayl)tetraacetic acid attached to 1,13-diamino-4,7,10-trioxatridecan-succinamic acid
  SITE 1: note = MISC_FEATURE - Xaa is 1,13-diamino-4,7,10-trioxatridecan-succinamic acid
  SITE 2: note = MISC_FEATURE - Xaa is l-norleucine
  REGION 5..14: note = MISC_FEATURE - cycle formed
  SITE 14: note = MISC_FEATURE - NH2 attached to Cys
XXDLCRMYFPAILC

SEQ ID NO: 218 - protein, 10 aa, synthetic construct
  REGION 1..10: note = synthetic
  SITE 1: note = MISC_FEATURE - pentanoic acid attached to Cys
  REGION 1..10: note = MISC_FEATURE - cycle formed
  SITE 2: note = MISC_FEATURE - Xaa is l-Citrulline
  SITE 3: note = MISC_FEATURE - Xaa is l-lysine Lu(III) DOTA conjugate
  SITE 7: note = MISC_FEATURE - Xaa is N-methyl-glycine
  SITE 9: note = MISC_FEATURE - Xaa is l-norvaline
  SITE 10: note = MISC_FEATURE - NH2 attached to Cys
CXXYFPXIXC

SEQ ID NO: 219 - protein, 10 aa, synthetic construct
  REGION 1..10: note = synthetic
  SITE 1: note = MISC_FEATURE - isocaproic acid attached to Cys
  REGION 1..10: note = MISC_FEATURE - cycle formed
  SITE 2: note = MISC_FEATURE - Xaa is l-Citrulline
  SITE 7: note = MISC_FEATURE - Xaa is d-alanine
  SITE 8: note = MISC_FEATURE - Xaa is l-cyclopentyl-glycine
  SITE 10: note = MISC_FEATURE - NH2 attached to Cys
CXQYFPXXLC

SEQ ID NO: 220 - protein, 10 aa, synthetic construct
  REGION 1..10: note = synthetic
  SITE 1: note = MISC_FEATURE - pentanoic acid attached to Cys
  REGION 1..10: note = MISC_FEATURE - cycle formed
  SITE 2: note = MISC_FEATURE - Xaa is l-Citrulline
  SITE 3: note = MISC_FEATURE - Xaa is l-lysine Lu(III) DOTA conjugate
  SITE 4: note = MISC_FEATURE - Xaa is l-4-guanidino-phenylalanine
  SITE 7: note = MISC_FEATURE - Xaa is 4-(R)-hydroxy-l-proline
  SITE 9: note = MISC_FEATURE - Xaa is l-norvaline
  SITE 10: note = MISC_FEATURE - NH2 attached to Cys
CXXXFPXIXC

SEQ ID NO: 221 - protein, 12 aa, synthetic construct
  REGION 1..12: note = synthetic
  SITE 1: note = MISC_FEATURE - hexanoic acid attached to Asp
  REGION 3..12: note = MISC_FEATURE - cycle formed
  SITE 9: note = MISC_FEATURE - Xaa is l-lysine DOTA conjugate
  SITE 12: note = MISC_FEATURE - NH2 attached to Cys
DLCRMYFPXILC

SEQ ID NO: 222 - protein, 10 aa, synthetic construct
  REGION 1..10: note = synthetic
  SITE 1: note = MISC_FEATURE - pentanoic acid attached to Cys
  REGION 1..10: note = MISC_FEATURE - cycle formed
  SITE 2: note = MISC_FEATURE - Xaa is l-Citrulline
  SITE 3: note = MISC_FEATURE - Xaa is l-lysine Lu(III) DOTA conjugate
  SITE 4: note = MISC_FEATURE - Xaa is 4-nitro-l-phenylalanine
  SITE 7: note = MISC_FEATURE - Xaa is 4-(R)-hydroxy-l-proline
  SITE 9: note = MISC_FEATURE - Xaa is l-norvaline
  SITE 10: note = MISC_FEATURE - NH2 attached to Cys
CXXXFPXIXC

SEQ ID NO: 223 - protein, 11 aa, synthetic construct
  REGION 1..11: note = synthetic
  SITE 1: note = MISC_FEATURE - pentanoic acid attached to Cys
  REGION 1..10: note = MISC_FEATURE - cycle formed
  SITE 2: note = MISC_FEATURE - Xaa is l-Citrulline
  SITE 7: note = MISC_FEATURE - Xaa is 4-(R)-hydroxy-l-proline
  SITE 9: note = MISC_FEATURE - Xaa is l-norvaline
  SITE 11: note = MISC_FEATURE - NH2 attached to -alanine
  SITE 11: note = MISC_FEATURE - Xaa is -alanine
CXQYFPXIXCX

SEQ ID NO: 224 - protein, 10 aa, synthetic construct
  REGION 1..10: note = synthetic
  SITE 1: note = MISC_FEATURE - isocaproic acid attached to Cys
  REGION 1..10: note = MISC_FEATURE - cycle formed
  SITE 2: note = MISC_FEATURE - Xaa is l-Citrulline
  SITE 6: note = MISC_FEATURE - Xaa is (2S,4S)-4-fluoro-pyrrolidine-2-carboxylic acid
  SITE 7: note = MISC_FEATURE - Xaa is d-alanine
  SITE 10: note = MISC_FEATURE - NH2 attached to Cys
CXQYFXXILC

SEQ ID NO: 225 - protein, 10 aa, synthetic construct
  REGION 1..10: note = synthetic
  SITE 1: note = MISC_FEATURE - pentanoic acid attached to Cys
  REGION 1..10: note = MISC_FEATURE - cycle formed
  SITE 2: note = MISC_FEATURE - Xaa is l-Citrulline
  SITE 3: note = MISC_FEATURE - Xaa is l-lysine In(III) DOTA conjugate
  SITE 5: note = MISC_FEATURE - Xaa is 4-chloro-l-phenylalanine
  SITE 7: note = MISC_FEATURE - Xaa is 4-(R)-hydroxy-l-proline
  SITE 9: note = MISC_FEATURE - Xaa is l-norvaline
  SITE 10: note = MISC_FEATURE - NH2 attached to Cys
CXXYXPXIXC

SEQ ID NO: 226 - protein, 10 aa, synthetic construct
  REGION 1..10: note = synthetic
  SITE 1: note = MISC_FEATURE - benzoic acid attached to Cys
  REGION 1..10: note = MISC_FEATURE - cycle formed
  SITE 7: note = MISC_FEATURE - Xaa is 4-(R)-hydroxy-l-proline
  SITE 9: note = MISC_FEATURE - Xaa is l-norvaline
  SITE 10: note = MISC_FEATURE - NH2 attached to Cys
CRQYFPXIXC

SEQ ID NO: 227 - protein, 10 aa, synthetic construct
  REGION 1..10: note = synthetic
  SITE 1: note = MISC_FEATURE - isocaproic acid attached to Cys
  REGION 1..10: note = MISC_FEATURE - cycle formed
  SITE 2: note = MISC_FEATURE - Xaa is l-Citrulline
  SITE 7: note = MISC_FEATURE - Xaa is d-arginine
  SITE 10: note = MISC_FEATURE - NH2 attached to Cys
CXQYFPXILC

SEQ ID NO: 228 - protein, 10 aa, synthetic construct
  REGION 1..10: note = synthetic
  SITE 1: note = MISC_FEATURE - n-butyloxycarbonyl attached to Cys
  REGION 1..10: note = MISC_FEATURE - cycle formed
  SITE 6: note = MISC_FEATURE - Xaa is (2S,4S)-4-fluoro-pyrrolidine-2-carboxylic acid
  SITE 7: note = MISC_FEATURE - Xaa is 4-(R)-hydroxy-l-proline
  SITE 9: note = MISC_FEATURE - Xaa is l-norvaline
  SITE 10: note = MISC_FEATURE - NH2 attached to Cys
CTQYFXXIXC

SEQ ID NO: 229 - protein, 10 aa, synthetic construct
  REGION 1..10: note = synthetic
  SITE 1: note = MISC_FEATURE - glutaric acid as linker attached to Cys
  REGION 1..10: note = MISC_FEATURE - cycle formed
  SITE 2: note = MISC_FEATURE - Xaa is l-Citrulline
  SITE 7: note = MISC_FEATURE - Xaa is d-alanine
  SITE 10: note = MISC_FEATURE - NH2 attached to Cys
CXQYFPXILC

SEQ ID NO: 230 - protein, 10 aa, synthetic construct
  REGION 1..10: note = synthetic
  SITE 1: note = MISC_FEATURE - pentanoic acid attached to Cys
  REGION 1..10: note = MISC_FEATURE - cycle formed
  SITE 2: note = MISC_FEATURE - Xaa is l-Citrulline
  SITE 3: note = MISC_FEATURE - Xaa is l-lysine DOTA conjugate
  SITE 5: note = MISC_FEATURE - Xaa is l-thienylalanine
  SITE 7: note = MISC_FEATURE - Xaa is 4-(R)-hydroxy-l-proline
  SITE 9: note = MISC_FEATURE - Xaa is l-norvaline
  SITE 10: note = MISC_FEATURE - NH2 attached to Cys
CXXYXPXIXC

SEQ ID NO: 231 - protein, 10 aa, synthetic construct
  REGION 1..10: note = synthetic
  SITE 1: note = MISC_FEATURE - pentanoic acid attached to Cys
  REGION 1..10: note = MISC_FEATURE - cycle formed
  SITE 7: note = MISC_FEATURE - Xaa is 4-(R)-hydroxy-l-proline
  SITE 9: note = MISC_FEATURE - Xaa is l-norvaline
  SITE 10: note = MISC_FEATURE - NH2 attached to Cys
CPQYFPXIXC

SEQ ID NO: 232 - protein, 10 aa, synthetic construct
  REGION 1..10: note = synthetic
  SITE 1: note = MISC_FEATURE - pentanoic acid attached to Cys
  REGION 1..10: note = MISC_FEATURE - cycle formed
  SITE 2: note = MISC_FEATURE - Xaa is l-Citrulline
  SITE 7: note = MISC_FEATURE - Xaa is d-alanine
  SITE 10: note = MISC_FEATURE - NH2 attached to Cys
CXQYFPXILC

SEQ ID NO: 233 - protein, 12 aa, synthetic construct
  REGION 1..12: note = synthetic
  SITE 1: note = MISC_FEATURE - hexanoic acid attached to Asp
  REGION 3..12: note = MISC_FEATURE - cycle formed
  SITE 12: note = MISC_FEATURE - NH2 attached to Cys
DLCRMYFPAILC

SEQ ID NO: 234 - protein, 10 aa, synthetic construct
  REGION 1..10: note = synthetic
  SITE 1: note = MISC_FEATURE - isocaproic acid attached to Cys
  REGION 1..10: note = MISC_FEATURE - cycle formed
  SITE 2: note = MISC_FEATURE - Xaa is d-citrulline
  SITE 7: note = MISC_FEATURE - Xaa is d-alanine
  SITE 10: note = MISC_FEATURE - NH2 attached to Cys
CXQYFPXILC

SEQ ID NO: 235 - protein, 10 aa, synthetic construct
  REGION 1..10: note = synthetic
  SITE 1: note = MISC_FEATURE - pentanoic acid attached to Cys
  REGION 1..10: note = MISC_FEATURE - cycle formed
  SITE 2: note = MISC_FEATURE - Xaa is l-Citrulline
  SITE 3: note = MISC_FEATURE - Xaa is l-lysine DOTA conjugate
  SITE 6: note = MISC_FEATURE - Xaa is (2S,4S)-4-fluoro-pyrrolidine-2-carboxylic acid
  SITE 7: note = MISC_FEATURE - Xaa is 4-(R)-hydroxy-l-proline
  SITE 9: note = MISC_FEATURE - Xaa is l-norvaline
  SITE 10: note = MISC_FEATURE - NH2 attached to Cys
CXXYFXXIXC

SEQ ID NO: 236 - protein, 10 aa, synthetic construct
  REGION 1..10: note = synthetic
  SITE 1: note = MISC_FEATURE - pentanoic acid attached to Cys
  REGION 1..10: note = MISC_FEATURE - cycle formed
  SITE 4: note = MISC_FEATURE - Xaa is l-homophenylalanine
  SITE 7: note = MISC_FEATURE - Xaa is 4-(R)-hydroxy-l-proline
  SITE 9: note = MISC_FEATURE - Xaa is l-norvaline
  SITE 10: note = MISC_FEATURE - NH2 attached to Cys
CRQXFPXIXC

SEQ ID NO: 237 - protein, 10 aa, synthetic construct
  REGION 1..10: note = synthetic
  SITE 1: note = MISC_FEATURE - isocaproic acid attached to Cys
  REGION 1..10: note = MISC_FEATURE - cycle formed
  SITE 7: note = MISC_FEATURE - Xaa is d-lysine DOTA conjugate
  SITE 10: note = MISC_FEATURE - NH2 attached to Cys
CRQYFPXILC

SEQ ID NO: 238 - protein, 10 aa, synthetic construct
  REGION 1..10: note = synthetic
  SITE 1: note = MISC_FEATURE - n-butyloxycarbonyl attached to Cys
  REGION 1..10: note = MISC_FEATURE - cycle formed
  SITE 3: note = MISC_FEATURE - Xaa is l-lysine DOTA conjugate
  SITE 6: note = MISC_FEATURE - Xaa is (2S,4S)-4-fluoro-pyrrolidine-2-carboxylic acid
  SITE 7: note = MISC_FEATURE - Xaa is 4-(R)-hydroxy-l-proline
  SITE 9: note = MISC_FEATURE - Xaa is l-homoserine
  SITE 10: note = MISC_FEATURE - NH2 attached to Cys
CTXYFXXIXC

SEQ ID NO: 239 - protein, 10 aa, synthetic construct
  REGION 1..10: note = synthetic
  SITE 1: note = MISC_FEATURE - n-butyloxycarbonyl attached to Cys
  REGION 1..10: note = MISC_FEATURE - cycle formed
  SITE 2: note = MISC_FEATURE - Xaa is l-Citrulline
  SITE 3: note = MISC_FEATURE - Xaa is l-lysine Lu(III) DOTA conjugate
  SITE 5: note = MISC_FEATURE - Xaa is 4-chloro-l-phenylalanine
  SITE 6: note = MISC_FEATURE - Xaa is (2S,4S)-4-fluoro-pyrrolidine-2-carboxylic acid
  SITE 7: note = MISC_FEATURE - Xaa is 4-(R)-hydroxy-l-proline
  SITE 9: note = MISC_FEATURE - Xaa is l-norvaline
  SITE 10: note = MISC_FEATURE - NH2 attached to Cys
CXXYXXXIXC

SEQ ID NO: 240 - protein, 10 aa, synthetic construct
  REGION 1..10: note = synthetic
  SITE 1: note = MISC_FEATURE - pentanoic acid attached to Cys
  REGION 1..10: note = MISC_FEATURE - cycle formed
  SITE 7: note = MISC_FEATURE - Xaa is 4-(R)-hydroxy-l-proline
  SITE 8: note = MISC_FEATURE - Xaa is l-neopentyl-glycine
  SITE 9: note = MISC_FEATURE - Xaa is l-norvaline
  SITE 10: note = MISC_FEATURE - NH2 attached to Cys
CRQYFPXXXC

SEQ ID NO: 241 - protein, 11 aa, synthetic construct
  REGION 1..11: note = synthetic
  SITE 1: note = MISC_FEATURE - 2,2 ,2 ,2 -(1,4,7,10-Tetraazacyclododecane-1,4,7,10-tetrayl)tetraacetic acid attached to Leu
  REGION 2..11: note = MISC_FEATURE - cycle formed
  SITE 3: note = MISC_FEATURE - Xaa is l-Citrulline
  SITE 8: note = MISC_FEATURE - Xaa is 4-(R)-hydroxy-l-proline
  SITE 10: note = MISC_FEATURE - Xaa is N-methyl-l-leucine
  SITE 11: note = MISC_FEATURE - NH2 attached to Cys
LCXQYFPXIXC

SEQ ID NO: 242 - protein, 11 aa, synthetic construct
  REGION 1..11: note = synthetic
  SITE 1: note = MISC_FEATURE - Acetyl attached to l-cyclohexyl-alanine
  SITE 1: note = MISC_FEATURE - Xaa is l-cyclohexyl-alanine
  REGION 2..11: note = MISC_FEATURE - cycle formed
  SITE 8: note = MISC_FEATURE - Xaa is 4-(R)-hydroxy-l-proline
  SITE 10: note = MISC_FEATURE - Xaa is l-norvaline
  SITE 11: note = MISC_FEATURE - NH2 attached to Cys
XCRQYFPXIXC

SEQ ID NO: 243 - protein, 10 aa, synthetic construct
  REGION 1..10: note = synthetic
  SITE 1: note = MISC_FEATURE - pentanoic acid attached to Cys
  REGION 1..10: note = MISC_FEATURE - cycle formed
  SITE 4: note = MISC_FEATURE - Xaa is l-cyclohexyl-alanine
  SITE 7: note = MISC_FEATURE - Xaa is 4-(R)-hydroxy-l-proline
  SITE 9: note = MISC_FEATURE - Xaa is l-norvaline
  SITE 10: note = MISC_FEATURE - NH2 attached to Cys
CRQXFPXIXC

SEQ ID NO: 244 - protein, 10 aa, synthetic construct
  REGION 1..10: note = synthetic
  SITE 1: note = MISC_FEATURE - isocaproic acid attached to Cys
  REGION 1..10: note = MISC_FEATURE - cycle formed
  SITE 2: note = MISC_FEATURE - Xaa is l-Citrulline
  SITE 6: note = MISC_FEATURE - Xaa is l-thiazolidine-4-carboxylic acid
  SITE 7: note = MISC_FEATURE - Xaa is d-alanine
  SITE 10: note = MISC_FEATURE - NH2 attached to Cys
CXQYFXXILC

SEQ ID NO: 245 - protein, 10 aa, synthetic construct
  REGION 1..10: note = synthetic
  SITE 1: note = MISC_FEATURE - pentanoic acid attached to Cys
  REGION 1..10: note = MISC_FEATURE - cycle formed
  SITE 2: note = MISC_FEATURE - Xaa is l-homoarginine
  SITE 3: note = MISC_FEATURE - Xaa is l-lysine Gd (III) DOTA conjugate
  SITE 7: note = MISC_FEATURE - Xaa is 4-(R)-hydroxy-l-proline
  SITE 9: note = MISC_FEATURE - Xaa is l-norvaline
  SITE 10: note = MISC_FEATURE - NH2 attached to Cys
CXXYFPXIXC

SEQ ID NO: 246 - protein, 10 aa, synthetic construct
  REGION 1..10: note = synthetic
  SITE 1: note = MISC_FEATURE - pentanoic acid attached to Cys
  REGION 1..10: note = MISC_FEATURE - cycle formed
  SITE 2: note = MISC_FEATURE - Xaa is l-Citrulline
  SITE 3: note = MISC_FEATURE - Xaa is l-lysine DOTA conjugate
  SITE 7: note = MISC_FEATURE - Xaa is (2S,4R)-4-amino-1-pyrrolidin-2-carboxylic acid
  SITE 9: note = MISC_FEATURE - Xaa is l-norvaline
  SITE 10: note = MISC_FEATURE - NH2 attached to Cys
CXXYFPXIXC

SEQ ID NO: 247 - protein, 10 aa, synthetic construct
  REGION 1..10: note = synthetic
  SITE 1: note = MISC_FEATURE - n-butyloxycarbonyl attached to Cys
  REGION 1..10: note = MISC_FEATURE - cycle formed
  SITE 3: note = MISC_FEATURE - Xaa is l-lysine DOTA conjugate
  SITE 5: note = MISC_FEATURE - Xaa is 4-cyano-l-phenylalanine
  SITE 6: note = MISC_FEATURE - Xaa is (2S,4S)-4-fluoro-pyrrolidine-2-carboxylic acid
  SITE 7: note = MISC_FEATURE - Xaa is 4-(R)-hydroxy-l-proline
  SITE 9: note = MISC_FEATURE - Xaa is l-norvaline
  SITE 10: note = MISC_FEATURE - NH2 attached to Cys
CTXYXXXIXC

SEQ ID NO: 248 - protein, 10 aa, synthetic construct
  REGION 1..10: note = synthetic
  SITE 1: note = MISC_FEATURE - pentanoic acid attached to Cys
  REGION 1..10: note = MISC_FEATURE - cycle formed
  SITE 7: note = MISC_FEATURE - Xaa is 4-(R)-hydroxy-l-proline
  SITE 9: note = MISC_FEATURE - Xaa is l-cyclopropyl alanine
  SITE 10: note = MISC_FEATURE - NH2 attached to Cys
CRQYFPXIXC

SEQ ID NO: 249 - protein, 10 aa, synthetic construct
  REGION 1..10: note = synthetic
  SITE 1: note = MISC_FEATURE - pentanoic acid attached to Cys
  REGION 1..10: note = MISC_FEATURE - cycle formed
  SITE 2: note = MISC_FEATURE - Xaa is l-Citrulline
  SITE 3: note = MISC_FEATURE - Xaa is l-lysine DOTA conjugate
  SITE 7: note = MISC_FEATURE - Xaa is 4-(R)-hydroxy-l-proline
  SITE 9: note = MISC_FEATURE - Xaa is l-O-methylserine
  SITE 10: note = MISC_FEATURE - NH2 attached to Cys
CXXYFPXIXC

SEQ ID NO: 250 - protein, 11 aa, synthetic construct
  REGION 1..11: note = synthetic
  SITE 1: note = MISC_FEATURE - Acetyl attached to Leu
  REGION 2..11: note = MISC_FEATURE - cycle formed
  SITE 11: note = MISC_FEATURE - NH2 attached to Cys
LCRQYFPAILC

SEQ ID NO: 251 - protein, 10 aa, synthetic construct
  REGION 1..10: note = synthetic
  SITE 1: note = MISC_FEATURE - isocaproic acid attached to Cys
  REGION 1..10: note = MISC_FEATURE - cycle formed
  SITE 2: note = MISC_FEATURE - Xaa is l-Citrulline
  SITE 3: note = MISC_FEATURE - Xaa is l-lysine DOTA conjugate
  SITE 10: note = MISC_FEATURE - NH2 attached to Cys
CXXYFPPILC

SEQ ID NO: 252 - protein, 10 aa, synthetic construct
  REGION 1..10: note = synthetic
  SITE 1: note = MISC_FEATURE - pentanoic acid attached to Cys
  REGION 1..10: note = MISC_FEATURE - cycle formed
  SITE 2: note = MISC_FEATURE - Xaa is l-ornithine mPEG12 conjugate
  SITE 3: note = MISC_FEATURE - Xaa is l-lysine DOTA conjugate
  SITE 7: note = MISC_FEATURE - Xaa is 4-(R)-hydroxy-l-proline
  SITE 9: note = MISC_FEATURE - Xaa is l-norvaline
  SITE 10: note = MISC_FEATURE - NH2 attached to Cys
CXXYFPXIXC

SEQ ID NO: 253 - protein, 10 aa, synthetic construct
  REGION 1..10: note = synthetic
  SITE 1: note = MISC_FEATURE - pentanoic acid attached to Cys
  REGION 1..10: note = MISC_FEATURE - cycle formed
  SITE 2: note = MISC_FEATURE - Xaa is l-Citrulline
  SITE 3: note = MISC_FEATURE - Xaa is l-lysine DOTA conjugate
  SITE 7: note = MISC_FEATURE - Xaa is N-methyl-d-alanine
  SITE 9: note = MISC_FEATURE - Xaa is l-norvaline
  SITE 10: note = MISC_FEATURE - NH2 attached to Cys
CXXYFPXIXC

SEQ ID NO: 254 - protein, 10 aa, synthetic construct
  REGION 1..10: note = synthetic
  SITE 1: note = MISC_FEATURE - pentanoic acid attached to Cys
  REGION 1..10: note = MISC_FEATURE - cycle formed
  SITE 7: note = MISC_FEATURE - Xaa is 4-(R)-hydroxy-l-proline
  SITE 9: note = MISC_FEATURE - Xaa is l-norvaline
  SITE 10: note = MISC_FEATURE - NH2 attached to Cys
CRQYFPXKXC

SEQ ID NO: 255 - protein, 10 aa, synthetic construct
  REGION 1..10: note = synthetic
  SITE 1: note = MISC_FEATURE - pentanoic acid attached to Cys
  REGION 1..10: note = MISC_FEATURE - cycle formed
  SITE 2: note = MISC_FEATURE - Xaa is -glutamyl AGLU conjugate
  SITE 7: note = MISC_FEATURE - Xaa is 4-(R)-hydroxy-l-proline
  SITE 9: note = MISC_FEATURE - Xaa is l-norvaline
  SITE 10: note = MISC_FEATURE - NH2 attached to Cys
CXQYFPXIXC

SEQ ID NO: 256 - protein, 10 aa, synthetic construct
  REGION 1..10: note = synthetic
  SITE 1: note = MISC_FEATURE - pentanoic acid attached to Cys
  REGION 1..10: note = MISC_FEATURE - cycle formed
  SITE 6: note = MISC_FEATURE - Xaa is (2S,3aS,7aS)- octahydroindolecarboxylic acid
  SITE 7: note = MISC_FEATURE - Xaa is 4-(R)-hydroxy-l-proline
  SITE 9: note = MISC_FEATURE - Xaa is l-norvaline
  SITE 10: note = MISC_FEATURE - NH2 attached to Cys
CRQYFXXIXC

SEQ ID NO: 257 - protein, 10 aa, synthetic construct
  REGION 1..10: note = synthetic
  SITE 1: note = MISC_FEATURE - pentanoic acid attached to Cys
  REGION 1..10: note = MISC_FEATURE - cycle formed
  SITE 3: note = MISC_FEATURE - Xaa is l-lysine DOTA conjugate
  SITE 6: note = MISC_FEATURE - Xaa is 4-(S)-hydroxy-l-proline
  SITE 7: note = MISC_FEATURE - Xaa is 4-(R)-hydroxy-l-proline
  SITE 9: note = MISC_FEATURE - Xaa is l-norvaline
  SITE 10: note = MISC_FEATURE - NH2 attached to Cys
CTXYFXXIXC

SEQ ID NO: 258 - protein, 10 aa, synthetic construct
  REGION 1..10: note = synthetic
  SITE 1: note = MISC_FEATURE - isocaproic acid attached to Cys
  REGION 1..10: note = MISC_FEATURE - cycle formed
  SITE 2: note = MISC_FEATURE - Xaa is l-Citrulline
  SITE 7: note = MISC_FEATURE - Xaa is Tap DOTA conjugate
  SITE 10: note = MISC_FEATURE - NH2 attached to Cys
CXQYFPXILC

SEQ ID NO: 259 - protein, 10 aa, synthetic construct
  REGION 1..10: note = synthetic
  SITE 1: note = MISC_FEATURE - pentanoic acid attached to (S)-2,4-diaminobutyric acid
  SITE 1: note = MISC_FEATURE - Xaa is (S)-2,4-diaminobutyric acid
  REGION 1..10: note = MISC_FEATURE - cycle formed
  SITE 7: note = MISC_FEATURE - Xaa is 4-(R)-hydroxy-l-proline
  SITE 9: note = MISC_FEATURE - Xaa is l-norvaline
  SITE 10: note = MISC_FEATURE - NH2 attached to Glu
XRQYFPXIXE

SEQ ID NO: 260 - protein, 10 aa, synthetic construct
  REGION 1..10: note = synthetic
  SITE 1: note = MISC_FEATURE - pentanoic acid attached to Cys
  REGION 1..10: note = MISC_FEATURE - cycle formed
  SITE 7: note = MISC_FEATURE - Xaa is 4-(R)-hydroxy-l-proline
  SITE 9: note = MISC_FEATURE - Xaa is l-norvaline
  SITE 10: note = MISC_FEATURE - NH2 attached to Cys
CLQYFPXIXC

SEQ ID NO: 261 - protein, 12 aa, synthetic construct
  REGION 1..12: note = synthetic
  SITE 1: note = MISC_FEATURE - Acetyl attached to Asp
  REGION 3..12: note = MISC_FEATURE - cycle formed
  SITE 4: note = MISC_FEATURE - Xaa is d-aspartic acid
  SITE 5: note = MISC_FEATURE - Xaa is l-lysine DOTA conjugate
  SITE 9: note = MISC_FEATURE - Xaa is d-alanine
  SITE 12: note = MISC_FEATURE - NH2 attached to Cys
DLCXXYFPXILC

SEQ ID NO: 262 - protein, 10 aa, synthetic construct
  REGION 1..10: note = synthetic
  SITE 1: note = MISC_FEATURE - isocaproic acid attached to Cys
  REGION 1..10: note = MISC_FEATURE - cycle formed
  SITE 2: note = MISC_FEATURE - Xaa is l-Citrulline
  SITE 4: note = MISC_FEATURE - Xaa is 3-pyridyl-alanine
  SITE 7: note = MISC_FEATURE - Xaa is d-alanine
  SITE 10: note = MISC_FEATURE - NH2 attached to Cys
CXQXFPXILC

SEQ ID NO: 263 - protein, 11 aa, synthetic construct
  REGION 1..11: note = synthetic
  SITE 1: note = MISC_FEATURE - Xaa is 5-aminopentanoic acid
  REGION 2..11: note = MISC_FEATURE - cycle formed
  SITE 3: note = MISC_FEATURE - Xaa is l-Citrulline
  SITE 8: note = MISC_FEATURE - Xaa is d-alanine
  SITE 11: note = MISC_FEATURE - NH2 attached to Cys
XCXQYFPXILC

SEQ ID NO: 264 - protein, 10 aa, synthetic construct
  REGION 1..10: note = synthetic
  SITE 1: note = MISC_FEATURE - pentanoic acid attached to Cys
  REGION 1..10: note = MISC_FEATURE - cycle formed
  SITE 4: note = MISC_FEATURE - Xaa is ortho-chloro-l-phenylalanine
  SITE 7: note = MISC_FEATURE - Xaa is 4-(R)-hydroxy-l-proline
  SITE 9: note = MISC_FEATURE - Xaa is l-norvaline
  SITE 10: note = MISC_FEATURE - NH2 attached to Cys
CRQXFPXIXC

SEQ ID NO: 265 - protein, 10 aa, synthetic construct
  REGION 1..10: note = synthetic
  SITE 1: note = MISC_FEATURE - pentanoic acid attached to Cys
  REGION 1..10: note = MISC_FEATURE - cycle formed
  SITE 2: note = MISC_FEATURE - Xaa is l-Citrulline
  SITE 3: note = MISC_FEATURE - Xaa is l-lysine DOTA conjugate
  SITE 10: note = MISC_FEATURE - NH2 attached to Cys
CXXYFPPILC

SEQ ID NO: 266 - protein, 10 aa, synthetic construct
  REGION 1..10: note = synthetic
  SITE 1: note = MISC_FEATURE - pentanoic acid attached to l-penicillamine
  SITE 1: note = MISC_FEATURE - Xaa is l-penicillamine
  REGION 1..10: note = MISC_FEATURE - cycle formed
  SITE 2: note = MISC_FEATURE - Xaa is l-Citrulline
  SITE 7: note = MISC_FEATURE - Xaa is 4-(R)-hydroxy-l-proline
  SITE 9: note = MISC_FEATURE - Xaa is l-norvaline
  SITE 10: note = MISC_FEATURE - NH2 attached to Cys
XXQYFPXIXC

SEQ ID NO: 267 - protein, 10 aa, synthetic construct
  REGION 1..10: note = synthetic
  SITE 1: note = MISC_FEATURE - pentanoic acid attached to Cys
  REGION 1..10: note = MISC_FEATURE - cycle formed
  SITE 2: note = MISC_FEATURE - Xaa is l-Citrulline
  SITE 3: note = MISC_FEATURE - Xaa is l-lysine DOTA conjugate
  SITE 5: note = MISC_FEATURE - Xaa is N-methyl-l-phenylalanine
  SITE 7: note = MISC_FEATURE - Xaa is 4-(R)-hydroxy-l-proline
  SITE 9: note = MISC_FEATURE - Xaa is l-norvaline
  SITE 10: note = MISC_FEATURE - NH2 attached to Cys
CXXYXPXIXC

SEQ ID NO: 268 - protein, 10 aa, synthetic construct
  REGION 1..10: note = synthetic
  SITE 1: note = MISC_FEATURE - pentanoic acid attached to Cys
  REGION 1..10: note = MISC_FEATURE - cycle formed
  SITE 2: note = MISC_FEATURE - Xaa is l-Citrulline
  SITE 3: note = MISC_FEATURE - Xaa is l-lysine DOTA conjugate
  SITE 4: note = MISC_FEATURE - Xaa is Levodopa / l-3,4-dihydroxyphenylalanine
  SITE 7: note = MISC_FEATURE - Xaa is 4-(R)-hydroxy-l-proline
  SITE 9: note = MISC_FEATURE - Xaa is l-norvaline
  SITE 10: note = MISC_FEATURE - NH2 attached to Cys
CXXXFPXIXC

SEQ ID NO: 269 - protein, 10 aa, synthetic construct
  REGION 1..10: note = synthetic
  SITE 1: note = MISC_FEATURE - pentanoic acid attached to Cys
  REGION 1..10: note = MISC_FEATURE - cycle formed
  SITE 7: note = MISC_FEATURE - Xaa is 4-(R)-hydroxy-l-proline
  SITE 9: note = MISC_FEATURE - Xaa is l-norvaline
  SITE 10: note = MISC_FEATURE - NH2 attached to Cys
CRQYFFXIXC

SEQ ID NO: 270 - protein, 10 aa, synthetic construct
  REGION 1..10: note = synthetic
  SITE 1: note = MISC_FEATURE - pentanoic acid attached to Cys
  REGION 1..10: note = MISC_FEATURE - cycle formed
  SITE 7: note = MISC_FEATURE - Xaa is 4-(R)-hydroxy-l-proline
  SITE 9: note = MISC_FEATURE - Xaa is l-norvaline
  SITE 10: note = MISC_FEATURE - NH2 attached to Cys
CRQWFPXIXC

SEQ ID NO: 271 - protein, 10 aa, synthetic construct
  REGION 1..10: note = synthetic
  SITE 1: note = MISC_FEATURE - isocaproic acid attached to Cys
  REGION 1..10: note = MISC_FEATURE - cycle formed
  SITE 2: note = MISC_FEATURE - Xaa is l-Citrulline
  SITE 7: note = MISC_FEATURE - Xaa is d-alanine
  SITE 10: note = MISC_FEATURE - NH2 attached to Cys
CXQYFPXIAC

SEQ ID NO: 272 - protein, 10 aa, synthetic construct
  REGION 1..10: note = synthetic
  SITE 1: note = MISC_FEATURE - pentanoic acid attached to Cys
  REGION 1..10: note = MISC_FEATURE - cycle formed
  SITE 2: note = MISC_FEATURE - Xaa is l-Citrulline
  SITE 3: note = MISC_FEATURE - Xaa is l-lysine DOTA conjugate
  SITE 6: note = MISC_FEATURE - Xaa is 4-(R)-hydroxy-l-proline
  SITE 7: note = MISC_FEATURE - Xaa is 4-(R)-hydroxy-l-proline
  SITE 9: note = MISC_FEATURE - Xaa is l-norvaline
  SITE 10: note = MISC_FEATURE - NH2 attached to Cys
CXXYFXXIXC

SEQ ID NO: 273 - protein, 10 aa, synthetic construct
  REGION 1..10: note = synthetic
  SITE 1: note = MISC_FEATURE - pentanoic acid attached to Cys
  REGION 1..10: note = MISC_FEATURE - cycle formed
  SITE 2: note = MISC_FEATURE - Xaa is l-Citrulline
  SITE 3: note = MISC_FEATURE - Xaa is l-lysine PEG12 In(III) DOTA conjugate
  SITE 7: note = MISC_FEATURE - Xaa is 4-(R)-hydroxy-l-proline
  SITE 9: note = MISC_FEATURE - Xaa is l-norvaline
  SITE 10: note = MISC_FEATURE - NH2 attached to Cys
CXXYFPXIXC

SEQ ID NO: 274 - protein, 10 aa, synthetic construct
  REGION 1..10: note = synthetic
  SITE 1: note = MISC_FEATURE - isocaproic acid attached to Cys
  REGION 1..10: note = MISC_FEATURE - cycle formed
  SITE 2: note = MISC_FEATURE - Xaa is l-Citrulline
  SITE 7: note = MISC_FEATURE - Xaa is d-alanine
  SITE 10: note = MISC_FEATURE - NH2 attached to Cys
CXQYFPXIIC

SEQ ID NO: 275 - protein, 12 aa, synthetic construct
  REGION 1..12: note = synthetic
  SITE 1: note = MISC_FEATURE - Acetyl attached to Asp
  REGION 3..12: note = MISC_FEATURE - cycle formed
  SITE 5: note = MISC_FEATURE - Xaa is l-norleucine
  SITE 9: note = MISC_FEATURE - Xaa is d-alanine
  SITE 12: note = MISC_FEATURE - NH2 attached to Cys
DLCRXYFPXILC

SEQ ID NO: 276 - protein, 10 aa, synthetic construct
  REGION 1..10: note = synthetic
  SITE 1: note = MISC_FEATURE - isocaproic acid attached to Cys
  REGION 1..10: note = MISC_FEATURE - cycle formed
  SITE 2: note = MISC_FEATURE - Xaa is l-Citrulline
  SITE 3: note = MISC_FEATURE - Xaa is N -methyl-l-glutamine
  SITE 7: note = MISC_FEATURE - Xaa is d-alanine
  SITE 10: note = MISC_FEATURE - NH2 attached to Cys
CXXYFPXILC

SEQ ID NO: 277 - protein, 10 aa, synthetic construct
  REGION 1..10: note = synthetic
  SITE 1: note = MISC_FEATURE - isocaproic acid attached to Cys
  REGION 1..10: note = MISC_FEATURE - cycle formed
  SITE 2: note = MISC_FEATURE - Xaa is l-lysine Lu(III) DOTA conjugate
  SITE 7: note = MISC_FEATURE - Xaa is d-alanine
  SITE 10: note = MISC_FEATURE - NH2 attached to Cys
CXQYFPXILC

SEQ ID NO: 278 - protein, 10 aa, synthetic construct
  REGION 1..10: note = synthetic
  SITE 1: note = MISC_FEATURE - pentanoic acid attached to Cys
  REGION 1..10: note = MISC_FEATURE - cycle formed
  SITE 7: note = MISC_FEATURE - Xaa is 4-(R)-hydroxy-l-proline
  SITE 9: note = MISC_FEATURE - Xaa is l-norvaline
  SITE 10: note = MISC_FEATURE - NH2 attached to Cys
CRGYFPXIXC

SEQ ID NO: 279 - protein, 10 aa, synthetic construct
  REGION 1..10: note = synthetic
  SITE 1: note = MISC_FEATURE - isocaproic acid attached to Cys
  REGION 1..10: note = MISC_FEATURE - cycle formed
  SITE 2: note = MISC_FEATURE - Xaa is l-Citrulline
  SITE 7: note = MISC_FEATURE - Xaa is 4-(R)-hydroxy-l-proline
  SITE 10: note = MISC_FEATURE - NH2 attached to Cys
CXDYFPXILC

SEQ ID NO: 280 - protein, 10 aa, synthetic construct
  REGION 1..10: note = synthetic
  SITE 1: note = MISC_FEATURE - pentanoic acid attached to Cys
  REGION 1..10: note = MISC_FEATURE - cycle formed
  SITE 7: note = MISC_FEATURE - Xaa is 4-(R)-hydroxy-l-proline
  SITE 9: note = MISC_FEATURE - Xaa is l-cyclobutyl-glycine
  SITE 10: note = MISC_FEATURE - NH2 attached to Cys
CRQYFPXIXC

SEQ ID NO: 281 - protein, 12 aa, synthetic construct
  REGION 1..12: note = synthetic
  SITE 1: note = MISC_FEATURE - Acetyl attached to Asp
  SITE 3: note = MISC_FEATURE - Xaa is d-cysteine
  REGION 3..12: note = MISC_FEATURE - cycle formed
  SITE 5: note = MISC_FEATURE - Xaa is l-norleucine
  SITE 12: note = MISC_FEATURE - NH2 attached to Cys
DLXRXYFPAILC

SEQ ID NO: 282 - protein, 10 aa, synthetic construct
  REGION 1..10: note = synthetic
  SITE 1: note = MISC_FEATURE - isocaproic acid attached to Cys
  REGION 1..10: note = MISC_FEATURE - cycle formed
  SITE 2: note = MISC_FEATURE - Xaa is l-Citrulline
  SITE 3: note = MISC_FEATURE - Xaa is N -acetyl-lysine
  SITE 7: note = MISC_FEATURE - Xaa is d-alanine
  SITE 10: note = MISC_FEATURE - NH2 attached to Cys
CXXYFPXILC

SEQ ID NO: 283 - protein, 10 aa, synthetic construct
  REGION 1..10: note = synthetic
  SITE 1: note = MISC_FEATURE - isocaproic acid attached to Cys
  REGION 1..10: note = MISC_FEATURE - cycle formed
  SITE 2: note = MISC_FEATURE - Xaa is d-alanine
  SITE 7: note = MISC_FEATURE - Xaa is l-lysine DOTA conjugate
  SITE 10: note = MISC_FEATURE - NH2 attached to Cys
CXQYFPXILC

SEQ ID NO: 284 - protein, 10 aa, synthetic construct
  REGION 1..10: note = synthetic
  SITE 1: note = MISC_FEATURE - n-butyloxycarbonyl attached to Cys
  REGION 1..10: note = MISC_FEATURE - cycle formed
  SITE 3: note = MISC_FEATURE - Xaa is l-ornithine DOTA conjugate
  SITE 4: note = MISC_FEATURE - Xaa is l-3-hydroxy-phenylalanine
  SITE 6: note = MISC_FEATURE - Xaa is (2S,4S)-4-fluoro-pyrrolidine-2-carboxylic acid
  SITE 7: note = MISC_FEATURE - Xaa is 4-(R)-hydroxy-l-proline
  SITE 9: note = MISC_FEATURE - Xaa is l-norvaline
  SITE 10: note = MISC_FEATURE - NH2 attached to Cys
CTXXFXXIXC

SEQ ID NO: 285 - protein, 10 aa, synthetic construct
  REGION 1..10: note = synthetic
  SITE 1: note = MISC_FEATURE - pentanoic acid attached to Cys
  REGION 1..10: note = MISC_FEATURE - cycle formed
  SITE 2: note = MISC_FEATURE - Xaa is l-Citrulline
  SITE 3: note = MISC_FEATURE - Xaa is l-lysine DOTA conjugate
  SITE 5: note = MISC_FEATURE - Xaa is -methyl-l-phenyl alanine
  SITE 7: note = MISC_FEATURE - Xaa is 4-(R)-hydroxy-l-proline
  SITE 9: note = MISC_FEATURE - Xaa is l-norvaline
  SITE 10: note = MISC_FEATURE - NH2 attached to Cys
CXXYXPXIXC

SEQ ID NO: 286 - protein, 10 aa, synthetic construct
  REGION 1..10: note = synthetic
  SITE 1: note = MISC_FEATURE - pentanoic acid attached to Cys
  REGION 1..10: note = MISC_FEATURE - cycle formed
  SITE 2: note = MISC_FEATURE - Xaa is l-Citrulline
  SITE 3: note = MISC_FEATURE - Xaa is l-lysine DOTA conjugate
  SITE 5: note = MISC_FEATURE - Xaa is 2-Aminoindane-2-carboxylic acid
  SITE 7: note = MISC_FEATURE - Xaa is 4-(R)-hydroxy-l-proline
  SITE 9: note = MISC_FEATURE - Xaa is l-norvaline
  SITE 10: note = MISC_FEATURE - NH2 attached to Cys
CXXYXPXIXC

SEQ ID NO: 287 - protein, 11 aa, synthetic construct
  REGION 1..11: note = synthetic
  SITE 1: note = MISC_FEATURE - Acetyl attached to Leu
  REGION 2..11: note = MISC_FEATURE - cycle formed
  SITE 3: note = MISC_FEATURE - Xaa is l-Citrulline
  SITE 8: note = MISC_FEATURE - Xaa is d-alanine
  SITE 11: note = MISC_FEATURE - NH2 attached to Cys
LCXQYFPXILC

SEQ ID NO: 288 - protein, 10 aa, synthetic construct
  REGION 1..10: note = synthetic
  SITE 1: note = MISC_FEATURE - pentanoic acid attached to Cys
  REGION 1..10: note = MISC_FEATURE - cycle formed
  SITE 3: note = MISC_FEATURE - Xaa is l-lysine DOTA conjugate
  SITE 6: note = MISC_FEATURE - Xaa is 1-amino-isobutyric acid
  SITE 7: note = MISC_FEATURE - Xaa is 4-(R)-hydroxy-l-proline
  SITE 9: note = MISC_FEATURE - Xaa is l-norvaline
  SITE 10: note = MISC_FEATURE - NH2 attached to Cys
CTXYFXXIXC

SEQ ID NO: 289 - protein, 12 aa, synthetic construct
  REGION 1..12: note = synthetic
  SITE 1: note = MISC_FEATURE - Acetyl attached to Asp
  REGION 3..12: note = MISC_FEATURE - cycle formed
  SITE 5: note = MISC_FEATURE - Xaa is l-norleucine
  SITE 10: note = MISC_FEATURE - Xaa is d-leucine
  SITE 12: note = MISC_FEATURE - NH2 attached to Cys
DLCRXYFPAXLC

SEQ ID NO: 290 - protein, 10 aa, synthetic construct
  REGION 1..10: note = synthetic
  SITE 1: note = MISC_FEATURE - n-butyloxycarbonyl attached to Cys
  REGION 1..10: note = MISC_FEATURE - cycle formed
  SITE 3: note = MISC_FEATURE - Xaa is l-lysine Kzw DOTA conjugate
  SITE 6: note = MISC_FEATURE - Xaa is (2S,4S)-4-fluoro-pyrrolidine-2-carboxylic acid
  SITE 7: note = MISC_FEATURE - Xaa is 4-(R)-hydroxy-l-proline
  SITE 9: note = MISC_FEATURE - Xaa is l-norvaline
  SITE 10: note = MISC_FEATURE - NH2 attached to Cys
CTXYFXXIXC

SEQ ID NO: 291 - protein, 12 aa, synthetic construct
  REGION 1..12: note = synthetic
  SITE 1: note = MISC_FEATURE - Acetyl attached to Asp
  REGION 3..12: note = MISC_FEATURE - cycle formed
  SITE 4: note = MISC_FEATURE - Xaa is l-Citrulline
  SITE 5: note = MISC_FEATURE - Xaa is l-lysine DOTA conjugate
  SITE 12: note = MISC_FEATURE - NH2 attached to Cys
DLCXXYFPRILC

SEQ ID NO: 292 - protein, 10 aa, synthetic construct
  REGION 1..10: note = synthetic
  SITE 1: note = MISC_FEATURE - n-butyloxycarbonyl attached to Cys
  REGION 1..10: note = MISC_FEATURE - cycle formed
  SITE 3: note = MISC_FEATURE - Xaa is l-lysine d-aspartate DOTA conjugate
  SITE 6: note = MISC_FEATURE - Xaa is (2S,4S)-4-fluoro-pyrrolidine-2-carboxylic acid
  SITE 7: note = MISC_FEATURE - Xaa is 4-(R)-hydroxy-l-proline
  SITE 9: note = MISC_FEATURE - Xaa is l-norvaline
  SITE 10: note = MISC_FEATURE - NH2 attached to Cys
CTXYFXXIXC

SEQ ID NO: 293 - protein, 10 aa, synthetic construct
  REGION 1..10: note = synthetic
  SITE 1: note = MISC_FEATURE - pentanoic acid attached to Cys
  REGION 1..10: note = MISC_FEATURE - cycle formed
  SITE 2: note = MISC_FEATURE - Xaa is l-Citrulline
  SITE 3: note = MISC_FEATURE - Xaa is l-lysine DOTA conjugate
  SITE 9: note = MISC_FEATURE - Xaa is l-norvaline
  SITE 10: note = MISC_FEATURE - NH2 attached to Cys
CXXYFPGIXC

SEQ ID NO: 294 - protein, 10 aa, synthetic construct
  REGION 1..10: note = synthetic
  SITE 1: note = MISC_FEATURE - isocaproic acid attached to Cys
  REGION 1..10: note = MISC_FEATURE - cycle formed
  SITE 2: note = MISC_FEATURE - Xaa is l-Citrulline
  SITE 6: note = MISC_FEATURE - Xaa is (S)-azetidine-2-carboxylic acid
  SITE 7: note = MISC_FEATURE - Xaa is d-alanine
  SITE 10: note = MISC_FEATURE - NH2 attached to Cys
CXQYFXXILC

SEQ ID NO: 295 - protein, 12 aa, synthetic construct
  REGION 1..12: note = synthetic
  SITE 1: note = MISC_FEATURE - hexanoic acid attached to Asp
  REGION 3..12: note = MISC_FEATURE - cycle formed
  SITE 5: note = MISC_FEATURE - Xaa is l-lysine DOTA conjugate
  SITE 12: note = MISC_FEATURE - NH2 attached to Cys
DLCRXYFPAILC

SEQ ID NO: 296 - protein, 11 aa, synthetic construct
  REGION 1..11: note = synthetic
  SITE 1: note = MISC_FEATURE - Xaa is N-methyl-l-norleucine
  REGION 2..11: note = MISC_FEATURE - cycle formed
  SITE 4: note = MISC_FEATURE - Xaa is l-lysine DOTA conjugate
  SITE 7: note = MISC_FEATURE - Xaa is (2S,4S)-4-fluoro-pyrrolidine-2-carboxylic acid
  SITE 8: note = MISC_FEATURE - Xaa is 4-(R)-hydroxy-l-proline
  SITE 10: note = MISC_FEATURE - Xaa is l-norvaline
  SITE 11: note = MISC_FEATURE - NH2 attached to Cys
XCTXYFXXIXC

SEQ ID NO: 297 - protein, 10 aa, synthetic construct
  REGION 1..10: note = synthetic
  SITE 1: note = MISC_FEATURE - isocaproic acid attached to Cys
  REGION 1..10: note = MISC_FEATURE - cycle formed
  SITE 2: note = MISC_FEATURE - Xaa is l-Citrulline
  SITE 7: note = MISC_FEATURE - Xaa is d-alanine
  SITE 9: note = MISC_FEATURE - Xaa is l-norvaline
  SITE 10: note = MISC_FEATURE - NH2 attached to Cys
CXQYFPXIXC

SEQ ID NO: 298 - protein, 10 aa, synthetic construct
  REGION 1..10: note = synthetic
  SITE 1: note = MISC_FEATURE - pentanoic acid attached to Cys
  REGION 1..10: note = MISC_FEATURE - cycle formed
  SITE 2: note = MISC_FEATURE - Xaa is l-Citrulline
  SITE 7: note = MISC_FEATURE - Xaa is 4-(R)-hydroxy-l-proline
  SITE 9: note = MISC_FEATURE - Xaa is l-norvaline
  SITE 10: note = MISC_FEATURE - ethylenediamine (used as C-terminus) attached to Cys
CXQYFPXIXC

SEQ ID NO: 299 - protein, 12 aa, synthetic construct
  REGION 1..12: note = synthetic
  SITE 1: note = MISC_FEATURE - Acetyl attached to Asp
  REGION 3..12: note = MISC_FEATURE - cycle formed
  SITE 5: note = MISC_FEATURE - Xaa is l-norleucine
  SITE 12: note = MISC_FEATURE - NH2 attached to Cys
DLCRXYFPPILC

SEQ ID NO: 300 - protein, 12 aa, synthetic construct
  REGION 1..12: note = synthetic
  SITE 1: note = MISC_FEATURE - Acetyl attached to Asp
  REGION 3..12: note = MISC_FEATURE - cycle formed
  SITE 5: note = MISC_FEATURE - Xaa is l-lysine DOTA conjugate
  SITE 9: note = MISC_FEATURE - Xaa is d-alanine
  SITE 12: note = MISC_FEATURE - NH2 attached to Cys
DLCDXYFPXILC

SEQ ID NO: 301 - protein, 10 aa, synthetic construct
  REGION 1..10: note = synthetic
  SITE 1: note = MISC_FEATURE - pentanoic acid attached to Cys
  REGION 1..10: note = MISC_FEATURE - cycle formed
  SITE 7: note = MISC_FEATURE - Xaa is 4-(R)-hydroxy-l-proline
  SITE 9: note = MISC_FEATURE - Xaa is l-norvaline
  SITE 10: note = MISC_FEATURE - NH2 attached to Cys
CRQYFLXIXC

SEQ ID NO: 302 - protein, 10 aa, synthetic construct
  REGION 1..10: note = synthetic
  SITE 1: note = MISC_FEATURE - isocaproic acid attached to Cys
  REGION 1..10: note = MISC_FEATURE - cycle formed
  SITE 2: note = MISC_FEATURE - Xaa is l-Citrulline
  SITE 7: note = MISC_FEATURE - Xaa is d-alanine
  SITE 10: note = MISC_FEATURE - NH2 attached to Cys
CXDYFPXILC

SEQ ID NO: 303 - protein, 10 aa, synthetic construct
  REGION 1..10: note = synthetic
  SITE 1: note = MISC_FEATURE - pentanoic acid attached to Cys
  REGION 1..10: note = MISC_FEATURE - cycle formed
  SITE 2: note = MISC_FEATURE - Xaa is l-Citrulline
  SITE 3: note = MISC_FEATURE - Xaa is l-lysine Gd (III) DOTA conjugate
  SITE 7: note = MISC_FEATURE - Xaa is 4-(R)-Fluoro-l-proline
  SITE 9: note = MISC_FEATURE - Xaa is l-norvaline
  SITE 10: note = MISC_FEATURE - NH2 attached to Cys
CXXYFPXIXC

SEQ ID NO: 304 - protein, 10 aa, synthetic construct
  REGION 1..10: note = synthetic
  SITE 1: note = MISC_FEATURE - pentanoic acid attached to Cys
  REGION 1..10: note = MISC_FEATURE - cycle formed
  SITE 7: note = MISC_FEATURE - Xaa is d-glutamic acid
  SITE 9: note = MISC_FEATURE - Xaa is l-norvaline
  SITE 10: note = MISC_FEATURE - NH2 attached to Cys
CRQYFPXIXC

SEQ ID NO: 305 - protein, 10 aa, synthetic construct
  REGION 1..10: note = synthetic
  SITE 1: note = MISC_FEATURE - pentanoic acid attached to Cys
  REGION 1..10: note = MISC_FEATURE - cycle formed
  SITE 7: note = MISC_FEATURE - Xaa is 4-(R)-hydroxy-l-proline
  SITE 8: note = MISC_FEATURE - Xaa is l-phenylglycine
  SITE 9: note = MISC_FEATURE - Xaa is l-norvaline
  SITE 10: note = MISC_FEATURE - NH2 attached to Cys
CRQYFPXXXC

SEQ ID NO: 306 - protein, 10 aa, synthetic construct
  REGION 1..10: note = synthetic
  SITE 1: note = MISC_FEATURE - pentanoic acid attached to Cys
  REGION 1..10: note = MISC_FEATURE - cycle formed
  SITE 7: note = MISC_FEATURE - Xaa is (R)-ornithine
  SITE 9: note = MISC_FEATURE - Xaa is l-norvaline
  SITE 10: note = MISC_FEATURE - NH2 attached to Cys
CRQYFPXIXC

SEQ ID NO: 307 - protein, 10 aa, synthetic construct
  REGION 1..10: note = synthetic
  SITE 1: note = MISC_FEATURE - isocaproic acid attached to Cys
  REGION 1..10: note = MISC_FEATURE - cycle formed
  SITE 2: note = MISC_FEATURE - Xaa is l-Citrulline
  SITE 6: note = MISC_FEATURE - Xaa is 4-(R)-hydroxy-l-proline
  SITE 7: note = MISC_FEATURE - Xaa is d-alanine
  SITE 10: note = MISC_FEATURE - NH2 attached to Cys
CXQYFXXILC

SEQ ID NO: 308 - protein, 12 aa, synthetic construct
  REGION 1..12: note = synthetic
  SITE 1: note = MISC_FEATURE - Acetyl attached to Asp
  REGION 3..12: note = MISC_FEATURE - cycle formed
  SITE 5: note = MISC_FEATURE - Xaa is l-norleucine
  SITE 9: note = MISC_FEATURE - Xaa is 1-amino-isobutyric acid
  SITE 12: note = MISC_FEATURE - NH2 attached to Cys
DLCRXYFPXILC

SEQ ID NO: 309 - protein, 11 aa, synthetic construct
  REGION 1..11: note = synthetic
  SITE 1: note = MISC_FEATURE - 2,2 ,2 ,2 -(1,4,7,10-Tetraazacyclododecane-1,4,7,10-tetrayl)tetraacetic acid attached to Leu
  REGION 2..11: note = MISC_FEATURE - cycle formed
  SITE 3: note = MISC_FEATURE - Xaa is l-Citrulline
  SITE 8: note = MISC_FEATURE - Xaa is d-alanine
  SITE 11: note = MISC_FEATURE - NH2 attached to Cys
LCXQYFPXILC

SEQ ID NO: 310 - protein, 10 aa, synthetic construct
  REGION 1..10: note = synthetic
  SITE 1: note = MISC_FEATURE - pentanoic acid attached to Cys
  REGION 1..10: note = MISC_FEATURE - cycle formed
  SITE 7: note = MISC_FEATURE - Xaa is 4-(R)-hydroxy-l-proline
  SITE 9: note = MISC_FEATURE - Xaa is l-norvaline
  SITE 10: note = MISC_FEATURE - NH2 attached to Cys
CRQKFPXIXC

SEQ ID NO: 311 - protein, 10 aa, synthetic construct
  REGION 1..10: note = synthetic
  SITE 1: note = MISC_FEATURE - n-butyloxycarbonyl attached to Cys
  REGION 1..10: note = MISC_FEATURE - cycle formed
  SITE 3: note = MISC_FEATURE - Xaa is l-lysine NODAGA conjugate
  SITE 4: note = MISC_FEATURE - Xaa is Levodopa / l-3,4-dihydroxyphenylalanine
  SITE 6: note = MISC_FEATURE - Xaa is (2S,4S)-4-fluoro-pyrrolidine-2-carboxylic acid
  SITE 7: note = MISC_FEATURE - Xaa is 4-(R)-hydroxy-l-proline
  SITE 9: note = MISC_FEATURE - Xaa is l-norvaline
  SITE 10: note = MISC_FEATURE - NH2 attached to Cys
CTXXFXXIXC

SEQ ID NO: 312 - protein, 10 aa, synthetic construct
  REGION 1..10: note = synthetic
  SITE 1: note = MISC_FEATURE - isocaproic acid attached to Cys
  REGION 1..10: note = MISC_FEATURE - cycle formed
  SITE 2: note = MISC_FEATURE - Xaa is l-Citrulline
  SITE 3: note = MISC_FEATURE - Xaa is l-Citrulline
  SITE 7: note = MISC_FEATURE - Xaa is d-alanine
  SITE 10: note = MISC_FEATURE - NH2 attached to Cys
CXXYFPXILC

SEQ ID NO: 313 - protein, 10 aa, synthetic construct
  REGION 1..10: note = synthetic
  SITE 1: note = MISC_FEATURE - isocaproic acid attached to Cys
  REGION 1..10: note = MISC_FEATURE - cycle formed
  SITE 2: note = MISC_FEATURE - Xaa is l-Citrulline
  SITE 7: note = MISC_FEATURE - Xaa is (S)-azetidine-2-carboxylic acid
  SITE 10: note = MISC_FEATURE - NH2 attached to Cys
CXQYFPXILC

SEQ ID NO: 314 - protein, 10 aa, synthetic construct
  REGION 1..10: note = synthetic
  SITE 1: note = MISC_FEATURE - pentanoic acid attached to Cys
  REGION 1..10: note = MISC_FEATURE - cycle formed
  SITE 7: note = MISC_FEATURE - Xaa is 4-(R)-hydroxy-l-proline
  SITE 9: note = MISC_FEATURE - Xaa is l-norvaline
  SITE 10: note = MISC_FEATURE - NH2 attached to Cys
CRQYFPXFXC

SEQ ID NO: 315 - protein, 10 aa, synthetic construct
  REGION 1..10: note = synthetic
  SITE 1: note = MISC_FEATURE - pentanoic acid attached to Cys
  REGION 1..10: note = MISC_FEATURE - cycle formed
  SITE 7: note = MISC_FEATURE - Xaa is 4-(R)-hydroxy-l-proline
  SITE 9: note = MISC_FEATURE - Xaa is l-norvaline
  SITE 10: note = MISC_FEATURE - NH2 attached to Cys
CRKYFPXIXC

SEQ ID NO: 316 - protein, 12 aa, synthetic construct
  REGION 1..12: note = synthetic
  SITE 1: note = MISC_FEATURE - isocaproic acid attached to Cys
  REGION 1..10: note = MISC_FEATURE - cycle formed
  SITE 7: note = MISC_FEATURE - Xaa is d-alanine
  SITE 11: note = MISC_FEATURE - Xaa is 8-amino-3,6-dioxaoctanoic acid
  SITE 12: note = MISC_FEATURE - NH2 attached to l-lysine DOTA conjugate
  SITE 12: note = MISC_FEATURE - Xaa is l-lysine DOTA conjugate
CRQYFPXILCXX

SEQ ID NO: 317 - protein, 10 aa, synthetic construct
  REGION 1..10: note = synthetic
  SITE 1: note = MISC_FEATURE - pentanoic acid attached to Cys
  REGION 1..10: note = MISC_FEATURE - cycle formed
  SITE 2: note = MISC_FEATURE - Xaa is l-Citrulline
  SITE 3: note = MISC_FEATURE - Xaa is l-lysine DOTA conjugate
  SITE 5: note = MISC_FEATURE - Xaa is ortho-chloro-l-phenylalanine
  SITE 7: note = MISC_FEATURE - Xaa is 4-(R)-hydroxy-l-proline
  SITE 9: note = MISC_FEATURE - Xaa is l-norvaline
  SITE 10: note = MISC_FEATURE - NH2 attached to Cys
CXXYXPXIXC

SEQ ID NO: 318 - protein, 10 aa, synthetic construct
  REGION 1..10: note = synthetic
  SITE 1: note = MISC_FEATURE - isocaproic acid attached to Cys
  REGION 1..10: note = MISC_FEATURE - cycle formed
  SITE 2: note = MISC_FEATURE - Xaa is l-Citrulline
  SITE 7: note = MISC_FEATURE - Xaa is d-alanine
  SITE 9: note = MISC_FEATURE - Xaa is 2S-aminobutyric acid
  SITE 10: note = MISC_FEATURE - NH2 attached to Cys
CXQYFPXIXC

SEQ ID NO: 319 - protein, 10 aa, synthetic construct
  REGION 1..10: note = synthetic
  SITE 1: note = MISC_FEATURE - isocaproic acid attached to Cys
  REGION 1..10: note = MISC_FEATURE - cycle formed
  SITE 2: note = MISC_FEATURE - Xaa is l-Citrulline
  SITE 3: note = MISC_FEATURE - Xaa is l-lysine DOTA conjugate
  SITE 7: note = MISC_FEATURE - Xaa is 1-amino-isobutyric acid
  SITE 10: note = MISC_FEATURE - NH2 attached to Cys
CXXYFPXILC

SEQ ID NO: 320 - protein, 10 aa, synthetic construct
  REGION 1..10: note = synthetic
  SITE 1: note = MISC_FEATURE - isocaproic acid attached to Cys
  REGION 1..10: note = MISC_FEATURE - cycle formed
  SITE 2: note = MISC_FEATURE - Xaa is l-Citrulline
  SITE 7: note = MISC_FEATURE - Xaa is d-alanine
  SITE 8: note = MISC_FEATURE - Xaa is l-cyclobutyl-glycine
  SITE 10: note = MISC_FEATURE - NH2 attached to Cys
CXQYFPXXLC

SEQ ID NO: 321 - protein, 10 aa, synthetic construct
  REGION 1..10: note = synthetic
  SITE 1: note = MISC_FEATURE - pentanoic acid attached to Cys
  REGION 1..10: note = MISC_FEATURE - cycle formed
  SITE 7: note = MISC_FEATURE - Xaa is 4-(R)-hydroxy-l-proline
  SITE 9: note = MISC_FEATURE - Xaa is l-norvaline
  SITE 10: note = MISC_FEATURE - NH2 attached to Cys
CYQYFPXIXC

SEQ ID NO: 322 - protein, 10 aa, synthetic construct
  REGION 1..10: note = synthetic
  SITE 1: note = MISC_FEATURE - n-butyloxycarbonyl attached to Cys
  REGION 1..10: note = MISC_FEATURE - cycle formed
  SITE 3: note = MISC_FEATURE - Xaa is Dap DOTA conjugate
  SITE 6: note = MISC_FEATURE - Xaa is (2S,4S)-4-fluoro-pyrrolidine-2-carboxylic acid
  SITE 7: note = MISC_FEATURE - Xaa is 4-(R)-hydroxy-l-proline
  SITE 9: note = MISC_FEATURE - Xaa is l-norvaline
  SITE 10: note = MISC_FEATURE - NH2 attached to Cys
CTXYFXXIXC

SEQ ID NO: 323 - protein, 10 aa, synthetic construct
  REGION 1..10: note = synthetic
  SITE 1: note = MISC_FEATURE - n-butyloxycarbonyl attached to Cys
  REGION 1..10: note = MISC_FEATURE - cycle formed
  SITE 3: note = MISC_FEATURE - Xaa is Dab DOTA conjugate
  SITE 4: note = MISC_FEATURE - Xaa is Levodopa / l-3,4-dihydroxyphenylalanine
  SITE 6: note = MISC_FEATURE - Xaa is (2S,4S)-4-fluoro-pyrrolidine-2-carboxylic acid
  SITE 7: note = MISC_FEATURE - Xaa is 4-(R)-hydroxy-l-proline
  SITE 9: note = MISC_FEATURE - Xaa is l-norvaline
  SITE 10: note = MISC_FEATURE - NH2 attached to Cys
CTXXFXXIXC

SEQ ID NO: 324 - protein, 10 aa, synthetic construct
  REGION 1..10: note = synthetic
  SITE 1: note = MISC_FEATURE - isocaproic acid attached to Cys
  REGION 1..10: note = MISC_FEATURE - cycle formed
  SITE 7: note = MISC_FEATURE - Xaa is 4-aminopiperidine-4-carboxylic acid Gd (III) DOTA conjugate
  SITE 10: note = MISC_FEATURE - NH2 attached to Cys
CRQYFPXILC

SEQ ID NO: 325 - protein, 10 aa, synthetic construct
  REGION 1..10: note = synthetic
  SITE 1: note = MISC_FEATURE - isocaproic acid attached to Cys
  REGION 1..10: note = MISC_FEATURE - cycle formed
  SITE 7: note = MISC_FEATURE - Xaa is 4-(R)-hydroxy-l-proline
  SITE 10: note = MISC_FEATURE - NH2 attached to Cys
CRDYFPXILC

SEQ ID NO: 326 - protein, 10 aa, synthetic construct
  REGION 1..10: note = synthetic
  SITE 1: note = MISC_FEATURE - n-butyloxycarbonyl attached to Cys
  REGION 1..10: note = MISC_FEATURE - cycle formed
  SITE 3: note = MISC_FEATURE - Xaa is l-lysine d-aspartate DOTA conjugate
  SITE 4: note = MISC_FEATURE - Xaa is Levodopa / l-3,4-dihydroxyphenylalanine
  SITE 6: note = MISC_FEATURE - Xaa is (2S,4S)-4-fluoro-pyrrolidine-2-carboxylic acid
  SITE 7: note = MISC_FEATURE - Xaa is 4-(R)-hydroxy-l-proline
  SITE 9: note = MISC_FEATURE - Xaa is l-norvaline
  SITE 10: note = MISC_FEATURE - NH2 attached to Cys
CTXXFXXIXC

SEQ ID NO: 327 - protein, 11 aa, synthetic construct
  REGION 1..11: note = synthetic
  SITE 1: note = MISC_FEATURE - succinic acid at N-terminus attached to l-norvaline
  SITE 1: note = MISC_FEATURE - Xaa is l-norvaline
  REGION 2..11: note = MISC_FEATURE - cycle formed
  SITE 3: note = MISC_FEATURE - Xaa is l-Citrulline
  SITE 4: note = MISC_FEATURE - Xaa is l-lysine Gd (III) DOTA conjugate
  SITE 8: note = MISC_FEATURE - Xaa is 4-(R)-hydroxy-l-proline
  SITE 10: note = MISC_FEATURE - Xaa is l-norvaline
  SITE 11: note = MISC_FEATURE - NH2 attached to Cys
XCXXYFPXIXC

SEQ ID NO: 328 - protein, 10 aa, synthetic construct
  REGION 1..10: note = synthetic
  SITE 1: note = MISC_FEATURE - pentanoic acid attached to Cys
  REGION 1..10: note = MISC_FEATURE - cycle formed
  SITE 7: note = MISC_FEATURE - Xaa is 4-(R)-hydroxy-l-proline
  SITE 8: note = MISC_FEATURE - Xaa is l-homophenylalanine
  SITE 9: note = MISC_FEATURE - Xaa is l-norvaline
  SITE 10: note = MISC_FEATURE - NH2 attached to Cys
CRQYFPXXXC

SEQ ID NO: 329 - protein, 11 aa, synthetic construct
  REGION 1..11: note = synthetic
  SITE 1: note = MISC_FEATURE - Xaa is N-ethyl glycine
  REGION 2..11: note = MISC_FEATURE - cycle formed
  SITE 3: note = MISC_FEATURE - Xaa is l-Citrulline
  SITE 8: note = MISC_FEATURE - Xaa is d-alanine
  SITE 11: note = MISC_FEATURE - NH2 attached to Cys
XCXQYFPXILC

SEQ ID NO: 330 - protein, 10 aa, synthetic construct
  REGION 1..10: note = synthetic
  SITE 1: note = MISC_FEATURE - isocaproic acid attached to Cys
  REGION 1..10: note = MISC_FEATURE - cycle formed
  SITE 2: note = MISC_FEATURE - Xaa is l-Citrulline
  SITE 3: note = MISC_FEATURE - Xaa is l-lysine Gd (III) DOTA conjugate
  SITE 7: note = MISC_FEATURE - Xaa is d-alanine
  SITE 10: note = MISC_FEATURE - NH2 attached to Cys
CXXYFPXILC

SEQ ID NO: 331 - protein, 10 aa, synthetic construct
  REGION 1..10: note = synthetic
  SITE 1: note = MISC_FEATURE - n-butyl-carbamoyl attached to Cys
  REGION 1..10: note = MISC_FEATURE - cycle formed
  SITE 2: note = MISC_FEATURE - Xaa is l-Citrulline
  SITE 3: note = MISC_FEATURE - Xaa is l-lysine Lu(III) DOTA conjugate
  SITE 7: note = MISC_FEATURE - Xaa is 4-(R)-hydroxy-l-proline
  SITE 9: note = MISC_FEATURE - Xaa is l-norvaline
  SITE 10: note = MISC_FEATURE - NH2 attached to Cys
CXXYFPXIXC

SEQ ID NO: 332 - protein, 10 aa, synthetic construct
  REGION 1..10: note = synthetic
  SITE 1: note = MISC_FEATURE - pentanoic acid attached to Cys
  REGION 1..10: note = MISC_FEATURE - cycle formed
  SITE 7: note = MISC_FEATURE - Xaa is d-tyrosine
  SITE 9: note = MISC_FEATURE - Xaa is l-norvaline
  SITE 10: note = MISC_FEATURE - NH2 attached to Cys
CRQYFPXIXC

SEQ ID NO: 333 - protein, 10 aa, synthetic construct
  REGION 1..10: note = synthetic
  SITE 1: note = MISC_FEATURE - isocaproic acid attached to Cys
  REGION 1..10: note = MISC_FEATURE - cycle formed
  SITE 2: note = MISC_FEATURE - Xaa is l-lysine DOTA conjugate
  SITE 10: note = MISC_FEATURE - NH2 attached to Cys
CXQYFPPILC

SEQ ID NO: 334 - protein, 10 aa, synthetic construct
  REGION 1..10: note = synthetic
  SITE 1: note = MISC_FEATURE - isocaproic acid attached to Cys
  REGION 1..10: note = MISC_FEATURE - cycle formed
  SITE 2: note = MISC_FEATURE - Xaa is d-arginine
  SITE 7: note = MISC_FEATURE - Xaa is d-alanine
  SITE 10: note = MISC_FEATURE - NH2 attached to Cys
CXQYFPXILC

SEQ ID NO: 335 - protein, 10 aa, synthetic construct
  REGION 1..10: note = synthetic
  SITE 1: note = MISC_FEATURE - isocaproic acid attached to Cys
  REGION 1..10: note = MISC_FEATURE - cycle formed
  SITE 2: note = MISC_FEATURE - Xaa is 1-amino-isobutyric acid
  SITE 7: note = MISC_FEATURE - Xaa is d-alanine
  SITE 10: note = MISC_FEATURE - NH2 attached to Cys
CXQYFPXILC

SEQ ID NO: 336 - protein, 10 aa, synthetic construct
  REGION 1..10: note = synthetic
  SITE 1: note = MISC_FEATURE - isocaproic acid attached to Cys
  REGION 1..10: note = MISC_FEATURE - cycle formed
  SITE 2: note = MISC_FEATURE - Xaa is l-Citrulline
  SITE 7: note = MISC_FEATURE - Xaa is (S)-pipecolic Acid
  SITE 10: note = MISC_FEATURE - NH2 attached to Cys
CXQYFPXILC

SEQ ID NO: 337 - protein, 10 aa, synthetic construct
  REGION 1..10: note = synthetic
  SITE 1: note = MISC_FEATURE - pentanoic acid attached to Cys
  REGION 1..10: note = MISC_FEATURE - cycle formed
  SITE 6: note = MISC_FEATURE - Xaa is N-methyl-l-valine
  SITE 7: note = MISC_FEATURE - Xaa is 4-(R)-hydroxy-l-proline
  SITE 9: note = MISC_FEATURE - Xaa is l-norvaline
  SITE 10: note = MISC_FEATURE - NH2 attached to Cys
CRQYFXXIXC

SEQ ID NO: 338 - protein, 10 aa, synthetic construct
  REGION 1..10: note = synthetic
  SITE 1: note = MISC_FEATURE - pentanoic acid attached to Cys
  REGION 1..10: note = MISC_FEATURE - cycle formed
  SITE 3: note = MISC_FEATURE - Xaa is l-lysine DOTA conjugate
  SITE 7: note = MISC_FEATURE - Xaa is 4-(R)-hydroxy-l-proline
  SITE 9: note = MISC_FEATURE - Xaa is l-norvaline
  SITE 10: note = MISC_FEATURE - NH2 attached to Cys
CEXYFPXIXC

SEQ ID NO: 339 - protein, 10 aa, synthetic construct
  REGION 1..10: note = synthetic
  SITE 1: note = MISC_FEATURE - pentanoic acid attached to Cys
  REGION 1..10: note = MISC_FEATURE - cycle formed
  SITE 2: note = MISC_FEATURE - Xaa is l-Citrulline
  SITE 3: note = MISC_FEATURE - Xaa is l-lysine DOTA conjugate
  SITE 9: note = MISC_FEATURE - Xaa is l-norvaline
  SITE 10: note = MISC_FEATURE - NH2 attached to Cys
CXXYFPPIXC

SEQ ID NO: 340 - protein, 10 aa, synthetic construct
  REGION 1..10: note = synthetic
  SITE 1: note = MISC_FEATURE - isocaproic acid attached to Cys
  REGION 1..10: note = MISC_FEATURE - cycle formed
  SITE 2: note = MISC_FEATURE - Xaa is l-Citrulline
  SITE 7: note = MISC_FEATURE - Xaa is d-alanine
  SITE 9: note = MISC_FEATURE - Xaa is l-cyclohexyl-alanine
  SITE 10: note = MISC_FEATURE - NH2 attached to Cys
CXQYFPXIXC

SEQ ID NO: 341 - protein, 10 aa, synthetic construct
  REGION 1..10: note = synthetic
  SITE 1: note = MISC_FEATURE - hexanoic acid attached to Cys
  REGION 1..10: note = MISC_FEATURE - cycle formed
  SITE 2: note = MISC_FEATURE - Xaa is l-Citrulline
  SITE 7: note = MISC_FEATURE - Xaa is d-alanine
  SITE 10: note = MISC_FEATURE - NH2 attached to Cys
CXQYFPXILC

SEQ ID NO: 342 - skipped

SEQ ID NO: 343 - protein, 10 aa, synthetic construct
  REGION 1..10: note = synthetic
  SITE 1: note = MISC_FEATURE - isocaproic acid attached to Cys
  REGION 1..10: note = MISC_FEATURE - cycle formed
  SITE 2: note = MISC_FEATURE - Xaa is l-Citrulline
  SITE 7: note = MISC_FEATURE - Xaa is d-alanine
  SITE 9: note = MISC_FEATURE - Xaa is l-neopentyl-glycine
  SITE 10: note = MISC_FEATURE - NH2 attached to Cys
CXQYFPXIXC

SEQ ID NO: 344 - protein, 10 aa, synthetic construct
  REGION 1..10: note = synthetic
  SITE 1: note = MISC_FEATURE - pentanoic acid attached to Cys
  REGION 1..10: note = MISC_FEATURE - cycle formed
  SITE 4: note = MISC_FEATURE - Xaa is -methyl-l-phenyl alanine
  SITE 7: note = MISC_FEATURE - Xaa is 4-(R)-hydroxy-l-proline
  SITE 9: note = MISC_FEATURE - Xaa is l-norvaline
  SITE 10: note = MISC_FEATURE - NH2 attached to Cys
CRQXFPXIXC

SEQ ID NO: 345 - protein, 10 aa, synthetic construct
  REGION 1..10: note = synthetic
  SITE 1: note = MISC_FEATURE - n-butyloxycarbonyl attached to Cys
  REGION 1..10: note = MISC_FEATURE - cycle formed
  SITE 3: note = MISC_FEATURE - Xaa is l-lysine Ttds AF488 conjugate
  SITE 4: note = MISC_FEATURE - Xaa is Levodopa / l-3,4-dihydroxyphenylalanine
  SITE 6: note = MISC_FEATURE - Xaa is (2S,4S)-4-fluoro-pyrrolidine-2-carboxylic acid
  SITE 7: note = MISC_FEATURE - Xaa is 4-(R)-hydroxy-l-proline
  SITE 9: note = MISC_FEATURE - Xaa is l-norvaline
  SITE 10: note = MISC_FEATURE - NH2 attached to Cys
CTXXFXXIXC

SEQ ID NO: 346 - protein, 10 aa, synthetic construct
  REGION 1..10: note = synthetic
  SITE 1: note = MISC_FEATURE - pentanoic acid attached to Cys
  REGION 1..10: note = MISC_FEATURE - cycle formed
  SITE 7: note = MISC_FEATURE - Xaa is 4-(R)-hydroxy-l-proline
  SITE 9: note = MISC_FEATURE - Xaa is N-methyl-l-leucine
  SITE 10: note = MISC_FEATURE - NH2 attached to Cys
CRQYFPXIXC

SEQ ID NO: 347 - protein, 10 aa, synthetic construct
  REGION 1..10: note = synthetic
  SITE 1: note = MISC_FEATURE - pentanoic acid attached to Cys
  REGION 1..10: note = MISC_FEATURE - cycle formed
  SITE 7: note = MISC_FEATURE - Xaa is 4-(R)-hydroxy-l-proline
  SITE 9: note = MISC_FEATURE - Xaa is l-norvaline
  SITE 10: note = MISC_FEATURE - Xaa is cysteamine
CRQYFPXIXX

SEQ ID NO: 348 - protein, 11 aa, synthetic construct
  REGION 1..11: note = synthetic
  SITE 1: note = MISC_FEATURE - Acetyl attached to 1-amino-1-cyclohexan-carboxylic acid
  SITE 1: note = MISC_FEATURE - Xaa is 1-amino-1-cyclohexan-carboxylic acid
  REGION 2..11: note = MISC_FEATURE - cycle formed
  SITE 8: note = MISC_FEATURE - Xaa is 4-(R)-hydroxy-l-proline
  SITE 10: note = MISC_FEATURE - Xaa is l-norvaline
  SITE 11: note = MISC_FEATURE - NH2 attached to Cys
XCRQYFPXIXC

SEQ ID NO: 349 - protein, 11 aa, synthetic construct
  REGION 1..11: note = synthetic
  SITE 1: note = MISC_FEATURE - Acetyl attached to N-methyl-l-leucine
  SITE 1: note = MISC_FEATURE - Xaa is N-methyl-l-leucine
  REGION 2..11: note = MISC_FEATURE - cycle formed
  SITE 8: note = MISC_FEATURE - Xaa is 4-(R)-hydroxy-l-proline
  SITE 10: note = MISC_FEATURE - Xaa is l-norvaline
  SITE 11: note = MISC_FEATURE - NH2 attached to Cys
XCRQYFPXIXC

SEQ ID NO: 350 - protein, 11 aa, synthetic construct
  REGION 1..11: note = synthetic
  SITE 1: note = MISC_FEATURE - Acetyl attached to l-homophenylalanine
  SITE 1: note = MISC_FEATURE - Xaa is l-homophenylalanine
  REGION 2..11: note = MISC_FEATURE - cycle formed
  SITE 8: note = MISC_FEATURE - Xaa is 4-(R)-hydroxy-l-proline
  SITE 10: note = MISC_FEATURE - Xaa is l-norvaline
  SITE 11: note = MISC_FEATURE - NH2 attached to Cys
XCRQYFPXIXC

SEQ ID NO: 351 - protein, 11 aa, synthetic construct
  REGION 1..11: note = synthetic
  SITE 1: note = MISC_FEATURE - Acetyl attached to -methyl-l-leucine
  SITE 1: note = MISC_FEATURE - Xaa is -methyl-l-leucine
  REGION 2..11: note = MISC_FEATURE - cycle formed
  SITE 8: note = MISC_FEATURE - Xaa is 4-(R)-hydroxy-l-proline
  SITE 10: note = MISC_FEATURE - Xaa is l-norvaline
  SITE 11: note = MISC_FEATURE - NH2 attached to Cys
XCRQYFPXIXC

SEQ ID NO: 352 - protein, 11 aa, synthetic construct
  REGION 1..11: note = synthetic
  SITE 1: note = MISC_FEATURE - Acetyl attached to l-phenylglycine
  SITE 1: note = MISC_FEATURE - Xaa is l-phenylglycine
  REGION 2..11: note = MISC_FEATURE - cycle formed
  SITE 8: note = MISC_FEATURE - Xaa is 4-(R)-hydroxy-l-proline
  SITE 10: note = MISC_FEATURE - Xaa is l-norvaline
  SITE 11: note = MISC_FEATURE - NH2 attached to Cys
XCRQYFPXIXC

SEQ ID NO: 353 - protein, 11 aa, synthetic construct
  REGION 1..11: note = synthetic
  SITE 1: note = MISC_FEATURE - methyl attached to N-methyl-l-leucine
  SITE 1: note = MISC_FEATURE - Xaa is N-methyl-l-leucine
  REGION 2..11: note = MISC_FEATURE - cycle formed
  SITE 8: note = MISC_FEATURE - Xaa is 4-(R)-hydroxy-l-proline
  SITE 10: note = MISC_FEATURE - Xaa is l-norvaline
  SITE 11: note = MISC_FEATURE - NH2 attached to Cys
XCRQYFPXIXC

SEQ ID NO: 354 - protein, 11 aa, synthetic construct
  REGION 1..11: note = synthetic
  SITE 1: note = MISC_FEATURE - Acetyl attached to Phe
  REGION 2..11: note = MISC_FEATURE - cycle formed
  SITE 8: note = MISC_FEATURE - Xaa is 4-(R)-hydroxy-l-proline
  SITE 10: note = MISC_FEATURE - Xaa is l-norvaline
  SITE 11: note = MISC_FEATURE - NH2 attached to Cys
FCRQYFPXIXC

SEQ ID NO: 355 - protein, 10 aa, synthetic construct
  REGION 1..10: note = synthetic
  SITE 1: note = MISC_FEATURE - n-butyloxycarbonyl attached to Cys
  REGION 1..10: note = MISC_FEATURE - cycle formed
  SITE 3: note = MISC_FEATURE - Xaa is l-ornithine Ga(III) DOTA conjugate
  SITE 4: note = MISC_FEATURE - Xaa is 4-carbamoyl-l-phenylalanine
  SITE 6: note = MISC_FEATURE - Xaa is (2S,4S)-4-fluoro-pyrrolidine-2-carboxylic acid
  SITE 7: note = MISC_FEATURE - Xaa is 4-(R)-hydroxy-l-proline
  SITE 9: note = MISC_FEATURE - Xaa is l-norvaline
  SITE 10: note = MISC_FEATURE - NH2 attached to Cys
CTXXFXXIXC

SEQ ID NO: 356 - protein, 10 aa, synthetic construct
  REGION 1..10: note = synthetic
  SITE 1: note = MISC_FEATURE - n-butyloxycarbonyl attached to Cys
  REGION 1..10: note = MISC_FEATURE - cycle formed
  SITE 3: note = MISC_FEATURE - Xaa is l-ornithine In(III) DOTA conjugate
  SITE 4: note = MISC_FEATURE - Xaa is 4-carbamoyl-l-phenylalanine
  SITE 6: note = MISC_FEATURE - Xaa is (2S,4S)-4-fluoro-pyrrolidine-2-carboxylic acid
  SITE 7: note = MISC_FEATURE - Xaa is 4-(R)-hydroxy-l-proline
  SITE 9: note = MISC_FEATURE - Xaa is l-norvaline
  SITE 10: note = MISC_FEATURE - NH2 attached to Cys
CTXXFXXIXC

SEQ ID NO: 357 - protein, 10 aa, synthetic construct
  REGION 1..10: note = synthetic
  SITE 1: note = MISC_FEATURE - n-butyloxycarbonyl attached to Cys
  REGION 1..10: note = MISC_FEATURE - cycle formed
  SITE 3: note = MISC_FEATURE - Xaa is l-ornithine Lu(III) DOTA conjugate
  SITE 4: note = MISC_FEATURE - Xaa is 4-carbamoyl-l-phenylalanine
  SITE 6: note = MISC_FEATURE - Xaa is (2S,4S)-4-fluoro-pyrrolidine-2-carboxylic acid
  SITE 7: note = MISC_FEATURE - Xaa is 4-(R)-hydroxy-l-proline
  SITE 9: note = MISC_FEATURE - Xaa is l-norvaline
  SITE 10: note = MISC_FEATURE - NH2 attached to Cys
CTXXFXXIXC